European Patent Application EP 4 141 112 A1, published March 1, 2023. Title: RNA expression modulating or editing method via regulation of Cas13 protein. Applicant: Korea Advanced Institute of Science and Technology. Application KR PCT/KR2022/009993, filed July 8, 2022. The sequence listing filed with the application follows.

SEQUENCE LISTING (75 sequences)

SEQ ID NO: 1 - protein, 272 aa, synthetic construct
  REGION 1..272: note = N272 Fragment amino acid sequence
MNIPALVENQKKYFGTYSVMAMLNAQTVLDHIQKVADIEGEQNENNENLWFHPVMSHLYNAKNGYDKQPEKTMFIIERLQSYFPFLKIMAENQREYSNGKYKQNRVEVNSNDIFEVLKRAFGVLKMYRDLTNHYKTYEEKLNDGCEFLTSTEQPLSGMINNYYTVALRNMNERYGYKTEDLAFIQDKRFKFVKDAYGKKKSQVNTGFFLSLQDYNGDTQKKLHLSGVGIALLICLFLDKQYINIFLSRLPIFSSYNAQSEERRIIIRSFGIN

SEQ ID NO: 2 - protein, 2583 aa, synthetic construct
  REGION 1..2583: note = C273 Fragment amino acid sequence
SERILELYSLEUPROLYSASPARGILEHISSERGLULYSSERASNLYSSERVALALAMETASPMETLEUASNGLUVALLYSARGCYSPROASPGLULEUPHETHRTHRLEUSERALAGLULYSGLNSERARGPHEARGILEILESERASPASPHISASNGLUVALLEUMETLYSARGSERSERASPARGPHEVALPROLEULEULEUGLNTYRILEASPTYRGLYLYSLEUPHEASPHISILEARGPHEHISVALASNMETGLYLYSLEUARGTYRLEULEULYSALAASPLYSTHRCYSILEASPGLYGLNTHRARGVALARGVALILEGLUGLNPROLEUASNGLYPHEGLYARGLEUGLUGLUALAGLUTHRMETARGLYSGLNGLUASNGLYTHRPHEGLYASNSERGLYILEARGILEARGASPPHEGLUASNMETLYSARGASPASPALAASNPROALAASNTYRPROTYRILEVALASPTHRTYRTHRHISTYRILELEUGLUASNASNLYSVALGLUMETPHEILEASNASPLYSGLUASPSERALAPROLEULEUPROVALILEGLUASPASPARGTYRVALVALLYSTHRILEPROSERCYSARGMETSERTHRLEUGLUILEPROALAMETALAPHEHISMETPHELEUPHEGLYSERLYSLYSTHRGLULYSLEUILEVALASPVALHISASNARGTYRLYSARGLEUPHEGLNALAMETGLNLYSGLUGLUVALTHRALAGLUASNILEALASERPHEGLYILEALAGLUSERASPLEUPROGLNLYSILELEUASPLEUILESERGLYASNALAHISGLYLYSASPVALASPALAPHEILEARGLEUTHRVALASPASPMETLEUTHRASPTHRGLUARGARGILELYSARGPHELYSASPASPARGLYSSERILEARGSERALAASPASNLYSMETGLYLYSARGGLYPHELYSGLNILESERTHRGLYLYSLEUALAASPPHELEUALALYSASPILEVALLEUPHEGLNPROSERVALASNASPGLYGLUASNLYSILETHRGLYLEUASNTYRARGILEMETGLNSERALAILEALAVALTYRASPSERGLYASPASPTYRGLUALALYSGLNGLNPHELYSLEUMETPHEGLULYSALAARGLEUILEGLYLYSGLYTHRTHRGLUPROHISPROPHELEUTYRLYSVALPHEALAARGSERILEPROALAASNALAVALGLUPHETYRGLUARGTYRLEUILEGLUARGLYSPHETYRLEUTHRGLYLEUSERASNGLUILELYSLYSGLYASNARGVALASPVALPROPHEILEARGARGASPGLNASNLYSTRPLYSTHRPROALAMETLYSTHRLEUGLYARGILETYRSERGLUASPLEUPROVALGLULEUPROARGGLNMETPHEASPASNGLUILELYSSERHISLEULYSSERLEUPROGLNMETGLUGLYILEASPPHEASNASNALAASNVALTHRTYRLEUILEALAGLUTYRMETLYSARGVALLEUASPASPASPPHEGLNTHRPHETYRGLNTRPASNARGASNTYRARGTYRMETASPMETLEULYSGLYGLUTYRASPARGLYSGLYSERLEUGLNHISCYSPHETHRSERVALGLUGLUARGGLUGLYLEUTRPLYSGLUARGALASERARGTHRGLUARGTYRARGLYSGLNALASERASNLYSILEARGSERASNARGGLNMETARGASNALASERSERGLUGLUILEGLUTHRILELEUASPLYSARGLEUSERASNSERARGASNGLUTYRGLNLYSSERGLULYSVALILEARGARGTYRARGVALGLNASPALALEULEUPHELEULEUALALYSLYSTHRLEUTHRGLULEUALAASPPHEASPGLYGLUARGPHELYSLEULYSGLUILEMETPROASPALAGLULYSGLYILELEUSERGLUILEMETPROMETSERPHETHRPHEGLULYSGLYGLYLYSLYSTYRTHRILETHRSERGLUGLYMETLYSLEULYSASNTYRGLYASPPHEPHEVALLEUALASERASPLYSARGILEGLYASNLEULEUGLULEUVALGLYSERASPILEVALSERLYSGLUASPILEMETGLUGLUPHEASNLYSTYRASPGLNCYSARGPROGLUILESERSERILEVALPHEASNLEUGLULYSTRPALAPHEASPTHRTYRPROGLULEUSERALAARGVALASPARGGLUGLULYSVALASPPHELYSSERILELEULYSILELEULEUASNASNLYSASNILEASNLYSGLUGLNSERASPILELEUARGLYSILEARGASNALAPHEASPHISASNASNTYRPROASPLYSGLYVALVALGLUILELYSALALEUPROGLUILEALAMETSERILELYSLYSALAPHEGLYGLUTYRALAILEMETLYSGLYSERLEUGLNLEUPROPROLEUGLUARGLEUTHRLEUGLYSERSERTYRPROTYRASPVALPROASPTYRALATYRPROTYRASPVALPROASPTYRALATYRPROTYRASPVALPROASPTYRALA

SEQ ID NO: 3 - protein, 286 aa, synthetic construct
  REGION 1..286: note = N286 Fragment amino acid sequence
MNIPALVENQKKYFGTYSVMAMLNAQTVLDHIQKVADIEGEQNENNENLWFHPVMSHLYNAKNGYDKQPEKTMFIIERLQSYFPFLKIMAENQREYSNGKYKQNRVEVNSNDIFEVLKRAFGVLKMYRDLTNHYKTYEEKLNDGCEFLTSTEQPLSGMINNYYTVALRNMNERYGYKTEDLAFIQDKRFKFVKDAYGKKKSQVNTGFFLSLQDYNGDTQKKLHLSGVGIALLICLFLDKQYINIFLSRLPIFSSYNAQSEERRIIIRSFGINSIKLPKDRIHSEKS

SEQ ID NO: 4 - protein, 2541 aa, synthetic construct
  REGION 1..2541: note = C287 Fragment amino acid sequence
ASNLYSSERVALALAMETASPMETLEUASNGLUVALLYSARGCYSPROASPGLULEUPHETHRTHRLEUSERALAGLULYSGLNSERARGPHEARGILEILESERASPASPHISASNGLUVALLEUMETLYSARGSERSERASPARGPHEVALPROLEULEULEUGLNTYRILEASPTYRGLYLYSLEUPHEASPHISILEARGPHEHISVALASNMETGLYLYSLEUARGTYRLEULEULYSALAASPLYSTHRCYSILEASPGLYGLNTHRARGVALARGVALILEGLUGLNPROLEUASNGLYPHEGLYARGLEUGLUGLUALAGLUTHRMETARGLYSGLNGLUASNGLYTHRPHEGLYASNSERGLYILEARGILEARGASPPHEGLUASNMETLYSARGASPASPALAASNPROALAASNTYRPROTYRILEVALASPTHRTYRTHRHISTYRILELEUGLUASNASNLYSVALGLUMETPHEILEASNASPLYSGLUASPSERALAPROLEULEUPROVALILEGLUASPASPARGTYRVALVALLYSTHRILEPROSERCYSARGMETSERTHRLEUGLUILEPROALAMETALAPHEHISMETPHELEUPHEGLYSERLYSLYSTHRGLULYSLEUILEVALASPVALHISASNARGTYRLYSARGLEUPHEGLNALAMETGLNLYSGLUGLUVALTHRALAGLUASNILEALASERPHEGLYILEALAGLUSERASPLEUPROGLNLYSILELEUASPLEUILESERGLYASNALAHISGLYLYSASPVALASPALAPHEILEARGLEUTHRVALASPASPMETLEUTHRASPTHRGLUARGARGILELYSARGPHELYSASPASPARGLYSSERILEARGSERALAASPASNLYSMETGLYLYSARGGLYPHELYSGLNILESERTHRGLYLYSLEUALAASPPHELEUALALYSASPILEVALLEUPHEGLNPROSERVALASNASPGLYGLUASNLYSILETHRGLYLEUASNTYRARGILEMETGLNSERALAILEALAVALTYRASPSERGLYASPASPTYRGLUALALYSGLNGLNPHELYSLEUMETPHEGLULYSALAARGLEUILEGLYLYSGLYTHRTHRGLUPROHISPROPHELEUTYRLYSVALPHEALAARGSERILEPROALAASNALAVALGLUPHETYRGLUARGTYRLEUILEGLUARGLYSPHETYRLEUTHRGLYLEUSERASNGLUILELYSLYSGLYASNARGVALASPVALPROPHEILEARGARGASPGLNASNLYSTRPLYSTHRPROALAMETLYSTHRLEUGLYARGILETYRSERGLUASPLEUPROVALGLULEUPROARGGLNMETPHEASPASNGLUILELYSSERHISLEULYSSERLEUPROGLNMETGLUGLYILEASPPHEASNASNALAASNVALTHRTYRLEUILEALAGLUTYRMETLYSARGVALLEUASPASPASPPHEGLNTHRPHETYRGLNTRPASNARGASNTYRARGTYRMETASPMETLEULYSGLYGLUTYRASPARGLYSGLYSERLEUGLNHISCYSPHETHRSERVALGLUGLUARGGLUGLYLEUTRPLYSGLUARGALASERARGTHRGLUARGTYRARGLYSGLNALASERASNLYSILEARGSERASNARGGLNMETARGASNALASERSERGLUGLUILEGLUTHRILELEUASPLYSARGLEUSERASNSERARGASNGLUTYRGLNLYSSERGLULYSVALILEARGARGTYRARGVALGLNASPALALEULEUPHELEULEUALALYSLYSTHRLEUTHRGLULEUALAASPPHEASPGLYGLUARGPHELYSLEULYSGLUILEMETPROASPALAGLULYSGLYILELEUSERGLUILEMETPROMETSERPHETHRPHEGLULYSGLYGLYLYSLYSTYRTHRILETHRSERGLUGLYMETLYSLEULYSASNTYRGLYASPPHEPHEVALLEUALASERASPLYSARGILEGLYASNLEULEUGLULEUVALGLYSERASPILEVALSERLYSGLUASPILEMETGLUGLUPHEASNLYSTYRASPGLNCYSARGPROGLUILESERSERILEVALPHEASNLEUGLULYSTRPALAPHEASPTHRTYRPROGLULEUSERALAARGVALASPARGGLUGLULYSVALASPPHELYSSERILELEULYSILELEULEUASNASNLYSASNILEASNLYSGLUGLNSERASPILELEUARGLYSILEARGASNALAPHEASPHISASNASNTYRPROASPLYSGLYVALVALGLUILELYSALALEUPROGLUILEALAMETSERILELYSLYSALAPHEGLYGLUTYRALAILEMETLYSGLYSERLEUGLNLEUPROPROLEUGLUARGLEUTHRLEUGLYSERSERTYRPROTYRASPVALPROASPTYRALATYRPROTYRASPVALPROASPTYRALATYRPROTYRASPVALPROASPTYRALA

SEQ ID NO: 5 - protein, 351 aa, synthetic construct
  REGION 1..351: note = N351 Fragment amino acid sequence
MNIPALVENQKKYFGTYSVMAMLNAQTVLDHIQKVADIEGEQNENNENLWFHPVMSHLYNAKNGYDKQPEKTMFIIERLQSYFPFLKIMAENQREYSNGKYKQNRVEVNSNDIFEVLKRAFGVLKMYRDLTNHYKTYEEKLNDGCEFLTSTEQPLSGMINNYYTVALRNMNERYGYKTEDLAFIQDKRFKFVKDAYGKKKSQVNTGFFLSLQDYNGDTQKKLHLSGVGIALLICLFLDKQYINIFLSRLPIFSSYNAQSEERRIIIRSFGINSIKLPKDRIHSEKSNKSVAMDMLNEVKRCPDELFTTLSAEKQSRFRIISDDHNEVLMKRSSDRFVPLLLQYIDYGKLFD

SEQ ID NO: 6 - protein, 2346 aa, synthetic construct
  REGION 1..2346: note = C352 Fragment amino acid sequence
HISILEARGPHEHISVALASNMETGLYLYSLEUARGTYRLEULEULYSALAASPLYSTHRCYSILEASPGLYGLNTHRARGVALARGVALILEGLUGLNPROLEUASNGLYPHEGLYARGLEUGLUGLUALAGLUTHRMETARGLYSGLNGLUASNGLYTHRPHEGLYASNSERGLYILEARGILEARGASPPHEGLUASNMETLYSARGASPASPALAASNPROALAASNTYRPROTYRILEVALASPTHRTYRTHRHISTYRILELEUGLUASNASNLYSVALGLUMETPHEILEASNASPLYSGLUASPSERALAPROLEULEUPROVALILEGLUASPASPARGTYRVALVALLYSTHRILEPROSERCYSARGMETSERTHRLEUGLUILEPROALAMETALAPHEHISMETPHELEUPHEGLYSERLYSLYSTHRGLULYSLEUILEVALASPVALHISASNARGTYRLYSARGLEUPHEGLNALAMETGLNLYSGLUGLUVALTHRALAGLUASNILEALASERPHEGLYILEALAGLUSERASPLEUPROGLNLYSILELEUASPLEUILESERGLYASNALAHISGLYLYSASPVALASPALAPHEILEARGLEUTHRVALASPASPMETLEUTHRASPTHRGLUARGARGILELYSARGPHELYSASPASPARGLYSSERILEARGSERALAASPASNLYSMETGLYLYSARGGLYPHELYSGLNILESERTHRGLYLYSLEUALAASPPHELEUALALYSASPILEVALLEUPHEGLNPROSERVALASNASPGLYGLUASNLYSILETHRGLYLEUASNTYRARGILEMETGLNSERALAILEALAVALTYRASPSERGLYASPASPTYRGLUALALYSGLNGLNPHELYSLEUMETPHEGLULYSALAARGLEUILEGLYLYSGLYTHRTHRGLUPROHISPROPHELEUTYRLYSVALPHEALAARGSERILEPROALAASNALAVALGLUPHETYRGLUARGTYRLEUILEGLUARGLYSPHETYRLEUTHRGLYLEUSERASNGLUILELYSLYSGLYASNARGVALASPVALPROPHEILEARGARGASPGLNASNLYSTRPLYSTHRPROALAMETLYSTHRLEUGLYARGILETYRSERGLUASPLEUPROVALGLULEUPROARGGLNMETPHEASPASNGLUILELYSSERHISLEULYSSERLEUPROGLNMETGLUGLYILEASPPHEASNASNALAASNVALTHRTYRLEUILEALAGLUTYRMETLYSARGVALLEUASPASPASPPHEGLNTHRPHETYRGLNTRPASNARGASNTYRARGTYRMETASPMETLEULYSGLYGLUTYRASPARGLYSGLYSERLEUGLNHISCYSPHETHRSERVALGLUGLUARGGLUGLYLEUTRPLYSGLUARGALASERARGTHRGLUARGTYRARGLYSGLNALASERASNLYSILEARGSERASNARGGLNMETARGASNALASERSERGLUGLUILEGLUTHRILELEUASPLYSARGLEUSERASNSERARGASNGLUTYRGLNLYSSERGLULYSVALILEARGARGTYRARGVALGLNASPALALEULEUPHELEULEUALALYSLYSTHRLEUTHRGLULEUALAASPPHEASPGLYGLUARGPHELYSLEULYSGLUILEMETPROASPALAGLULYSGLYILELEUSERGLUILEMETPROMETSERPHETHRPHEGLULYSGLYGLYLYSLYSTYRTHRILETHRSERGLUGLYMETLYSLEULYSASNTYRGLYASPPHEPHEVALLEUALASERASPLYSARGILEGLYASNLEULEUGLULEUVALGLYSERASPILEVALSERLYSGLUASPILEMETGLUGLUPHEASNLYSTYRASPGLNCYSARGPROGLUILESERSERILEVALPHEASNLEUGLULYSTRPALAPHEASPTHRTYRPROGLULEUSERALAARGVALASPARGGLUGLULYSVALASPPHELYSSERILELEULYSILELEULEUASNASNLYSASNILEASNLYSGLUGLNSERASPILELEUARGLYSILEARGASNALAPHEASPHISASNASNTYRPROASPLYSGLYVALVALGLUILELYSALALEUPROGLUILEALAMETSERILELYSLYSALAPHEGLYGLUTYRALAILEMETLYSGLYSERLEUGLNLEUPROPROLEUGLUARGLEUTHRLEUGLYSERSERTYRPROTYRASPVALPROASPTYRALATYRPROTYRASPVALPROASPTYRALATYRPROTYRASPVALPROASPTYRALA

SEQ ID NO: 7 - protein, 480 aa, synthetic construct
  REGION 1..480: note = N480 Fragment amino acid sequence
MNIPALVENQKKYFGTYSVMAMLNAQTVLDHIQKVADIEGEQNENNENLWFHPVMSHLYNAKNGYDKQPEKTMFIIERLQSYFPFLKIMAENQREYSNGKYKQNRVEVNSNDIFEVLKRAFGVLKMYRDLTNHYKTYEEKLNDGCEFLTSTEQPLSGMINNYYTVALRNMNERYGYKTEDLAFIQDKRFKFVKDAYGKKKSQVNTGFFLSLQDYNGDTQKKLHLSGVGIALLICLFLDKQYINIFLSRLPIFSSYNAQSEERRIIIRSFGINSIKLPKDRIHSEKSNKSVAMDMLNEVKRCPDELFTTLSAEKQSRFRIISDDHNEVLMKRSSDRFVPLLLQYIDYGKLFDHIRFHVNMGKLRYLLKADKTCIDGQTRVRVIEQPLNGFGRLEEAETMRKQENGTFGNSGIRIRDFENMKRDDANPANYPYIVDTYTHYILENNKVEMFINDKEDSAPLLPVIEDDRYVVKTIPSCRMST

SEQ ID NO: 8 - protein, 1959 aa, synthetic construct
  REGION 1..1959: note = C481 Fragment amino acid sequence
LEUGLUILEPROALAMETALAPHEHISMETPHELEUPHEGLYSERLYSLYSTHRGLULYSLEUILEVALASPVALHISASNARGTYRLYSARGLEUPHEGLNALAMETGLNLYSGLUGLUVALTHRALAGLUASNILEALASERPHEGLYILEALAGLUSERASPLEUPROGLNLYSILELEUASPLEUILESERGLYASNALAHISGLYLYSASPVALASPALAPHEILEARGLEUTHRVALASPASPMETLEUTHRASPTHRGLUARGARGILELYSARGPHELYSASPASPARGLYSSERILEARGSERALAASPASNLYSMETGLYLYSARGGLYPHELYSGLNILESERTHRGLYLYSLEUALAASPPHELEUALALYSASPILEVALLEUPHEGLNPROSERVALASNASPGLYGLUASNLYSILETHRGLYLEUASNTYRARGILEMETGLNSERALAILEALAVALTYRASPSERGLYASPASPTYRGLUALALYSGLNGLNPHELYSLEUMETPHEGLULYSALAARGLEUILEGLYLYSGLYTHRTHRGLUPROHISPROPHELEUTYRLYSVALPHEALAARGSERILEPROALAASNALAVALGLUPHETYRGLUARGTYRLEUILEGLUARGLYSPHETYRLEUTHRGLYLEUSERASNGLUILELYSLYSGLYASNARGVALASPVALPROPHEILEARGARGASPGLNASNLYSTRPLYSTHRPROALAMETLYSTHRLEUGLYARGILETYRSERGLUASPLEUPROVALGLULEUPROARGGLNMETPHEASPASNGLUILELYSSERHISLEULYSSERLEUPROGLNMETGLUGLYILEASPPHEASNASNALAASNVALTHRTYRLEUILEALAGLUTYRMETLYSARGVALLEUASPASPASPPHEGLNTHRPHETYRGLNTRPASNARGASNTYRARGTYRMETASPMETLEULYSGLYGLUTYRASPARGLYSGLYSERLEUGLNHISCYSPHETHRSERVALGLUGLUARGGLUGLYLEUTRPLYSGLUARGALASERARGTHRGLUARGTYRARGLYSGLNALASERASNLYSILEARGSERASNARGGLNMETARGASNALASERSERGLUGLUILEGLUTHRILELEUASPLYSARGLEUSERASNSERARGASNGLUTYRGLNLYSSERGLULYSVALILEARGARGTYRARGVALGLNASPALALEULEUPHELEULEUALALYSLYSTHRLEUTHRGLULEUALAASPPHEASPGLYGLUARGPHELYSLEULYSGLUILEMETPROASPALAGLULYSGLYILELEUSERGLUILEMETPROMETSERPHETHRPHEGLULYSGLYGLYLYSLYSTYRTHRILETHRSERGLUGLYMETLYSLEULYSASNTYRGLYASPPHEPHEVALLEUALASERASPLYSARGILEGLYASNLEULEUGLULEUVALGLYSERASPILEVALSERLYSGLUASPILEMETGLUGLUPHEASNLYSTYRASPGLNCYSARGPROGLUILESERSERILEVALPHEASNLEUGLULYSTRPALAPHEASPTHRTYRPROGLULEUSERALAARGVALASPARGGLUGLULYSVALASPPHELYSSERILELEULYSILELEULEUASNASNLYSASNILEASNLYSGLUGLNSERASPILELEUARGLYSILEARGASNALAPHEASPHISASNASNTYRPROASPLYSGLYVALVALGLUILELYSALALEUPROGLUILEALAMETSERILELYSLYSALAPHEGLYGLUTYRALAILEMETLYSGLYSERLEUGLNLEUPROPROLEUGLUARGLEUTHRLEUGLYSERSERTYRPROTYRASPVALPROASPTYRALATYRPROTYRASPVALPROASPTYRALATYRPROTYRASPVALPROASPTYRALA

SEQ ID NO: 9 - protein, 550 aa, synthetic construct
  REGION 1..550: note = N550 Fragment amino acid sequence
MNIPALVENQKKYFGTYSVMAMLNAQTVLDHIQKVADIEGEQNENNENLWFHPVMSHLYNAKNGYDKQPEKTMFIIERLQSYFPFLKIMAENQREYSNGKYKQNRVEVNSNDIFEVLKRAFGVLKMYRDLTNHYKTYEEKLNDGCEFLTSTEQPLSGMINNYYTVALRNMNERYGYKTEDLAFIQDKRFKFVKDAYGKKKSQVNTGFFLSLQDYNGDTQKKLHLSGVGIALLICLFLDKQYINIFLSRLPIFSSYNAQSEERRIIIRSFGINSIKLPKDRIHSEKSNKSVAMDMLNEVKRCPDELFTTLSAEKQSRFRIISDDHNEVLMKRSSDRFVPLLLQYIDYGKLFDHIRFHVNMGKLRYLLKADKTCIDGQTRVRVIEQPLNGFGRLEEAETMRKQENGTFGNSGIRIRDFENMKRDDANPANYPYIVDTYTHYILENNKVEMFINDKEDSAPLLPVIEDDRYVVKTIPSCRMSTLEIPAMAFHMFLFGSKKTEKLIVDVHNRYKRLFQAMQKEEVTAENIASFGIAESDLPQKILDLISGNAHG

SEQ ID NO: 10 - protein, 1749 aa, synthetic construct
  REGION 1..1749: note = C551 Fragment amino acid sequence
LYSASPVALASPALAPHEILEARGLEUTHRVALASPASPMETLEUTHRASPTHRGLUARGARGILELYSARGPHELYSASPASPARGLYSSERILEARGSERALAASPASNLYSMETGLYLYSARGGLYPHELYSGLNILESERTHRGLYLYSLEUALAASPPHELEUALALYSASPILEVALLEUPHEGLNPROSERVALASNASPGLYGLUASNLYSILETHRGLYLEUASNTYRARGILEMETGLNSERALAILEALAVALTYRASPSERGLYASPASPTYRGLUALALYSGLNGLNPHELYSLEUMETPHEGLULYSALAARGLEUILEGLYLYSGLYTHRTHRGLUPROHISPROPHELEUTYRLYSVALPHEALAARGSERILEPROALAASNALAVALGLUPHETYRGLUARGTYRLEUILEGLUARGLYSPHETYRLEUTHRGLYLEUSERASNGLUILELYSLYSGLYASNARGVALASPVALPROPHEILEARGARGASPGLNASNLYSTRPLYSTHRPROALAMETLYSTHRLEUGLYARGILETYRSERGLUASPLEUPROVALGLULEUPROARGGLNMETPHEASPASNGLUILELYSSERHISLEULYSSERLEUPROGLNMETGLUGLYILEASPPHEASNASNALAASNVALTHRTYRLEUILEALAGLUTYRMETLYSARGVALLEUASPASPASPPHEGLNTHRPHETYRGLNTRPASNARGASNTYRARGTYRMETASPMETLEULYSGLYGLUTYRASPARGLYSGLYSERLEUGLNHISCYSPHETHRSERVALGLUGLUARGGLUGLYLEUTRPLYSGLUARGALASERARGTHRGLUARGTYRARGLYSGLNALASERASNLYSILEARGSERASNARGGLNMETARGASNALASERSERGLUGLUILEGLUTHRILELEUASPLYSARGLEUSERASNSERARGASNGLUTYRGLNLYSSERGLULYSVALILEARGARGTYRARGVALGLNASPALALEULEUPHELEULEUALALYSLYSTHRLEUTHRGLULEUALAASPPHEASPGLYGLUARGPHELYSLEULYSGLUILEMETPROASPALAGLULYSGLYILELEUSERGLUILEMETPROMETSERPHETHRPHEGLULYSGLYGLYLYSLYSTYRTHRILETHRSERGLUGLYMETLYSLEULYSASNTYRGLYASPPHEPHEVALLEUALASERASPLYSARGILEGLYASNLEULEUGLULEUVALGLYSERASPILEVALSERLYSGLUASPILEMETGLUGLUPHEASNLYSTYRASPGLNCYSARGPROGLUILESERSERILEVALPHEASNLEUGLULYSTRPALAPHEASPTHRTYRPROGLULEUSERALAARGVALASPARGGLUGLULYSVALASPPHELYSSERILELEULYSILELEULEUASNASNLYSASNILEASNLYSGLUGLNSERASPILELEUARGLYSILEARGASNALAPHEASPHISASNASNTYRPROASPLYSGLYVALVALGLUILELYSALALEUPROGLUILEALAMETSERILELYSLYSALAPHEGLYGLUTYRALAILEMETLYSGLYSERLEUGLNLEUPROPROLEUGLUARGLEUTHRLEUGLYSERSERTYRPROTYRASPVALPROASPTYRALATYRPROTYRASPVALPROASPTYRALATYRPROTYRASPVALPROASPTYRALA

SEQ ID NO: 11 - protein, 624 aa, synthetic construct
  REGION 1..624: note = N624 Fragment amino acid sequence
MNIPALVENQKKYFGTYSVMAMLNAQTVLDHIQKVADIEGEQNENNENLWFHPVMSHLYNAKNGYDKQPEKTMFIIERLQSYFPFLKIMAENQREYSNGKYKQNRVEVNSNDIFEVLKRAFGVLKMYRDLTNHYKTYEEKLNDGCEFLTSTEQPLSGMINNYYTVALRNMNERYGYKTEDLAFIQDKRFKFVKDAYGKKKSQVNTGFFLSLQDYNGDTQKKLHLSGVGIALLICLFLDKQYINIFLSRLPIFSSYNAQSEERRIIIRSFGINSIKLPKDRIHSEKSNKSVAMDMLNEVKRCPDELFTTLSAEKQSRFRIISDDHNEVLMKRSSDRFVPLLLQYIDYGKLFDHIRFHVNMGKLRYLLKADKTCIDGQTRVRVIEQPLNGFGRLEEAETMRKQENGTFGNSGIRIRDFENMKRDDANPANYPYIVDTYTHYILENNKVEMFINDKEDSAPLLPVIEDDRYVVKTIPSCRMSTLEIPAMAFHMFLFGSKKTEKLIVDVHNRYKRLFQAMQKEEVTAENIASFGIAESDLPQKILDLISGNAHGKDVDAFIRLTVDDMLTDTERRIKRFKDDRKSIRSADNKMGKRGFKQISTGKLADFLAKDIVLFQPSVNDGENKI

SEQ ID NO: 12 - protein, 1527 aa, synthetic construct
  REGION 1..1527: note = C625 Fragment amino acid sequence
THRGLYLEUASNTYRARGILEMETGLNSERALAILEALAVALTYRASPSERGLYASPASPTYRGLUALALYSGLNGLNPHELYSLEUMETPHEGLULYSALAARGLEUILEGLYLYSGLYTHRTHRGLUPROHISPROPHELEUTYRLYSVALPHEALAARGSERILEPROALAASNALAVALGLUPHETYRGLUARGTYRLEUILEGLUARGLYSPHETYRLEUTHRGLYLEUSERASNGLUILELYSLYSGLYASNARGVALASPVALPROPHEILEARGARGASPGLNASNLYSTRPLYSTHRPROALAMETLYSTHRLEUGLYARGILETYRSERGLUASPLEUPROVALGLULEUPROARGGLNMETPHEASPASNGLUILELYSSERHISLEULYSSERLEUPROGLNMETGLUGLYILEASPPHEASNASNALAASNVALTHRTYRLEUILEALAGLUTYRMETLYSARGVALLEUASPASPASPPHEGLNTHRPHETYRGLNTRPASNARGASNTYRARGTYRMETASPMETLEULYSGLYGLUTYRASPARGLYSGLYSERLEUGLNHISCYSPHETHRSERVALGLUGLUARGGLUGLYLEUTRPLYSGLUARGALASERARGTHRGLUARGTYRARGLYSGLNALASERASNLYSILEARGSERASNARGGLNMETARGASNALASERSERGLUGLUILEGLUTHRILELEUASPLYSARGLEUSERASNSERARGASNGLUTYRGLNLYSSERGLULYSVALILEARGARGTYRARGVALGLNASPALALEULEUPHELEULEUALALYSLYSTHRLEUTHRGLULEUALAASPPHEASPGLYGLUARGPHELYSLEULYSGLUILEMETPROASPALAGLULYSGLYILELEUSERGLUILEMETPROMETSERPHETHRPHEGLULYSGLYGLYLYSLYSTYRTHRILETHRSERGLUGLYMETLYSLEULYSASNTYRGLYASPPHEPHEVALLEUALASERASPLYSARGILEGLYASNLEULEUGLULEUVALGLYSERASPILEVALSERLYSGLUASPILEMETGLUGLUPHEASNLYSTYRASPGLNCYSARGPROGLUILESERSERILEVALPHEASNLEUGLULYSTRPALAPHEASPTHRTYRPROGLULEUSERALAARGVALASPARGGLUGLULYSVALASPPHELYSSERILELEULYSILELEULEUASNASNLYSASNILEASNLYSGLUGLNSERASPILELEUARGLYSILEARGASNALAPHEASPHISASNASNTYRPROASPLYSGLYVALVALGLUILELYSALALEUPROGLUILEALAMETSERILELYSLYSALAPHEGLYGLUTYRALAILEMETLYSGLYSERLEUGLNLEUPROPROLEUGLUARGLEUTHRLEUGLYSERSERTYRPROTYRASPVALPROASPTYRALATYRPROTYRASPVALPROASPTYRALATYRPROTYRASPVALPROASPTYRALA

SEQ ID NO: 13 - protein, 725 aa, synthetic construct
  REGION 1..725: note = N725 Fragment amino acid sequence
MNIPALVENQKKYFGTYSVMAMLNAQTVLDHIQKVADIEGEQNENNENLWFHPVMSHLYNAKNGYDKQPEKTMFIIERLQSYFPFLKIMAENQREYSNGKYKQNRVEVNSNDIFEVLKRAFGVLKMYRDLTNHYKTYEEKLNDGCEFLTSTEQPLSGMINNYYTVALRNMNERYGYKTEDLAFIQDKRFKFVKDAYGKKKSQVNTGFFLSLQDYNGDTQKKLHLSGVGIALLICLFLDKQYINIFLSRLPIFSSYNAQSEERRIIIRSFGINSIKLPKDRIHSEKSNKSVAMDMLNEVKRCPDELFTTLSAEKQSRFRIISDDHNEVLMKRSSDRFVPLLLQYIDYGKLFDHIRFHVNMGKLRYLLKADKTCIDGQTRVRVIEQPLNGFGRLEEAETMRKQENGTFGNSGIRIRDFENMKRDDANPANYPYIVDTYTHYILENNKVEMFINDKEDSAPLLPVIEDDRYVVKTIPSCRMSTLEIPAMAFHMFLFGSKKTEKLIVDVHNRYKRLFQAMQKEEVTAENIASFGIAESDLPQKILDLISGNAHGKDVDAFIRLTVDDMLTDTERRIKRFKDDRKSIRSADNKMGKRGFKQISTGKLADFLAKDIVLFQPSVNDGENKITGLNYRIMQSAIAVYDSGDDYEAKQQFKLMFEKARLIGKGTTEPHPFLYKVFARSIPANAVEFYERYLIERKFYLTGLSNEIKKGNRVDVPFIRRDQNKWK

SEQ ID NO: 14 - protein, 1224 aa, synthetic construct
  REGION 1..1224: note = C726 Fragment amino acid sequence
THRPROALAMETLYSTHRLEUGLYARGILETYRSERGLUASPLEUPROVALGLULEUPROARGGLNMETPHEASPASNGLUILELYSSERHISLEULYSSERLEUPROGLNMETGLUGLYILEASPPHEASNASNALAASNVALTHRTYRLEUILEALAGLUTYRMETLYSARGVALLEUASPASPASPPHEGLNTHRPHETYRGLNTRPASNARGASNTYRARGTYRMETASPMETLEULYSGLYGLUTYRASPARGLYSGLYSERLEUGLNHISCYSPHETHRSERVALGLUGLUARGGLUGLYLEUTRPLYSGLUARGALASERARGTHRGLUARGTYRARGLYSGLNALASERASNLYSILEARGSERASNARGGLNMETARGASNALASERSERGLUGLUILEGLUTHRILELEUASPLYSARGLEUSERASNSERARGASNGLUTYRGLNLYSSERGLULYSVALILEARGARGTYRARGVALGLNASPALALEULEUPHELEULEUALALYSLYSTHRLEUTHRGLULEUALAASPPHEASPGLYGLUARGPHELYSLEULYSGLUILEMETPROASPALAGLULYSGLYILELEUSERGLUILEMETPROMETSERPHETHRPHEGLULYSGLYGLYLYSLYSTYRTHRILETHRSERGLUGLYMETLYSLEULYSASNTYRGLYASPPHEPHEVALLEUALASERASPLYSARGILEGLYASNLEULEUGLULEUVALGLYSERASPILEVALSERLYSGLUASPILEMETGLUGLUPHEASNLYSTYRASPGLNCYSARGPROGLUILESERSERILEVALPHEASNLEUGLULYSTRPALAPHEASPTHRTYRPROGLULEUSERALAARGVALASPARGGLUGLULYSVALASPPHELYSSERILELEULYSILELEULEUASNASNLYSASNILEASNLYSGLUGLNSERASPILELEUARGLYSILEARGASNALAPHEASPHISASNASNTYRPROASPLYSGLYVALVALGLUILELYSALALEUPROGLUILEALAMETSERILELYSLYSALAPHEGLYGLUTYRALAILEMETLYSGLYSERLEUGLNLEUPROPROLEUGLUARGLEUTHRLEUGLYSERSERTYRPROTYRASPVALPROASPTYRALATYRPROTYRASPVALPROASPTYRALATYRPROTYRASPVALPROASPTYRALA

SEQ ID NO: 15 - protein, 928 aa, synthetic construct
  REGION 1..928: note = N928 Fragment amino acid sequence
MNIPALVENQKKYFGTYSVMAMLNAQTVLDHIQKVADIEGEQNENNENLWFHPVMSHLYNAKNGYDKQPEKTMFIIERLQSYFPFLKIMAENQREYSNGKYKQNRVEVNSNDIFEVLKRAFGVLKMYRDLTNHYKTYEEKLNDGCEFLTSTEQPLSGMINNYYTVALRNMNERYGYKTEDLAFIQDKRFKFVKDAYGKKKSQVNTGFFLSLQDYNGDTQKKLHLSGVGIALLICLFLDKQYINIFLSRLPIFSSYNAQSEERRIIIRSFGINSIKLPKDRIHSEKSNKSVAMDMLNEVKRCPDELFTTLSAEKQSRFRIISDDHNEVLMKRSSDRFVPLLLQYIDYGKLFDHIRFHVNMGKLRYLLKADKTCIDGQTRVRVIEQPLNGFGRLEEAETMRKQENGTFGNSGIRIRDFENMKRDDANPANYPYIVDTYTHYILENNKVEMFINDKEDSAPLLPVIEDDRYVVKTIPSCRMSTLEIPAMAFHMFLFGSKKTEKLIVDVHNRYKRLFQAMQKEEVTAENIASFGIAESDLPQKILDLISGNAHGKDVDAFIRLTVDDMLTDTERRIKRFKDDRKSIRSADNKMGKRGFKQISTGKLADFLAKDIVLFQPSVNDGENKITGLNYRIMQSAIAVYDSGDDYEAKQQFKLMFEKARLIGKGTTEPHPFLYKVFARSIPANAVEFYERYLIERKFYLTGLSNEIKKGNRVDVPFIRRDQNKWKTPAMKTLGRIYSEDLPVELPRQMFDNEIKSHLKSLPQMEGIDFNNANVTYLIAEYMKRVLDDDFQTFYQWNRNYRYMDMLKGEYDRKGSLQHCFTSVEEREGLWKERASRTERYRKQASNKIRSNRQMRNASSEEIETILDKRLSNSRNEYQKSEKVIRRYRVQDALLFLLAKKTLTELADFDGERFKLKEIMPDAEKGILSE

SEQ ID NO: 16 - protein, 615 aa, synthetic construct
  REGION 1..615: note = C929 Fragment amino acid sequence
ILEMETPROMETSERPHETHRPHEGLULYSGLYGLYLYSLYSTYRTHRILETHRSERGLUGLYMETLYSLEULYSASNTYRGLYASPPHEPHEVALLEUALASERASPLYSARGILEGLYASNLEULEUGLULEUVALGLYSERASPILEVALSERLYSGLUASPILEMETGLUGLUPHEASNLYSTYRASPGLNCYSARGPROGLUILESERSERILEVALPHEASNLEUGLULYSTRPALAPHEASPTHRTYRPROGLULEUSERALAARGVALASPARGGLUGLULYSVALASPPHELYSSERILELEULYSILELEULEUASNASNLYSASNILEASNLYSGLUGLNSERASPILELEUARGLYSILEARGASNALAPHEASPHISASNASNTYRPROASPLYSGLYVALVALGLUILELYSALALEUPROGLUILEALAMETSERILELYSLYSALAPHEGLYGLUTYRALAILEMETLYSGLYSERLEUGLNLEUPROPROLEUGLUARGLEUTHRLEUGLYSERSERTYRPROTYRASPVALPROASPTYRALATYRPROTYRASPVALPROASPTYRALATYRPROTYRASPVALPROASPTYRALA

SEQ ID NO: 17 - protein, 93 aa, synthetic construct [sequence omitted]

SEQ ID NO: 18 - protein, 107 aa, synthetic construct
  REGION 1..107: note = FKBP amino acid sequence
GVQVETISPGDGRTFPKRGQTCVVHYTGMLEDGKKFDSSRDRNKPFKFMLGKQEVIRGWEEGVAQMSVGQRAKLTISPDYAYGATGHPGIIPPHATLVFDVELLKLE

SEQ ID NO: 19 - protein, 150 aa, synthetic construct
  REGION 1..150: note = nMag amino acid sequence
HTLYAPGGYDIMGYLDQIGNRPNPQVELGPVDTSCALILCDLKQKDTPIVYASEAFLYMTGYSNAEVLGRNCRFLQSPDGMVKPKSTRKYVDSNTINTMRKAIDRNAEVQVEVVNFKKNGQRFVNFLTMIPVRDETGEYRYSMGFQCETE

SEQ ID NO: 20 - protein, 150 aa, synthetic construct
  REGION 1..150: note = pMag amino acid sequence
HTLYAPGGYDIMGYLRQIRNRPNPQVELGPVDTSCALILCDLKQKDTPIVYASEAFLYMTGYSNAEVLGRNCRFLQSPDGMVKPKSTRKYVDSNTINTIRKAIDRNAEVQVEVVNFKKNGQRFVNFLTIIPVRDETGEYRYSMGFQCETE

SEQ ID NO: 21 - protein, 32 aa, synthetic construct
  REGION 1..32: note = linker
GSGSGSGSGSGSGSGSGSGSGSGSGSGSGSGS

SEQ ID NO: 22 - DNA, 816 bp, synthetic construct
  misc_feature 1..816: note = N272 Fragment polynucleotide sequence
  source 1..816: mol_type = other DNA
atgaacatccccgctctggtggaaaaccagaagaagtactttggcacctacagcgtgatggccatgctgaacgctcagaccgtgctggaccacatccagaaggtggccgatattgagggcgagcagaacgagaacaacgagaatctgtggtttcaccccgtgatgagccacctgtacaacgccaagaacggctacgacaagcagcccgagaaaaccatgttcatcatcgagcggctgcagagctacttcccattcctgaagatcatggccgagaaccagagagagtacagcaacggcaagtacaagcagaaccgcgtggaagtgaacagcaacgacatcttcgaggtgctgaagcgcgccttcggcgtgctgaagatgtacagggacctgaccaaccactacaagacctacgaggaaaagctgaacgacggctgcgagttcctgaccagcacagagcaacctctgagcggcatgatcaacaactactacacagtggccctgcggaacatgaacgagagatacggctacaagacagaggacctggccttcatccaggacaagcggttcaagttcgtgaaggacgcctacggcaagaaaaagtcccaagtgaataccggattcttcctgagcctgcaggactacaacggcgacacacagaagaagctgcacctgagcggagtgggaatcgccctgctgatctgcctgttcctggacaagcagtacatcaacatctttctgagcaggctgcccatcttctccagctacaatgcccagagcgaggaacggcggatcatcatcagatccttcggcatcaac

SEQ ID NO: 23 - DNA, 2586 bp, synthetic construct
  misc_feature 1..2586: note = C273 Fragment polynucleotide sequence
  source 1..2586: mol_type = other DNA
agcatcaagctgcccaaggaccggatccacagcgagaagtccaacaagagcgtggccatggatatgctcaacgaagtgaagcggtgccccgacgagctgttcacaacactgtctgccgagaagcagtcccggttcagaatcatcagcgacgaccacaatgaagtgctgatgaagcggagcagcgacagattcgtgcctctgctgctgcagtatatcgattacggcaagctgttcgaccacatcaggttccacgtgaacatgggcaagctgagatacctgctgaaggccgacaagacctgcatcgacggccagaccagagtcagagtgatcgagcagcccctgaacggcttcggcagactggaagaggccgagacaatgcggaagcaagagaacggcaccttcggcaacagcggcatccggatcagagacttcgagaacatgaagcgggacgacgccaatcctgccaactatccctacatcgtggacacctacacacactacatcctggaaaacaacaaggtcgagatgtttatcaacgacaaagaggacagcgccccactgctgcccgtgatcgaggatgatagatacgtggtcaagacaatccccagctgccggatgagcaccctggaaattccagccatggccttccacatgtttctgttcggcagcaagaaaaccgagaagctgatcgtggacgtgcacaaccggtacaagagactgttccaggccatgcagaaagaagaagtgaccgccgagaatatcgccagcttcggaatcgccgagagcgacctgcctcagaagatcctggatctgatcagcggcaatgcccacggcaaggatgtggacgccttcatcagactgaccgtggacgacatgctgaccgacaccgagcggagaatcaagagattcaaggacgaccggaagtccattcggagcgccgacaacaagatgggaaagagaggcttcaagcagatctccacaggcaagctggccgacttcctggccaaggacatcgtgctgtttcagcccagcgtgaacgatggcgagaacaagatcaccggcctgaactaccggatcatgcagagcgccattgccgtgtacgatagcggcgacgattacgaggccaagcagcagttcaagctgatgttcgagaaggcccggctgatcggcaagggcacaacagagcctcatccatttctgtacaaggtgttcgcccgcagcatccccgccaatgccgtcgagttctacgagcgctacctgatcgagcggaagttctacctgaccggcctgtccaacgagatcaagaaaggcaacagagtggatgtgcccttcatccggcgggaccagaacaagtggaaaacacccgccatgaagaccctgggcagaatctacagcgaggatctgcccgtggaactgcccagacagatgttcgacaatgagatcaagtcccacctgaagtccctgccacagatggaaggcatcgacttcaacaatgccaacgtgacctatctgatcgccgagtacatgaagagagtgctggacgacgacttccagaccttctaccagtggaaccgcaactaccggtacatggacatgcttaagggcgagtacgacagaaagggctccctgcagcactgcttcaccagcgtggaagagagagaaggcctctggaaagagcgggcctccagaacagagcggtacagaaagcaggccagcaacaagatccgcagcaaccggcagatgagaaacgccagcagcgaagagatcgagacaatcctggataagcggctgagcaacagccggaacgagtaccagaaaagcgagaaagtgatccggcgctacagagtgcaggatgccctgctgtttctgctggccaaaaagaccctgaccgaactggccgatttcgacggcgagaggttcaaactgaaagaaatcatgcccgacgccgagaagggaatcctgagcgagatcatgcccatgagcttcaccttcgagaaaggcggcaagaagtacaccatcaccagcgagggcatgaagctgaagaactacggcgacttctttgtgctggctagcgacaagaggatcggcaacctgctggaactcgtgggcagcgacatcgtgtccaaagaggatatcatggaagagttcaacaaatacgaccagtgcaggcccgagatcagctccatcgtgttcaacctggaaaagtgggccttcgacacataccccgagctgtctgccagagtggaccgggaagagaaggtggacttcaagagcatcctgaaaatcctgctgaacaacaagaacatcaacaaagagcagagcgacatcctgcggaagatccggaacgccttcgatcacaacaattaccccgacaaaggcgtggtggaaatcaaggccctgcctgagatcgccatgagcatcaagaaggcctttggggagtacgccatcatgaagggatcccttcaactgcctccacttgaaagactgacactgggtagttcctacccatacgatgttccagattacgcttatccctacgacgtgcctgattatgcatacccatatgatgtccccgactatgcctaa

SEQ ID NO: 24 - DNA, 858 bp, synthetic construct
  misc_feature 1..858: note = N286 Fragment polynucleotide sequence
  source 1..858: mol_type = other DNA
atgaacatccccgctctggtggaaaaccagaagaagtactttggcacctacagcgtgatggccatgctgaacgctcagaccgtgctggaccacatccagaaggtggccgatattgagggcgagcagaacgagaacaacgagaatctgtggtttcaccccgtgatgagccacctgtacaacgccaagaacggctacgacaagcagcccgagaaaaccatgttcatcatcgagcggctgcagagctacttcccattcctgaagatcatggccgagaaccagagagagtacagcaacggcaagtacaagcagaaccgcgtggaagtgaacagcaacgacatcttcgaggtgctgaagcgcgccttcggcgtgctgaagatgtacagggacctgaccaaccactacaagacctacgaggaaaagctgaacgacggctgcgagttcctgaccagcacagagcaacctctgagcggcatgatcaacaactactacacagtggccctgcggaacatgaacgagagatacggctacaagacagaggacctggccttcatccaggacaagcggttcaagttcgtgaaggacgcctacggcaagaaaaagtcccaagtgaataccggattcttcctgagcctgcaggactacaacggcgacacacagaagaagctgcacctgagcggagtgggaatcgccctgctgatctgcctgttcctggacaagcagtacatcaacatctttctgagcaggctgcccatcttctccagctacaatgcccagagcgaggaacggcggatcatcatcagatccttcggcatcaacagcatcaagctgcccaaggaccggatccacagcgagaagtcc

SEQ ID NO: 25 - DNA, 2544 bp, synthetic construct
  misc_feature 1..2544: note = C287 Fragment polynucleotide sequence
  source 1..2544: mol_type = other DNA
aacaagagcgtggccatggatatgctcaacgaagtgaagcggtgccccgacgagctgttcacaacactgtctgccgagaagcagtcccggttcagaatcatcagcgacgaccacaatgaagtgctgatgaagcggagcagcgacagattcgtgcctctgctgctgcagtatatcgattacggcaagctgttcgaccacatcaggttccacgtgaacatgggcaagctgagatacctgctgaaggccgacaagacctgcatcgacggccagaccagagtcagagtgatcgagcagcccctgaacggcttcggcagactggaagaggccgagacaatgcggaagcaagagaacggcaccttcggcaacagcggcatccggatcagagacttcgagaacatgaagcgggacgacgccaatcctgccaactatccctacatcgtggacacctacacacactacatcctggaaaacaacaaggtcgagatgtttatcaacgacaaagaggacagcgccccactgctgcccgtgatcgaggatgatagatacgtggtcaagacaatccccagctgccggatgagcaccctggaaattccagccatggccttccacatgtttctgttcggcagcaagaaaaccgagaagctgatcgtggacgtgcacaaccggtacaagagactgttccaggccatgcagaaagaagaagtgaccgccgagaatatcgccagcttcggaatcgccgagagcgacctgcctcagaagatcctggatctgatcagcggcaatgcccacggcaaggatgtggacgccttcatcagactgaccgtggacgacatgctgaccgacaccgagcggagaatcaagagattcaaggacgaccggaagtccattcggagcgccgacaacaagatgggaaagagaggcttcaagcagatctccacaggcaagctggccgacttcctggccaaggacatcgtgctgtttcagcccagcgtgaacgatggcgagaacaagatcaccggcctgaactaccggatcatgcagagcgccattgccgtgtacgatagcggcgacgattacgaggccaagcagcagttcaagctgatgttcgagaaggcccggctgatcggcaagggcacaacagagcctcatccatttctgtacaaggtgttcgcccgcagcatccccgccaatgccgtcgagttctacgagcgctacctgatcgagcggaagttctacctgaccggcctgtccaacgagatcaagaaaggcaacagagtggatgtgcccttcatccggcgggaccagaacaagtggaaaacacccgccatgaagaccctgggcagaatctacagcgaggatctgcccgtggaactgcccagacagatgttcgacaatgagatcaagtcccacctgaagtccctgccacagatggaaggcatcgacttcaacaatgccaacgtgacctatctgatcgccgagtacatgaagagagtgctggacgacgacttccagaccttctaccagtggaaccgcaactaccggtacatggacatgcttaagggcgagtacgacagaaagggctccctgcagcactgcttcaccagcgtggaagagagagaaggcctctggaaagagcgggcctccagaacagagcggtacagaaagcaggccagcaacaagatccgcagcaaccggcagatgagaaacgccagcagcgaagagatcgagacaatcctggataagcggctgagcaacagccggaacgagtaccagaaaagcgagaaagtgatccggcgctacagagtgcaggatgccctgctgtttctgctggccaaaaagaccctgaccgaactggccgatttcgacggcgagaggttcaaactgaaagaaatcatgcccgacgccgagaagggaatcctgagcgagatcatgcccatgagcttcaccttcgagaaaggcggcaagaagtacaccatcaccagcgagggcatgaagctgaagaactacggcgacttctttgtgctggctagcgacaagaggatcggcaacctgctggaactcgtgggcagcgacatcgtgtccaaagaggatatcatggaagagttcaacaaatacgaccagtgcaggcccgagatcagctccatcgtgttcaacctggaaaagtgggccttcgacacataccccgagctgtctgccagagtggaccgggaagagaaggtggacttcaagagcatcctgaaaatcctgctgaacaacaagaacatcaacaaagagcagagcgacatcctgcggaagatccggaacgccttcgatcacaacaattaccccgacaaaggcgtggtggaaatcaaggccctgcctgagatcgccatgagcatcaagaaggcctttggggagtacgccatcatgaagggatcccttcaactgcctccacttgaaagactgacactgggtagttcctacccatacgatgttccagattacgcttatccctacgacgtgcctgattatgcatacccatatgatgtccccgactatgcctaa

SEQ ID NO: 26 - DNA, 1053 bp, synthetic construct
  misc_feature 1..1053: note = N351 Fragment polynucleotide sequence
  source 1..1053: mol_type = other DNA
atgaacatccccgctctggtggaaaaccagaagaagtactttggcacctacagcgtgatggccatgctgaacgctcagaccgtgctggaccacatccagaaggtggccgatattgagggcgagcagaacgagaacaacgagaatctgtggtttcaccccgtgatgagccacctgtacaacgccaagaacggctacgacaagcagcccgagaaaaccatgttcatcatcgagcggctgcagagctacttcccattcctgaagatcatggccgagaaccagagagagtacagcaacggcaagtacaagcagaaccgcgtggaagtgaacagcaacgacatcttcgaggtgctgaagcgcgccttcggcgtgctgaagatgtacagggacctgaccaaccactacaagacctacgaggaaaagctgaacgacggctgcgagttcctgaccagcacagagcaacctctgagcggcatgatcaacaactactacacagtggccctgcggaacatgaacgagagatacggctacaagacagaggacctggccttcatccaggacaagcggttcaagttcgtgaaggacgcctacggcaagaaaaagtcccaagtgaataccggattcttcctgagcctgcaggactacaacggcgacacacagaagaagctgcacctgagcggagtgggaatcgccctgctgatctgcctgttcctggacaagcagtacatcaacatctttctgagcaggctgcccatcttctccagctacaatgcccagagcgaggaacggcggatcatcatcagatccttcggcatcaacagcatcaagctgcccaaggaccggatccacagcgagaagtccaacaagagcgtggccatggatatgctcaacgaagtgaagcggtgccccgacgagctgttcacaacactgtctgccgagaagcagtcccggttcagaatcatcagcgacgaccacaatgaagtgctgatgaagcggagcagcgacagattcgtgcctctgctgctgcagtatatcgattacggcaagctgttcgac

SEQ ID NO: 27 - DNA, 2349 bp, synthetic construct
  misc_feature 1..2349: note = C352 Fragment polynucleotide sequence
  source 1..2349: mol_type = other DNA
cacatcaggttccacgtgaacatgggcaagctgagatacctgctgaaggccgacaagacctgcatcgacggccagaccagagtcagagtgatcgagcagcccctgaacggcttcggcagactggaagaggccgagacaatgcggaagcaagagaacggcaccttcggcaacagcggcatccggatcagagacttcgagaacatgaagcgggacgacgccaatcctgccaactatccctacatcgtggacacctacacacactacatcctggaaaacaacaaggtcgagatgtttatcaacgacaaagaggacagcgccccactgctgcccgtgatcgaggatgatagatacgtggtcaagacaatccccagctgccggatgagcaccctggaaattccagccatggccttccacatgtttctgttcggcagcaagaaaaccgagaagctgatcgtggacgtgcacaaccggtacaagagactgttccaggccatgcagaaagaagaagtgaccgccgagaatatcgccagcttcggaatcgccgagagcgacctgcctcagaagatcctggatctgatcagcggcaatgcccacggcaaggatgtggacgccttcatcagactgaccgtggacgacatgctgaccgacaccgagcggagaatcaagagattcaaggacgaccggaagtccattcggagcgccgacaacaagatgggaaagagaggcttcaagcagatctccacaggcaagctggccgacttcctggccaaggacatcgtgctgtttcagcccagcgtgaacgatggcgagaacaagatcaccggcctgaactaccggatcatgcagagcgccattgccgtgtacgatagcggcgacgattacgaggccaagcagcagttcaagctgatgttcgagaaggcccggctgatcggcaagggcacaacagagcctcatccatttctgtacaaggtgttcgcccgcagcatccccgccaatgccgtcgagttctacgagcgctacctgatcgagcggaagttctacctgaccggcctgtccaacgagatcaagaaaggcaacagagtggatgtgcccttcatccggcgggaccagaacaagtggaaaacacccgccatgaagaccctgggcagaatctacagcgaggatctgcccgtggaactgcccagacagatgttcgacaatgagatcaagtcccacctgaagtccctgccacagatggaaggcatcgacttcaacaatgccaacgtgacctatctgatcgccgagtacatgaagagagtgctggacgacgacttccagaccttctaccagtggaaccgcaactaccggtacatggacatgcttaagggcgagtacgacagaaagggctccctgcagcactgcttcaccagcgtggaagagagagaaggcctctggaaagagcgggcctccagaacagagcggtacagaaagcaggccagcaacaagatccgcagcaaccggcagatgagaaacgccagcagcgaagagatcgagacaatcctggataagcggctgagcaacagccggaacgagtaccagaaaagcgagaaagtgatccggcgctacagagtgcaggatgccctgctgtttctgctggccaaaaagaccctgaccgaactggccgatttcgacggcgagaggttcaaactgaaagaaatcatgcccgacgccgagaagggaatcctgagcgagatcatgcccatgagcttcaccttcgagaaaggcggcaagaagtacaccatcaccagcgagggcatgaagctgaagaactacggcgacttctttgtgctggctagcgacaagaggatcggcaacctgctggaactcgtgggcagcgacatcgtgtccaaagaggatatcatggaagagttcaacaaatacgaccagtgcaggcccgagatcagctccatcgtgttcaacctggaaaagtgggccttcgacacataccccgagctgtctgccagagtggaccgggaagagaaggtggacttcaagagcatcctgaaaatcctgctgaacaacaagaacatcaacaaagagcagagcgacatcctgcggaagatccggaacgccttcgatcacaacaattaccccgacaaaggcgtggtggaaatcaaggccctgcctgagatcgccatgagcatcaagaaggcctttggggagtacgccatcatgaagggatcccttcaactgcctccacttgaaagactgacactgggtagttcctacccatacgatgttccagattacgcttatccctacgacgtgcctgattatgcatacccatatgatgtccccgactatgcctaa

SEQ ID NO: 28 - DNA, 1440 bp, synthetic construct
  misc_feature 1..1440: note = N480 Fragment polynucleotide sequence
  source 1..1440: mol_type = other DNA
atgaacatccccgctctggtggaaaaccagaagaagtactttggcacctacagcgtgatggccatgctgaacgctcagaccgtgctggaccacatccagaaggtggccgatattgagggcgagcagaacgagaacaacgagaatctgtggtttcaccccgtgatgagccacctgtacaacgccaagaacggctacgacaagcagcccgagaaaaccatgttcatcatcgagcggctgcagagctacttcccattcctgaagatcatggccgagaaccagagagagtacagcaacggcaagtacaagcagaaccgcgtggaagtgaacagcaacgacatcttcgaggtgctgaagcgcgccttcggcgtgctgaagatgtacagggacctgaccaaccactacaagacctacgaggaaaagctgaacgacggctgcgagttcctgaccagcacagagcaacctctgagcggcatgatcaacaactactacacagtggccctgcggaacatgaacgagagatacggctacaagacagaggacctggccttcatccaggacaagcggttcaagttcgtgaaggacgcctacggcaagaaaaagtcccaagtgaataccggattcttcctgagcctgcaggactacaacggcgacacacagaagaagctgcacctgagcggagtgggaatcgccctgctgatctgcctgttcctggacaagcagtacatcaacatctttctgagcaggctgcccatcttctccagctacaatgcccagagcgaggaacggcggatcatcatcagatccttcggcatcaacagcatcaagctgcccaaggaccggatccacagcgagaagtccaacaagagcgtggccatggatatgctcaacgaagtgaagcggtgccccgacgagctgttcacaacactgtctgccgagaagcagtcccggttcagaatcatcagcgacgaccacaatgaagtgctgatgaagcggagcagcgacagattcgtgcctctgctgctgcagtatatcgattacggcaagctgttcgaccacatcaggttccacgtgaacatgggcaagctgagatacctgctgaaggccgacaagacctgcatcgacggccagaccagagtcagagtgatcgagcagcccctgaacggcttcggcagactggaagaggccgagacaatgcggaagcaagagaacggcaccttcggcaacagcggcatccggatcagagacttcgagaacatgaagcgggacgacgccaatcctgccaactatccctacatcgtggacacctacacacactacatcctggaaaacaacaaggtcgagatgtttatcaacgacaaagaggacagcgccccactgctgcccgtgatcgaggatgatagatacgtggtcaagacaatccccagctgccggatgagcacc

SEQ ID NO: 29 - DNA, 1962 bp, synthetic construct
  misc_feature 1..1962: note = C481 Fragment polynucleotide sequence
  source 1..1962: mol_type = other DNA
ctggaaattccagccatggccttccacatgtttctgttcggcagcaagaaaaccgagaagctgatcgtggacgtgcacaaccggtacaagagactgttccaggccatgcagaaagaagaagtgaccgccgagaatatcgccagcttcggaatcgccgagagcgacctgcctcagaagatcctggatctgatcagcggcaatgcccacggcaaggatgtggacgccttcatcagactgaccgtggacgacatgctgaccgacaccgagcggagaatcaagagattcaaggacgaccggaagtccattcggagcgccgacaacaagatgggaaagagaggcttcaagcagatctccacaggcaagctggccgacttcctggccaaggacatcgtgctgtttcagcccagcgtgaacgatggcgagaacaagatcaccggcctgaactaccggatcatgcagagcgccattgccgtgtacgatagcggcgacgattacgaggccaagcagcagttcaagctgatgttcgagaaggcccggctgatcggcaagggcacaacagagcctcatccatttctgtacaaggtgttcgcccgcagcatccccgccaatgccgtcgagttctacgagcgctacctgatcgagcggaagttctacctgaccggcctgtccaacgagatcaagaaaggcaacagagtggatgtgcccttcatccggcgggaccagaacaagtggaaaacacccgccatgaagaccctgggcagaatctacagcgaggatctgcccgtggaactgcccagacagatgttcgacaatgagatcaagtcccacctgaagtccctgccacagatggaaggcatcgacttcaacaatgccaacgtgacctatctgatcgccgagtacatgaagagagtgctggacgacgacttccagaccttctaccagtggaaccgcaactaccggtacatggacatgcttaagggcgagtacgacagaaagggctccctgcagcactgcttcaccagcgtggaagagagagaaggcctctggaaagagcgggcctccagaacagagcggtacagaaagcaggccagcaacaagatccgcagcaaccggcagatgagaaacgccagcagcgaagagatcgagacaatcctggataagcggctgagcaacagccggaacgagtaccagaaaagcgagaaagtgatccggcgctacagagtgcaggatgccctgctgtttctgctggccaaaaagaccctgaccgaactggccgatttcgacggcgagaggttcaaactgaaagaaatcatgcccgacgccgagaagggaatcctgagcgagatcatgcccatgagcttcaccttcgagaaaggcggcaagaagtacaccatcaccagcgagggcatgaagctgaagaactacggcgacttctttgtgctggctagcgacaagaggatcggcaacctgctggaactcgtgggcagcgacatcgtgtccaaagaggatatcatggaagagttcaacaaatacgaccagtgcaggcccgagatcagctccatcgtgttcaacctggaaaagtgggccttcgacacataccccgagctgtctgccagagtggaccgggaagagaaggtggacttcaagagcatcctgaaaatcctgctgaacaacaagaacatcaacaaagagcagagcgacatcctgcggaagatccggaacgccttcgatcacaacaattaccccgacaaaggcgtggtggaaatcaaggccctgcctgagatcgccatgagcatcaagaaggcctttggggagtacgccatcatgaagggatcccttcaactgcctccacttgaaagactgacactgggtagttcctacccatacgatgttccagattacgcttatccctacgacgtgcctgattatgcatacccatatgatgtccccgactatgcctaa

SEQ ID NO: 30 - DNA, 1650 bp, synthetic construct
  misc_feature 1..1650: note = N550 Fragment polynucleotide sequence
  source 1..1650: mol_type = other DNA
atgaacatccccgctctggtggaaaaccagaagaagtactttggcacctacagcgtgatggccatgctgaacgctcagaccgtgctggaccacatccagaaggtggccgatattgagggcgagcagaacgagaacaacgagaatctgtggtttcaccccgtgatgagccacctgtacaacgccaagaacggctacgacaagcagcccgagaaaaccatgttcatcatcgagcggctgcagagctacttcccattcctgaagatcatggccgagaaccagagagagtacagcaacggcaagtacaagcagaaccgcgtggaagtgaacagcaacgacatcttcgaggtgctgaagcgcgccttcggcgtgctgaagatgtacagggacctgaccaaccactacaagacctacgaggaaaagctgaacgacggctgcgagttcctgaccagcacagagcaacctctgagcggcatgatcaacaactactacacagtggccctgcggaacatgaacgagagatacggctacaagacagaggacctggccttcatccaggacaagcggttcaagttcgtgaaggacgcctacggcaagaaaaagtcccaagtgaataccggattcttcctgagcctgcaggactacaacggcgacacacagaagaagctgcacctgagcggagtgggaatcgccctgctgatctgcctgttcctggacaagcagtacatcaacatctttctgagcaggctgcccatcttctccagctacaatgcccagagcgaggaacggcggatcatcatcagatccttcggcatcaacagcatcaagctgcccaaggaccggatccacagcgagaagtccaacaagagcgtggccatggatatgctcaacgaagtgaagcggtgccccgacgagctgttcacaacactgtctgccgagaagcagtcccggttcagaatcatcagcgacgaccacaatgaagtgctgatgaagcggagcagcgacagattcgtgcctctgctgctgcagtatatcgattacggcaagctgttcgaccacatcaggttccacgtgaacatgggcaagctgagatacctgctgaaggccgacaagacctgcatcgacggccagaccagagtcagagtgatcgagcagcccctgaacggcttcggcagactggaagaggccgagacaatgcggaagcaagagaacggcaccttcggcaacagcggcatccggatcagagacttcgagaacatgaagcgggacgacgccaatcctgccaactatccctacatcgtggacacctacacacactacatcctggaaaacaacaaggtcgagatgtttatcaacgacaaagaggacagcgccccactgctgcccgtgatcgaggatgatagatacgtggtcaagacaatccccagctgccggatgagcaccctggaaattccagccatggccttccacatgtttctgttcggcagcaagaaaaccgagaagctgatcgtggacgtgcacaaccggtacaagagactgttccaggccatgcagaaagaagaagtgaccgccgagaatatcgccagcttcggaatcgccgagagcgacctgcctcagaagatcctggatctgatcagcggcaatgcccacggc

SEQ ID NO: 31 - DNA, 1752 bp, synthetic construct
  misc_feature 1..1752: note = C551 Fragment polynucleotide sequence
  source 1..1752: mol_type = other DNA
aaggatgtggacgccttcatcagactgaccgtggacgacatgctgaccgacaccgagcggagaatcaagagattcaaggacgaccggaagtccattcggagcgccgacaacaagatgggaaagagaggcttcaagcagatctccacaggcaagctggccgacttcctggccaaggacatcgtgctgtttcagcccagcgtgaacgatggcgagaacaagatcaccggcctgaactaccggatcatgcagagcgccattgccgtgtacgatagcggcgacgattacgaggccaagcagcagttcaagctgatgttcgagaaggcccggctgatcggcaagggcacaacagagcctcatccatttctgtacaaggtgttcgcccgcagcatccccgccaatgccgtcgagttctacgagcgctacctgatcgagcggaagttctacctgaccggcctgtccaacgagatcaagaaaggcaacagagtggatgtgcccttcatccggcgggaccagaacaagtggaaaacacccgccatgaagaccctgggcagaatctacagcgaggatctgcccgtggaactgcccagacagatgttcgacaatgagatcaagtcccacctgaagtccctgccacagatggaaggcatcgacttcaacaatgccaacgtgacctatctgatcgccgagtacatgaagagagtgctggacgacgacttccagaccttctaccagtggaaccgcaactaccggtacatggacatgcttaagggcgagtacgacagaaagggctccctgcagcactgcttcaccagcgtggaagagagagaaggcctctggaaagagcgggcctccagaacagagcggtacagaaagcaggccagcaacaagatccgcagcaaccggcagatgagaaacgccagcagcgaagagatcgagacaatcctggataagcggctgagcaacagccggaacgagtaccagaaaagcgagaaagtgatccggcgctacagagtgcaggatgccctgctgtttctgctggccaaaaagaccctgaccgaactggccgatttcgacggcgagaggttcaaactgaaagaaatcatgcccgacgccgagaagggaatcctgagcgagatcatgcccatgagcttcaccttcgagaaaggcggcaagaagtacaccatcaccagcgagggcatgaagctgaagaactacggcgacttctttgtgctggctagcgacaagaggatcggcaacctgctggaactcgtgggcagcgacatcgtgtccaaagaggatatcatggaagagttcaacaaatacgaccagtgcaggcccgagatcagctccatcgtgttcaacctggaaaagtgggccttcgacacataccccgagctgtctgccagagtggaccgggaagagaaggtggacttcaagagcatcctgaaaatcctgctgaacaacaagaacatcaacaaagagcagagcgacatcctgcggaagatccggaacgccttcgatcacaacaattaccccgacaaaggcgtggtggaaatcaaggccctgcctgagatcgccatgagcatcaagaaggcctttggggagtacgccatcatgaagggatcccttcaactgcctccacttgaaagactgacactgggtagttcctacccatacgatgttccagattacgcttatccctacgacgtgcctgattatgcatacccatatgatgtccccgactatgcctaa

SEQ ID NO: 32 - DNA, 1872 bp, synthetic construct
  misc_feature 1..1872: note = N624 Fragment polynucleotide sequence
  source 1..1872: mol_type = other DNA
atgaacatccccgctctggtggaaaaccagaagaagtactttggcacctacagcgtgatggccatgctgaacgctcagaccgtgctggaccacatccagaaggtggccgatattgagggcgagcagaacgagaacaacgagaatctgtggtttcaccccgtgatgagccacctgtacaacgccaagaacggctacgacaagcagcccgagaaaaccatgttcatcatcgagcggctgcagagctacttcccattcctgaagatcatggccgagaaccagagagagtacagcaacggcaagtacaagcagaaccgcgtggaagtgaacagcaacgacatcttcgaggtgctgaagcgcgccttcggcgtgctgaagatgtacagggacctgaccaaccactacaagacctacgaggaaaagctgaacgacggctgcgagttcctgaccagcacagagcaacctctgagcggcatgatcaacaactactacacagtggccctgcggaacatgaacgagagatacggctacaagacagaggacctggccttcatccaggacaagcggttcaagttcgtgaaggacgcctacggcaagaaaaagtcccaagtgaataccggattcttcctgagcctgcaggactacaacggcgacacacagaagaagctgcacctgagcggagtgggaatcgccctgctgatctgcctgttcctggacaagcagtacatcaacatctttctgagcaggctgcccatcttctccagctacaatgcccagagcgaggaacggcggatcatcatcagatccttcggcatcaacagcatcaagctgcccaaggaccggatccacagcgagaagtccaacaagagcgtggccatggatatgctcaacgaagtgaagcggtgccccgacgagctgttcacaacactgtctgccgagaagcagtcccggttcagaatcatcagcgacgaccacaatgaagtgctgatgaagcggagcagcgacagattcgtgcctctgctgctgcagtatatcgattacggcaagctgttcgaccacatcaggttccacgtgaacatgggcaagctgagatacctgctgaaggccgacaagacctgcatcgacggccagaccagagtcagagtgatcgagcagcccctgaacggcttcggcagactggaagaggccgagacaatgcggaagcaagagaacggcaccttcggcaacagcggcatccggatcagagacttcgagaacatgaagcgggacgacgccaatcctgccaactatccctacatcgtggacacctacacacactacatcctggaaaacaacaaggtcgagatgtttatcaacgacaaagaggacagcgccccactgctgcccgtgatcgaggatgatagatacgtggtcaagacaatccccagctgccggatgagcaccctggaaattccagccatggccttccacatgtttctgttcggcagcaagaaaaccgagaagctgatcgtggacgtgcacaaccggtacaagagactgttccaggccatgcagaaagaagaagtgaccgccgagaatatcgccagcttcggaatcgccgagagcgacctgcctcagaagatcctggatctgatcagcggcaatgcccacggcaaggatgtggacgccttcatcagactgaccgtggacgacatgctgaccgacaccgagcggagaatcaagagattcaaggacgaccggaagtccattcggagcgccgacaacaagatgggaaagagaggcttcaagcagatctccacaggcaagctggccgacttcctggccaaggacatcgtgctgtttcagcccagcgtgaacgatggcgagaacaagatc

SEQ ID NO: 33 - DNA, 1530 bp, synthetic construct
  misc_feature 1..1530: note = C625 Fragment polynucleotide sequence
  source 1..1530: mol_type = other DNA
accggcctgaactaccggatcatgcagagcgccattgccgtgtacgatagcggcgacgattacgaggccaagcagcagttcaagctgatgttcgagaaggcccggctgatcggcaagggcacaacagagcctcatccatttctgtacaaggtgttcgcccgcagcatccccgccaatgccgtcgagttctacgagcgctacctgatcgagcggaagttctacctgaccggcctgtccaacgagatcaagaaaggcaacagagtggatgtgcccttcatccggcgggaccagaacaagtggaaaacacccgccatgaagaccctgggcagaatctacagcgaggatctgcccgtggaactgcccagacagatgttcgacaatgagatcaagtcccacctgaagtccctgccacagatggaaggcatcgacttcaacaatgccaacgtgacctatctgatcgccgagtacatgaagagagtgctggacgacgacttccagaccttctaccagtggaaccgcaactaccggtacatggacatgcttaagggcgagtacgacagaaagggctccctgcagcactgcttcaccagcgtggaagagagagaaggcctctggaaagagcgggcctccagaacagagcggtacagaaagcaggccagcaacaagatccgcagcaaccggcagatgagaaacgccagcagcgaagagatcgagacaatcctggataagcggctgagcaacagccggaacgagtaccagaaaagcgagaaagtgatccggcgctacagagtgcaggatgccctgctgtttctgctggccaaaaagaccctgaccgaactggccgatttcgacggcgagaggttcaaactgaaagaaatcatgcccgacgccgagaagggaatcctgagcgagatcatgcccatgagcttcaccttcgagaaaggcggcaagaagtacaccatcaccagcgagggcatgaagctgaagaactacggcgacttctttgtgctggctagcgacaagaggatcggcaacctgctggaactcgtgggcagcgacatcgtgtccaaagaggatatcatggaagagttcaacaaatacgaccagtgcaggcccgagatcagctccatcgtgttcaacctggaaaagtgggccttcgacacataccccgagctgtctgccagagtggaccgggaagagaaggtggacttcaagagcatcctgaaaatcctgctgaacaacaagaacatcaacaaagagcagagcgacatcctgcggaagatccggaacgccttcgatcacaacaattaccccgacaaaggcgtggtggaaatcaaggccctgcctgagatcgccatgagcatcaagaaggcctttggggagtacgccatcatgaagggatcccttcaactgcctccacttgaaagactgacactgggtagttcctacccatacgatgttccagattacgcttatccctacgacgtgcctgattatgcatacccatatgatgtccccgactatgcctaa

SEQ ID NO: 34 - DNA, 2175 bp, synthetic construct
  misc_feature 1..2175: note = N725 Fragment polynucleotide sequence
  source 1..2175: mol_type = other DNA
atgaacatccccgctctggtggaaaaccagaagaagtactttggcacctacagcgtgatggccatgctgaacgctcagaccgtgctggaccacatccagaaggtggccgatattgagggcgagcagaacgagaacaacgagaatctgtggtttcaccccgtgatgagccacctgtacaacgccaagaacggctacgacaagcagcccgagaaaaccatgttcatcatcgagcggctgcagagctacttcccattcctgaagatcatggccgagaaccagagagagtacagcaacggcaagtacaagcagaaccgcgtggaagtgaacagcaacgacatcttcgaggtgctgaagcgcgccttcggcgtgctgaagatgtacagggacctgaccaaccactacaagacctacgaggaaaagctgaacgacggctgcgagttcctgaccagcacagagcaacctctgagcggcatgatcaacaactactacacagtggccctgcggaacatgaacgagagatacggctacaagacagaggacctggccttcatccaggacaagcggttcaagttcgtgaaggacgcctacggcaagaaaaagtcccaagtgaataccggattcttcctgagcctgcaggactacaacggcgacacacagaagaagctgcacctgagcggagtgggaatcgccctgctgatctgcctgttcctggacaagcagtacatcaacatctttctgagcaggctgcccatcttctccagctacaatgcccagagcgaggaacggcggatcatcatcagatccttcggcatcaacagcatcaagctgcccaaggaccggatccacagcgagaagtccaacaagagcgtggccatggatatgctcaacgaagtgaagcggtgccccgacgagctgttcacaacactgtctgccgagaagcagtcccggttcagaatcatcagcgacgaccacaatgaagtgctgatgaagcggagcagcgacagattcgtgcctctgctgctgcagtatatcgattacggcaagctgttcgaccacatcaggttccacgtgaacatgggcaagctgagatacctgctgaaggccgacaagacctgcatcgacggccagaccagagtcagagtgatcgagcagcccctgaacggcttcggcagactggaagaggccgagacaatgcggaagcaagagaacggcaccttcggcaacagcggcatccggatcagagacttcgagaacatgaagcgggacgacgccaatcctgccaactatccctacatcgtggacacctacacacactacatcctggaaaacaacaaggtcgagatgtttatcaacgacaaagaggacagcgccccactgctgcccgtgatcgaggatgatagatacgtggtcaagacaatccccagctgccggatgagcaccctggaaattccagccatggccttccacatgtttctgttcggcagcaagaaaaccgagaagctgatcgtggacgtgcacaaccggtacaagagactgttccaggccatgcagaaagaagaagtgaccgccgagaatatcgccagcttcggaatcgccgagagcgacctgcctcagaagatcctggatctgatcagcggcaatgcccacggcaaggatgtggacgccttcatcagactgaccgtggacgacatgctgaccgacaccgagcggagaatcaagagattcaaggacgaccggaagtccattcggagcgccgacaacaagatgggaaagagaggcttcaagcagatctccacaggcaagctggccgacttcctggccaaggacatcgtgctgtttcagcccagcgtgaacgatggcgagaacaagatcaccggcctgaactaccggatcatgcagagcgccattgccgtgtacgatagcggcgacgattacgaggccaagcagcagttcaagctgatgttcgagaaggcccggctgatcggcaagggcacaacagagcctcatccatttctgtacaaggtgttcgcccgcagcatccccgccaatgccgtcgagttctacgagcgctacctgatcgagcggaagttctacctgaccggcctgtccaacgagatcaagaaaggcaacagagtggatgtgcccttcatccggcgggaccagaacaagtggaaa

SEQ ID NO: 35 - DNA, 1227 bp, synthetic construct
  misc_feature 1..1227: note = C726 Fragment polynucleotide sequence
  source 1..1227: mol_type = other DNA
acacccgccatgaagaccctgggcagaatctacagcgaggatctgcccgtggaactgcccagacagatgttcgacaatgagatcaagtcccacctgaagtccctgccacagatggaaggcatcgacttcaacaatgccaacgtgacctatctgatcgccgagtacatgaagagagtgctggacgacgacttccagaccttctaccagtggaaccgcaactaccggtacatggacatgcttaagggcgagtacgacagaaagggctccctgcagcactgcttcaccagcgtggaagagagagaaggcctctggaaagagcgggcctccagaacagagcggtacagaaagcaggccagcaacaagatccgcagcaaccggcagatgagaaacgccagcagcgaagagatcgagacaatcctggataagcggctgagcaacagccggaacgagtaccagaaaagcgagaaagtgatccggcgctacagagtgcaggatgccctgctgtttctgctggccaaaaagaccctgaccgaactggccgatttcgacggcgagaggttcaaactgaaagaaatcatgcccgacgccgagaagggaatcctgagcgagatcatgcccatgagcttcaccttcgagaaaggcggcaagaagtacaccatcaccagcgagggcatgaagctgaagaactacggcgacttctttgtgctggctagcgacaagaggatcggcaacctgctggaactcgtgggcagcgacatcgtgtccaaagaggatatcatggaagagttcaacaaatacgaccagtgcaggcccgagatcagctccatcgtgttcaacctggaaaagtgggccttcgacacataccccgagctgtctgccagagtggaccgggaagagaaggtggacttcaagagcatcctgaaaatcctgctgaacaacaagaacatcaacaaagagcagagcgacatcctgcggaagatccggaacgccttcgatcacaacaattaccccgacaaaggcgtggtggaaatcaaggccctgcctgagatcgccatgagcatcaagaaggcctttggggagtacgccatcatgaagggatcccttcaactgcctccacttgaaagactgacactgggtagttcctacccatacgatgttccagattacgcttatccctacgacgtgcctgattatgcatacccatatgatgtccccgactatgcctaa

SEQ ID NO: 36 - DNA, 2784 bp, synthetic construct
  misc_feature 1..2784: note = N928 Fragment polynucleotide sequence
  source 1..2784: mol_type = other DNA
atgaacatccccgctctggtggaaaaccagaagaagtactttggcacctacagcgtgatggccatgctgaacgctcagaccgtgctggaccacatccagaaggtggccgatattgagggcgagcagaacgagaacaacgagaatctgtggtttcaccccgtgatgagccacctgtacaacgccaagaacggctacgacaagcagcccgagaaaaccatgttcatcatcgagcggctgcagagctacttcccattcctgaagatcatggccgagaaccagagagagtacagcaacggcaagtacaagcagaaccgcgtggaagtgaacagcaacgacatcttcgaggtgctgaagcgcgccttcggcgtgctgaagatgtacagggacctgaccaaccactacaagacctacgaggaaaagctgaacgacggctgcgagttcctgaccagcacagagcaacctctgagcggcatgatcaacaactactacacagtggccctgcggaacatgaacgagagatacggctacaagacagaggacctggccttcatccaggacaagcggttcaagttcgtgaaggacgcctacggcaagaaaaagtcccaagtgaataccggattcttcctgagcctgcaggactacaacggcgacacacagaagaagctgcacctgagcggagtgggaatcgccctgctgatctgcctgttcctggacaagcagtacatcaacatctttctgagcaggctgcccatcttctccagctacaatgcccagagcgaggaacggcggatcatcatcagatccttcggcatcaacagcatcaagctgcccaaggaccggatccacagcgagaagtccaacaagagcgtggccatggatatgctcaacgaagtgaagcggtgccccgacgagctgttcacaacactgtctgccgagaagcagtcccggttcagaatcatcagcgacgaccacaatgaagtgctgatgaagcggagcagcgacagattcgtgcctctgctgctgcagtatatcgattacggcaagctgttcgaccacatcaggttccacgtgaacatgggcaagctgagatacctgctgaaggccgacaagacctgcatcgacggccagaccagagtcagagtgatcgagcagcccctgaacggcttcggcagactggaagaggccgagacaatgcggaagcaagagaacggcaccttcggcaacagcggcatccggatcagagacttcgagaacatgaagcgggacgacgccaatcctgccaactatccctacatcgtggacacctacacacactacatcctggaaaacaacaaggtcgagatgtttatcaacgacaaagaggacagcgccccactgctgcccgtgatcgaggatgatagatacgtggtcaagacaatccccagctgccggatgagcaccctggaaattccagccatggccttccacatgtttctgttcggcagcaagaaaaccgagaagctgatcgtggacgtgcacaaccggtacaagagactgttccaggccatgcagaaagaagaagtgaccgccgagaatatcgccagcttcggaatcgccgagagcgacctgcctcagaagatcctggatctgatcagcggcaatgcccacggcaaggatgtggacgccttcatcagactgaccgtggacgacatgctgaccgacaccgagcggagaatcaagagattcaaggacgaccggaagtccattcggagcgccgacaacaagatgggaaagagaggcttcaagcagatctccacaggcaagctggccgacttcctggccaaggacatcgtgctgtttcagcccagcgtgaacgatggcgagaacaagatcaccggcctgaactaccggatcatgcagagcgccattgccgtgtacgatagcggcgacgattacgaggccaagcagcagttcaagctgatgttcgagaaggcccggctgatcggcaagggcacaacagagcctcatccatttctgtacaaggtgttcgcccgcagcatccccgccaatgccgtcgagttctacgagcgctacctgatcgagcggaagttctacctgaccggcctgtccaacgagatcaagaaaggcaacagagtggatgtgcccttcatccggcgggaccagaacaagtggaaaacacccgccatgaagaccctgggcagaatctacagcgaggatctgcccgtggaactgcccagacagatgttcgacaatgagatcaagtcccacctgaagtccctgccacagatggaaggcatcgacttcaacaatgccaacgtgacctatctgatcgccgagtacatgaagagagtgctggacgacgacttccagaccttctaccagtggaaccgcaactaccggtacatggacatgcttaagggcgagtacgacagaaagggctccctgcagcactgcttcaccagcgtggaagagagagaaggcctctggaaagagcgggcctccagaacagagcggtacagaaagcaggccagcaacaagatccgcagcaaccggcagatgagaaacgccagcagcgaagagatcgagacaatcctggataagcggctgagcaacagccggaacgagtaccagaaaagcgagaaagtgatccggcgctacagagtgcaggatgccctgctgtttctgctggccaaaaagaccctgaccgaactggccgatttcgacggcgagaggttcaaactgaaagaaatcatgcccgacgccgagaagggaatcctgagcgag

SEQ ID NO: 37 - DNA, 618 bp, synthetic construct
  misc_feature 1..618: note = C929 Fragment polynucleotide sequence
  source 1..618: mol_type = other DNA
atcatgcccatgagcttcaccttcgagaaaggcggcaagaagtacaccatcaccagcgagggcatgaagctgaagaactacggcgacttctttgtgctggctagcgacaagaggatcggcaacctgctggaactcgtgggcagcgacatcgtgtccaaagaggatatcatggaagagttcaacaaatacgaccagtgcaggcccgagatcagctccatcgtgttcaacctggaaaagtgggccttcgacacataccccgagctgtctgccagagtggaccgggaagagaaggtggacttcaagagcatcctgaaaatcctgctgaacaacaagaacatcaacaaagagcagagcgacatcctgcggaagatccggaacgccttcgatcacaacaattaccccgacaaaggcgtggtggaaatcaaggccctgcctgagatcgccatgagcatcaagaaggcctttggggagtacgccatcatgaagggatcccttcaactgcctccacttgaaagactgacactgggtagttcctacccatacgatgttccagattacgcttatccctacgacgtgcctgattatgcatacccatatgatgtccccgactatgcctaa

SEQ ID NO: 38 - DNA, 279 bp, synthetic construct
  misc_feature 1..279: note = FRB polynucleotide sequence
  source 1..279: mol_type = other DNA
atcctctggcatgagatgtggcatgaaggcctggaagaggcatctcgtttgtactttggggaaaggaacgtgaaaggcatgtttgaggtgctggagcccttgcatgctatgatggaacggggcccccagactctgaaggaaacatcctttaatcaggcctatggtcgagatttaatggaggcccaagagtggtgcaggaagtacatgaaatcagggaatgtcaaggacctcacccaagcctgggacctctattatcatgtgttccgacgaatctcaaag

SEQ ID NO: 39 - DNA, 321 bp, synthetic construct
  misc_feature 1..321: note = FKBP polynucleotide sequence
  source 1..321: mol_type = other DNA
ggagtgcaggtggaaaccatctccccaggagacgggcgcaccttccccaagcgcggccagacctgcgtggtgcactacaccgggatgcttgaagatggaaagaaatttgattcctcccgggacagaaacaagccctttaagtttatgctaggcaagcaggaggtgatccgaggctgggaagaaggggttgcccagatgagtgtgggtcagagagccaaactgactatatctccagattatgcctatggtgccactgggcacccaggcatcatcccaccacatgccactctcgtcttcgatgtggagcttctaaaactggaa

SEQ ID NO: 40 - DNA, 450 bp, synthetic construct
  misc_feature 1..450: note = nMag polynucleotide sequence
  source 1..450: mol_type = other DNA
cacaccctgtacgcccccggcggctacgacatcatgggctacctggaccagatcggcaacagacccaacccccaggtggagctgggccccgtggacaccagctgcgccctgatcctgtgcgacctgaagcagaaggacacccccatcgtgtacgccagcgaggccttcctgtatatgaccggctacagcaacgccgaggtgctgggcagaaactgcagattcctgcagagccccgacggcatggtgaagcccaagagcaccagaaagtacgtggacagcaacaccatcaacaccatgagaaaggccatcgacagaaacgccgaggtgcaggtggaggtggtgaacttcaagaagaacggccagagattcgtgaacttcctgaccatgatccccgtgagagacgagaccggcgagtacagatacagcatgggcttccagtgcgagaccgag

SEQ ID NO: 41 - DNA, 450 bp, synthetic construct
  misc_feature 1..450: note = pMag polynucleotide sequence
  source 1..450: mol_type = other DNA
cacaccctgtacgcccccggcggctacgacatcatgggctacctgagacagatcagaaacagacccaacccccaggtggagctgggccccgtggacaccagctgcgccctgatcctgtgcgacctgaagcagaaggacacccccatcgtgtacgccagcgaggccttcctgtatatgaccggctacagcaacgccgaggtgctgggcagaaactgcagattcctgcagagccccgacggcatggtgaagcccaagagcaccagaaagtacgtggacagcaacaccatcaacaccatcagaaaggccatcgacagaaacgccgaggtgcaggtggaggtggtgaacttcaagaagaacggccagagattcgtgaacttcctgaccatcatccccgtgagagacgagaccggcgagtacagatacagcatgggcttccagtgcgagaccgag

SEQ ID NO: 42 - DNA, 1206 bp, synthetic construct
  misc_feature 1..1206: note = N272-GS16-FRB-GS16 polynucleotide sequence
  source 1..1206: mol_type = other DNA
atgaacatccccgctctggtggaaaaccagaagaagtactttggcacctacagcgtgatggccatgctgaacgctcagaccgtgctggaccacatccagaaggtggccgatattgagggcgagcagaacgagaacaacgagaatctgtggtttcaccccgtgatgagccacctgtacaacgccaagaacggctacgacaagcagcccgagaaaaccatgttcatcatcgagcggctgcagagctacttcccattcctgaagatcatggccgagaaccagagagagtacagcaacggcaagtacaagcagaaccgcgtggaagtgaacagcaacgacatcttcgaggtgctgaagcgcgccttcggcgtgctgaagatgtacagggacctgaccaaccactacaagacctacgaggaaaagctgaacgacggctgcgagttcctgaccagcacagagcaacctctgagcggcatgatcaacaactactacacagtggccctgcggaacatgaacgagagatacggctacaagacagaggacctggccttcatccaggacaagcggttcaagttcgtgaaggacgcctacggcaagaaaaagtcccaagtgaataccggattcttcctgagcctgcaggactacaacggcgacacacagaagaagctgcacctgagcggagtgggaatcgccctgctgatctgcctgttcctggacaagcagtacatcaacatctttctgagcaggctgcccatcttctccagctacaatgcccagagcgaggaacggcggatcatcatcagatccttcggcatcaacaacccgggatccggaggaagtggcagctctggcggcagtggagggtctggtggcagcggaatcctctggcatgagatgtggcatgaaggcctggaagaggcatctcgtttgtactttggggaaaggaacgtgaaaggcatgtttgaggtgctggagcccttgcatgctatgatggaacggggcccccagactctgaaggaaacatcctttaatcaggcctatggtcgagatttaatggaggcccaagagtggtgcaggaagtacatgaaatcagggaatgtcaaggacctcacccaagcctgggacctctattatcatgtgttccgacgaatctcaaagggaggaagcggcggttccggggggggatccggaagtggttccggggggtag

SEQ ID NO: 43 - DNA, 3012 bp, synthetic construct
  misc_feature 1..3012: note = GS16-FKBP-GS16-C273 polynucleotide sequence
  source 1..3012: mol_type = other DNA
atgggaggaagtggcagctctggcggcagtggagggtctggtggcagcggaggagtgcaggtggaaaccatctccccaggagacgggcgcaccttccccaagcgcggccagacctgcgtggtgcactacaccgggatgcttgaagatggaaagaaatttgattcctcccgggacagaaacaagccctttaagtttatgctaggcaagcaggaggtgatccgaggctgggaagaaggggttgcccagatgagtgtgggtcagagagccaaactgactatatctccagattatgcctatggtgccactgggcacccaggcatcatcccaccacatgccactctcgtcttcgatgtggagcttctaaaactggaaggaggaagcggcggttccggggggggatccggaagtggttccggggggtgtacaagcatcaagctgcccaaggaccggatccacagcgagaagtccaacaagagcgtggccatggatatgctcaacgaagtgaagcggtgccccgacgagctgttcacaacactgtctgccgagaagcagtcccggttcagaatcatcagcgacgaccacaatgaagtgctgatgaagcggagcagcgacagattcgtgcctctgctgctgcagtatatcgattacggcaagctgttcgaccacatcaggttccacgtgaacatgggcaagctgagatacctgctgaaggccgacaagacctgcatcgacggccagaccagagtcagagtgatcgagcagcccctgaacggcttcggcagactggaagaggccgagacaatgcggaagcaagagaacggcaccttcggcaacagcggcatccggatcagagacttcgagaacatgaagcgggacgacgccaatcctgccaactatccctacatcgtggacacctacacacactacatcctggaaaacaacaaggtcgagatgtttatcaacgacaaagaggacagcgccccactgctgcccgtgatcgaggatgatagatacgtggtcaagacaatccccagctgccggatgagcaccctggaaattccagccatggccttccacatgtttctgttcggcagcaagaaaaccgagaagctgatcgtggacgtgcacaaccggtacaagagactgttccaggccatgcagaaagaagaagtgaccgccgagaatatcgccagcttcggaatcgccgagagcgacctgcctcagaagatcctggatctgatcagcggcaatgcccacggcaaggatgtggacgccttcatcagactgaccgtggacgacatgctgaccgacaccgagcggagaatcaagagattcaaggacgaccggaagtccattcggagcgccgacaacaagatgggaaagagaggcttcaagcagatctccacaggcaagctggccgacttcctggccaaggacatcgtgctgtttcagcccagcgtgaacgatggcgagaacaagatcaccggcctgaactaccggatcatgcagagcgccattgccgtgtacgatagcggcgacgattacgaggccaagcagcagttcaagctgatgttcgagaaggcccggctgatcggcaagggcacaacagagcctcatccatttctgtacaaggtgttcgcccgcagcatccccgccaatgccgtcgagttctacgagcgctacctgatcgagcggaagttctacctgaccggcctgtccaacgagatcaagaaaggcaacagagtggatgtgcccttcatccggcgggaccagaacaagtggaaaacacccgccatgaagaccctgggcagaatctacagcgaggatctgcccgtggaactgcccagacagatgttcgacaatgagatcaagtcccacctgaagtccctgccacagatggaaggcatcgacttcaacaatgccaacgtgacctatctgatcgccgagtacatgaagagagtgctggacgacgacttccagaccttctaccagtggaaccgcaactaccggtacatggacatgcttaagggcgagtacgacagaaagggctccctgcagcactgcttcaccagcgtggaagagagagaaggcctctggaaagagcgggcctccagaacagagcggtacagaaagcaggccagcaacaagatccgcagcaaccggcagatgagaaacgccagcagcgaagagatcgagacaatcctggataagcggctgagcaacagccggaacgagtaccagaaaagcgagaaagtgatccggcgctacagagtgcaggatgccctgctgtttctgctggccaaaaagaccctgaccgaactggccgatttcgacggcgagaggttcaaactgaaagaaatcatgcccgacgccgagaagggaatcctgagcgagatcatgcccatgagcttcaccttcgagaaaggcggcaagaagtacaccatcaccagcgagggcatgaagctgaagaactacggcgacttctttgtgctggctagcgacaagaggatcggcaacctgctggaactcgtgggcagcgacatcgtgtccaaagaggatatcatggaagagttcaacaaatacgaccagtgcaggcccgagatcagctccatcgtgttcaacctggaaaagtgggccttcgacacataccccgagctgtctgccagagtggaccgggaagagaaggtggacttcaagagcatcctgaaaatcctgctgaacaacaagaacatcaacaaagagcagagcgacatcctgcggaagatccggaacgccttcgatcacaacaattaccccgacaaaggcgtggtggaaatcaaggccctgcctgagatcgccatgagcatcaagaaggcctttggggagtacgccatcatgaagggatcccttcaactgcctccacttgaaagactgacactgggtagttcctacccatacgatgttccagattacgcttatccctacgacgtgcctgattatgcatacccatatgatgtccccgactatgcctaa

SEQ ID NO: 44 - DNA, 1248 bp, synthetic construct
  misc_feature 1..1248: note = N286-GS16-FRB-GS16 polynucleotide sequence
  source 1..1248: mol_type = other DNA
atgaacatccccgctctggtggaaaaccagaagaagtactttggcacctacagcgtgatggccatgctgaacgctcagaccgtgctggaccacatccagaaggtggccgatattgagggcgagcagaacgagaacaacgagaatctgtggtttcaccccgtgatgagccacctgtacaacgccaagaacggctacgacaagcagcccgagaaaaccatgttcatcatcgagcggctgcagagctacttcccattcctgaagatcatggccgagaaccagagagagtacagcaacggcaagtacaagcagaaccgcgtggaagtgaacagcaacgacatcttcgaggtgctgaagcgcgccttcggcgtgctgaagatgtacagggacctgaccaaccactacaagacctacgaggaaaagctgaacgacggctgcgagttcctgaccagcacagagcaacctctgagcggcatgatcaacaactactacacagtggccctgcggaacatgaacgagagatacggctacaagacagaggacctggccttcatccaggacaagcggttcaagttcgtgaaggacgcctacggcaagaaaaagtcccaagtgaataccggattcttcctgagcctgcaggactacaacggcgacacacagaagaagctgcacctgagcggagtgggaatcgccctgctgatctgcctgttcctggacaagcagtacatcaacatctttctgagcaggctgcccatcttctccagctacaatgcccagagcgaggaacggcggatcatcatcagatccttcggcatcaacagcatcaagctgcccaaggaccggatccacagcgagaagtccaacccgggatccggaggaagtggcagctctggcggcagtggagggtctggtggcagcggaatcctctggcatgagatgtggcatgaaggcctggaagaggcatctcgtttgtactttggggaaaggaacgtgaaaggcatgtttgaggtgctggagcccttgcatgctatgatggaacggggcccccagactctgaaggaaacatcctttaatcaggcctatggtcgagatttaatggaggcccaagagtggtgcaggaagtacatgaaatcagggaatgtcaaggacctcacccaagcctgggacctctattatcatgtgttccgacgaatctcaaagggaggaagcggcggttccggggggggatccggaagtggttccggggggtag

SEQ ID NO: 45 - DNA, 2970 bp, synthetic construct
  misc_feature 1..2970: note = GS16-FKBP-GS16-C287 polynucleotide sequence
  source 1..2970: mol_type = other DNA
atgggaggaagtggcagctctggcggcagtggagggtctggtggcagcggaggagtgcaggtggaaaccatctccccaggagacgggcgcaccttccccaagcgcggccagacctgcgtggtgcactacaccgggatgcttgaagatggaaagaaatttgattcctcccgggacagaaacaagccctttaagtttatgctaggcaagcaggaggtgatccgaggctgggaagaaggggttgcccagatgagtgtgggtcagagagccaaactgactatatctccagattatgcctatggtgccactgggcacccaggcatcatcccaccacatgccactctcgtcttcgatgtggagcttctaaaactggaaggaggaagcggcggttccggggggggatccggaagtggttccggggggtgtacaaacaagagcgtggccatggatatgctcaacgaagtgaagcggtgccccgacgagctgttcacaacactgtctgccgagaagcagtcccggttcagaatcatcagcgacgaccacaatgaagtgctgatgaagcggagcagcgacagattcgtgcctctgctgctgcagtatatcgattacggcaagctgttcgaccacatcaggttccacgtgaacatgggcaagctgagatacctgctgaaggccgacaagacctgcatcgacggccagaccagagtcagagtgatcgagcagcccctgaacggcttcggcagactggaagaggccgagacaatgcggaagcaagagaacggcaccttcggcaacagcggcatccggatcagagacttcgagaacatgaagcgggacgacgccaatcctgccaactatccctacatcgtggacacctacacacactacatcctggaaaacaacaaggtcgagatgtttatcaacgacaaagaggacagcgccccactgctgcccgtgatcgaggatgatagatacgtggtcaagacaatccccagctgccggatgagcaccctggaaattccagccatggccttccacatgtttctgttcggcagcaagaaaaccgagaagctgatcgtggacgtgcacaaccggtacaagagactgttccaggccatgcagaaagaagaagtgaccgccgagaatatcgccagcttcggaatcgccgagagcgacctgcctcagaagatcctggatctgatcagcggcaatgcccacggcaaggatgtggacgccttcatcagactgaccgtggacgacatgctgaccgacaccgagcggagaatcaagagattcaaggacgaccggaagtccattcggagcgccgacaacaagatgggaaagagaggcttcaagcagatctccacaggcaagctggccgacttcctggccaaggacatcgtgctgtttcagcccagcgtgaacgatggcgagaacaagatcaccggcctgaactaccggatcatgcagagcgccattgccgtgtacgatagcggcgacgattacgaggccaagcagcagttcaagctgatgttcgagaaggcccggctgatcggcaagggcacaacagagcctcatccatttctgtacaaggtgttcgcccgcagcatccccgccaatgccgtcgagttctacgagcgctacctgatcgagcggaagttctacctgaccggcctgtccaacgagatcaagaaaggcaacagagtggatgtgcccttcatccggcgggaccagaacaagtggaaaacacccgccatgaagaccctgggcagaatctacagcgaggatctgcccgtggaactgcccagacagatgttcgacaatgagatcaagtcccacctgaagtccctgccacagatggaaggcatcgacttcaacaatgccaacgtgacctatctgatcgccgagtacatgaagagagtgctggacgacgacttccagaccttctaccagtggaaccgcaactaccggtacatggacatgcttaagggcgagtacgacagaaagggctccctgcagcactgcttcaccagcgtggaagagagagaaggcctctggaaagagcgggcctccagaacagagcggtacagaaagcaggccagcaacaagatccgcagcaaccggcagatgagaaacgccagcagcgaagagatcgagacaatcctggataagcggctgagcaacagccggaacgagtaccagaaaagcgagaaagtgatccggcgctacagagtgcaggatgccctgctgtttctgctggccaaaaagaccctgaccgaactggccgatttcgacggcgagaggttcaaactgaaagaaatcatgcccgacgccgagaagggaatcctgagcgagatcatgcccatgagcttcaccttcgagaaaggcggcaagaagtacaccatcaccagcgagggcatgaagctgaagaactacggcgacttctttgtgctggctagcgacaagaggatcggcaacctgctggaactcgtgggcagcgacatcgtgtccaaagaggatatcatggaagagttcaacaaatacgaccagtgcaggcccgagatcagctccatcgtgttcaacctggaaaagtgggccttcgacacataccccgagctgtctgccagagtggaccgggaagagaaggtggacttcaagagcatcctgaaaatcctgctgaacaacaagaacatcaacaaagagcagagcgacatcctgcggaagatccggaacgccttcgatcacaacaattaccccgacaaaggcgtggtggaaatcaaggccctgcctgagatcgccatgagcatcaagaaggcctttggggagtacgccatcatgaagggatcccttcaactgcctccacttgaaagactgacactgggtagttcctacccatacgatgttccagattacgcttatccctacgacgtgcctgattatgcatacccatatgatgtccccgactatgcctaa

SEQ ID NO: 46 - DNA, 1443 bp, synthetic construct
  misc_feature 1..1443: note = N351-GS16-FRB-GS16 polynucleotide sequence
  source 1..1443: mol_type = other DNA
atgaacatccccgctctggtggaaaaccagaagaagtactttggcacctacagcgtgatggccatgctgaacgctcagaccgtgctggaccacatccagaaggtggccgatattgagggcgagcagaacgagaacaacgagaatctgtggtttcaccccgtgatgagccacctgtacaacgccaagaacggctacgacaagcagcccgagaaaaccatgttcatcatcgagcggctgcagagctacttcccattcctgaagatcatggccgagaaccagagagagtacagcaacggcaagtacaagcagaaccgcgtggaagtgaacagcaacgacatcttcgaggtgctgaagcgcgccttcggcgtgctgaagatgtacagggacctgaccaaccactacaagacctacgaggaaaagctgaacgacggctgcgagttcctgaccagcacagagcaacctctgagcggcatgatcaacaactactacacagtggccctgcggaacatgaacgagagatacggctacaagacagaggacctggccttcatccaggacaagcggttcaagttcgtgaaggacgcctacggcaagaaaaagtcccaagtgaataccggattcttcctgagcctgcaggactacaacggcgacacacagaagaagctgcacctgagcggagtgggaatcgccctgctgatctgcctgttcctggacaagcagtacatcaacatctttctgagcaggctgcccatcttctccagctacaatgcccagagcgaggaacggcggatcatcatcagatccttcggcatcaacagcatcaagctgcccaaggaccggatccacagcgagaagtccaacaagagcgtggccatggatatgctcaacgaagtgaagcggtgccccgacgagctgttcacaacactgtctgccgagaagcagtcccggttcagaatcatcagcgacgaccacaatgaagtgctgatgaagcggagcagcgacagattcgtgcctctgctgctgcagtatatcgattacggcaagctgttcgaccttccgggatccggaggaagtggcagctctggcggcagtggagggtctggtggcagcggaatcctctggcatgagatgtggcatgaaggcctggaagaggcatctcgtttgtactttggggaaaggaacgtgaaaggcatgtttgaggtgctggagcccttgcatgctatgatggaacggggcccccagactctgaaggaaacatcctttaatcaggcctatggtcgagatttaatggaggcccaagagtggtgcaggaagtacatgaaatcagggaatgtcaaggacctcacccaagcctgggacctctattatcatgtgttccgacgaatctcaaagggaggaagcggcggttccggggggggatccggaagtggttccggggggtag

SEQ ID NO: 47 - DNA, 2775 bp, synthetic construct
  misc_feature 1..2775: note = GS16-FKBP-GS16-C352 polynucleotide sequence
  source 1..2775: mol_type = other DNA
atgggaggaagtggcagctctggcggcagtggagggtctggtggcagcggaggagtgcaggtggaaaccatctccccaggagacgggcgcaccttccccaagcgcggccagacctgcgtggtgcactacaccgggatgcttgaagatggaaagaaatttgattcctcccgggacagaaacaagccctttaagtttatgctaggcaagcaggaggtgatccgaggctgggaagaaggggttgcccagatgagtgtgggtcagagagccaaactgactatatctccagattatgcctatggtgccactgggcacccaggcatcatcccaccacatgccactctcgtcttcgatgtggagcttctaaaactggaaggaggaagcggcggttccggggggggatccggaagtggttccggggggtgtacacacatcaggttccacgtgaacatgggcaagctgagatacctgctgaaggccgacaagacctgcatcgacggccagaccagagtcagagtgatcgagcagcccctgaacggcttcggcagactggaagaggccgagacaatgcggaagcaagagaacggcaccttcggcaacagcggcatccggatcagagacttcgagaacatgaagcgggacgacgccaatcctgccaactatccctacatcgtggacacctacacacactacatcctggaaaacaacaaggtcgagatgtttatcaacgacaaagaggacagcgccccactgctgcccgtgatcgaggatgatagatacgtggtcaagacaatccccagctgccggatgagcaccctggaaattccagccatggccttccacatgtttctgttcggcagcaagaaaaccgagaagctgatcgtggacgtgcacaaccggtacaagagactgttccaggccatgcagaaagaagaagtgaccgccgagaatatcgccagcttcggaatcgccgagagcgacctgcctcagaagatcctggatctgatcagcggcaatgcccacggcaaggatgtggacgccttcatcagactgaccgtggacgacatgctgaccgacaccgagcggagaatcaagagattcaaggacgaccggaagtccattcggagcgccgacaacaagatgggaaagagaggcttcaagcagatctccacaggcaagctggccgacttcctggccaaggacatcgtgctgtttcagcccagcgtgaacgatggcgagaacaagatcaccggcctgaactaccggatcatgcagagcgccattgccgtgtacgatagcggcgacgattacgaggccaagcagcagttcaagctgatgttcgagaaggcccggctgatcggcaagggcacaacagagcctcatccatttctgtacaaggtgttcgcccgcagcatccccgccaatgccgtcgagttctacgagcgctacctgatcgagcggaagttctacctgaccggcctgtccaacgagatcaagaaaggcaacagagtggatgtgcccttcatccggcgggaccagaacaagtggaaaacacccgccatgaagaccctgggcagaatctacagcgaggatctgcccgtggaactgcccagacagatgttcgacaatgagatcaagtcccacctgaagtccctgccacagatggaaggcatcgacttcaacaatgccaacgtgacctatctgatcgccgagtacatgaagagagtgctggacgacgacttccagaccttctaccagtggaaccgcaactaccggtacatggacatgcttaagggcgagtacgacagaaagggctccctgcagcactgcttcaccagcgtggaagagagagaaggcctctggaaagagcgggcctccagaacagagcggtacagaaagcaggccagcaacaagatccgcagcaaccggcagatgagaaacgccagcagcgaagagatcgagacaatcctggataagcggctgagcaacagccggaacgagtaccagaaaagcgagaaagtgatccggcgctacagagtgcaggatgccctgctgtttctgctggccaaaaagaccctgaccgaactggccgatttcgacggcgagaggttcaaactgaaagaaatcatgcccgacgccgagaagggaatcctgagcgagatcatgcccatgagcttcaccttcgagaaaggcggcaagaagtacaccatcaccagcgagggcatgaagctgaagaactacggcgacttctttgtgctggctagcgacaagaggatcggcaacctgctggaactcgtgggcagcgacatcgtgtccaaagaggatatcatggaagagttcaacaaatacgaccagtgcaggcccgagatcagctccatcgtgttcaacctggaaaagtgggccttcgacacataccccgagctgtctgccagagtggaccgggaagagaaggtggacttcaagagcatcctgaaaatcctgctgaacaacaagaacatcaacaaagagcagagcgacatcctgcggaagatccggaacgccttcgatcacaacaattaccccgacaaaggcgtggtggaaatcaaggccctgcctgagatcgccatgagcatcaagaaggcctttggggagtacgccatcatgaagggatcccttcaactgcctccacttgaaagactgacactgggtagttcctacccatacgatgttccagattacgcttatccctacgacgtgcctgattatgcatacccatatgatgtccccgactatgcctaa

SEQ ID NO: 48 - DNA, 1830 bp, synthetic construct
  misc_feature 1..1830: note = N480-GS16-FRB-GS16 polynucleotide sequence
  source 1..1830: mol_type = other DNA
atgaacatccccgctctggtggaaaaccagaagaagtactttggcacctacagcgtgatggccatgctgaacgctcagaccgtgctggaccacatccagaaggtggccgatattgagggcgagcagaacgagaacaacgagaatctgtggtttcaccccgtgatgagccacctgtacaacgccaagaacggctacgacaagcagcccgagaaaaccatgttcatcatcgagcggctgcagagctacttcccattcctgaagatcatggccgagaaccagagagagtacagcaacggcaagtacaagcagaaccgcgtggaagtgaacagcaacgacatcttcgaggtgctgaagcgcgccttcggcgtgctgaagatgtacagggacctgaccaaccactacaagacctacgaggaaaagctgaacgacggctgcgagttcctgaccagcacagagcaacctctgagcggcatgatcaacaactactacacagtggccctgcggaacatgaacgagagatacggctacaagacagaggacctggccttcatccaggacaagcggttcaagttcgtgaaggacgcctacggcaagaaaaagtcccaagtgaataccggattcttcctgagcctgcaggactacaacggcgacacacagaagaagctgcacctgagcggagtgggaatcgccctgctgatctgcctgttcctggacaagcagtacatcaacatctttctgagcaggctgcccatcttctccagctacaatgcccagagcgaggaacggcggatcatcatcagatccttcggcatcaacagcatcaagctgcccaaggaccggatccacagcgagaagtccaacaagagcgtggccatggatatgctcaacgaagtgaagcggtgccccgacgagctgttcacaacactgtctgccgagaagcagtcccggttcagaatcatcagcgacgaccacaatgaagtgctgatgaagcggagcagcgacagattcgtgcctctgctgctgcagtatatcgattacggcaagctgttcgaccacatcaggttccacgtgaacatgggcaagctgagatacctgctgaaggccgacaagacctgcatcgacggccagaccagagtcagagtgatcgagcagcccctgaacggcttcggcagactggaagaggccgagacaatgcggaagcaagagaacggcaccttcggcaacagcggcatccggatcagagacttcgagaacatgaagcgggacgacgccaatcctgccaactatccctacatcgtggacacctacacacactacatcctggaaaacaacaaggtcgagatgtttatcaacgacaaagaggacagcgccccactgctgcccgtgatcgaggatgatagatacgtggtcaagacaatccccagctgccggatgagcacccttccgggatccggaggaagtggcagctctggcggcagtggagggtctggtggcagcggaatcctctggcatgagatgtggcatgaaggcctggaagaggcatctcgtttgtactttggggaaaggaacgtgaaaggcatgtttgaggtgctggagcccttgcatgctatgatggaacggggcccccagactctgaaggaaacatcctttaatcaggcctatggtcgagatttaatggaggcccaagagtggtgcaggaagtacatgaaatcagggaatgtcaaggacctcacccaagcctgggacctctattatcatgtgttccgacgaatctcaaagggaggaagcggcggttccggggggggatccggaagtggttccggggggtag

SEQ ID NO: 49 - DNA, 2388 bp, synthetic construct
  misc_feature 1..2388: note = GS16-FKBP-GS16-C481 polynucleotide sequence
  source 1..2388: mol_type = other DNA
atgggaggaagtggcagctctggcggcagtggagggtctggtggcagcggaggagtgcaggtggaaaccatctccccaggagacgggcgcaccttccccaagcgcggccagacctgcgtggtgcactacaccgggatgcttgaagatggaaagaaatttgattcctcccgggacagaaacaagccctttaagtttatgctaggcaagcaggaggtgatccgaggctgggaagaaggggttgcccagatgagtgtgggtcagagagccaaactgactatatctccagattatgcctatggtgccactgggcacccaggcatcatcccaccacatgccactctcgtcttcgatgtggagcttctaaaactggaaggaggaagcggcggttccggggggggatccggaagtggttccggggggtgtacactggaaattccagccatggccttccacatgtttctgttcggcagcaagaaaaccgagaagctgatcgtggacgtgcacaaccggtacaagagactgttccaggccatgcagaaagaagaagtgaccgccgagaatatcgccagcttcggaatcgccgagagcgacctgcctcagaagatcctggatctgatcagcggcaatgcccacggcaaggatgtggacgccttcatcagactgaccgtggacgacatgctgaccgacaccgagcggagaatcaagagattcaaggacgaccggaagtccattcggagcgccgacaacaagatgggaaagagaggcttcaagcagatctccacaggcaagctggccgacttcctggccaaggacatcgtgctgtttcagcccagcgtgaacgatggcgagaacaagatcaccggcctgaactaccggatcatgcagagcgccattgccgtgtacgatagcggcgacgattacgaggccaagcagcagttcaagctgatgttcgagaaggcccggctgatcggcaagggcacaacagagcctcatccatttctgtacaaggtgttcgcccgcagcatccccgccaatgccgtcgagttctacgagcgctacctgatcgagcggaagttctacctgaccggcctgtccaacgagatcaagaaaggcaacagagtggatgtgcccttcatccggcgggaccagaacaagtggaaaacacccgccatgaagaccctgggcagaatctacagcgaggatctgcccgtggaactgcccagacagatgttcgacaatgagatcaagtcccacctgaagtccctgccacagatggaaggcatcgacttcaacaatgccaacgtgacctatctgatcgccgagtacatgaagagagtgctggacgacgacttccagaccttctaccagtggaaccgcaactaccggtacatggacatgcttaagggcgagtacgacagaaagggctccctgcagcactgcttcaccagcgtggaagagagagaaggcctctggaaagagcgggcctccagaacagagcggtacagaaagcaggccagcaacaagatccgcagcaaccggcagatgagaaacgccagcagcgaagagatcgagacaatcctggataagcggctgagcaacagccggaacgagtaccagaaaagcgagaaagtgatccggcgctacagagtgcaggatgccctgctgtttctgctggccaaaaagaccctgaccgaactggccgatttcgacggcgagaggttcaaactgaaagaaatcatgcccgacgccgagaagggaatcctgagcgagatcatgcccatgagcttcaccttcgagaaaggcggcaagaagtacaccatcaccagcgagggcatgaagctgaagaactacggcgacttctttgtgctggctagcgacaagaggatcggcaacctgctggaactcgtgggcagcgacatcgtgtccaaagaggatatcatggaagagttcaacaaatacgaccagtgcaggcccgagatcagctccatcgtgttcaacctggaaaagtgggccttcgacacataccccgagctgtctgccagagtggaccgggaagagaaggtggacttcaagagcatcctgaaaatcctgctgaacaacaagaacatcaacaaagagcagagcgacatcctgcggaagatccggaacgccttcgatcacaacaattaccccgacaaaggcgtggtggaaatcaaggccctgcctgagatcgccatgagcatcaagaaggcctttggggagtacgccatcatgaagggatcccttcaactgcctccacttgaaagactgacactgggtagttcctacccatacgatgttccagattacgcttatccctacgacgtgcctgattatgcatacccatatgatgtccccgactatgcctaa

SEQ ID NO: 50 - DNA, 2040 bp, synthetic construct
  misc_feature 1..2040: note = N550-GS16-FRB-GS16 polynucleotide sequence
  source 1..2040: mol_type = other DNA
atgaacatccccgctctggtggaaaaccagaagaagtactttggcacctacagcgtgatggccatgctgaacgctcagaccgtgctggaccacatccagaaggtggccgatattgagggcgagcagaacgagaacaacgagaatctgtggtttcaccccgtgatgagccacctgtacaacgccaagaacggctacgacaagcagcccgagaaaaccatgttcatcatcgagcggctgcagagctacttcccattcctgaagatcatggccgagaaccagagagagtacagcaacggcaagtacaagcagaaccgcgtggaagtgaacagcaacgacatcttcgaggtgctgaagcgcgccttcggcgtgctgaagatgtacagggacctgaccaaccactacaagacctacgaggaaaagctgaacgacggctgcgagttcctgaccagcacagagcaacctctgagcggcatgatcaacaactactacacagtggccctgcggaacatgaacgagagatacggctacaagacagaggacctggccttcatccaggacaagcggttcaagttcgtgaaggacgcctacggcaagaaaaagtcccaagtgaataccggattcttcctgagcctgcaggactacaacggcgacacacagaagaagctgcacctgagcggagtgggaatcgccctgctgatctgcctgttcctggacaagcagtacatcaacatctttctgagcaggctgcccatcttctccagctacaatgcccagagcgaggaacggcggatcatcatcagatccttcggcatcaacagcatcaagctgcccaaggaccggatccacagcgagaagtccaacaagagcgtggccatggatatgctcaacgaagtgaagcggtgccccgacgagctgttcacaacactgtctgccgagaagcagtcccggttcagaatcatcagcgacgaccacaatgaagtgctgatgaagcggagcagcgacagattcgtgcctctgctgctgcagtatatcgattacggcaagctgttcgaccacatcaggttccacgtgaacatgggcaagctgagatacctgctgaaggccgacaagacctgcatcgacggccagaccagagtcagagtgatcgagcagcccctgaacggcttcggcagactggaagaggccgagacaatgcggaagcaagagaacggcaccttcggcaacagcggcatccggatcagagacttcgagaacatgaagcgggacgacgccaatcctgccaactatccctacatcgtggacacctacacacactacatcctggaaaacaacaaggtcgagatgtttatcaacgacaaagaggacagcgccccactgctgcccgtgatcgaggatgatagatacgtggtcaagacaatccccagctgccggatgagcaccctggaaattccagccatggccttccacatgtttctgttcggcagcaagaaaaccgagaagctgatcgtggacgtgcacaaccggtacaagagactgttccaggccatgcagaaagaagaagtgaccgccgagaatatcgccagcttcggaatcgccgagagcgacctgcctcagaagatcctggatctgatcagcggcaatgcccacggcttcccgggatccggaggaagtggcagctctggcggcagtggagggtctggtggcagcggaatcctctggcatgagatgtggcatgaaggcctggaagaggcatctcgtttgtactttggggaaaggaacgtgaaaggcatgtttgaggtgctggagcccttgcatgctatgatggaacggggcccccagactctgaaggaaacatcctttaatcaggcctatggtcgagatttaatggaggcccaagagtggtgcaggaagtacatgaaatcagggaatgtcaaggacctcacccaagcctgggacctctattatcatgtgttccgacgaatctcaaagggaggaagcggcggttccggggggggatccggaagtggttccggggggtag

SEQ ID NO: 51 - DNA, 2178 bp, synthetic construct
  misc_feature 1..2178: note = GS16-FKBP-GS16-C551 polynucleotide sequence
  source 1..2178: mol_type = other DNA
atgggaggaagtggcagctctggcggcagtggagggtctggtggcagcggaggagtgcaggtggaaaccatctccccaggagacgggcgcaccttccccaagcgcggccagacctgcgtggtgcactacaccgggatgcttgaagatggaaagaaatttgattcctcccgggacagaaacaagccctttaagtttatgctaggcaagcaggaggtgatccgaggctgggaagaaggggttgcccagatgagtgtgggtcagagagccaaactgactatatctccagattatgcctatggtgccactgggcacccaggcatcatcccaccacatgccactctcgtcttcgatgtggagcttctaaaactggaaggaggaagcggcggttccggggggggatccggaagtggttccggggggtgtacaaaggatgtggacgccttcatcagactgaccgtggacgacatgctgaccgacaccgagcggagaatcaagagattcaaggacgaccggaagtccattcggagcgccgacaacaagatgggaaagagaggcttcaagcagatctccacaggcaagctggccgacttcctggccaaggacatcgtgctgtttcagcccagcgtgaacgatggcgagaacaagatcaccggcctgaactaccggatcatgcagagcgccattgccgtgtacgatagcggcgacgattacgaggccaagcagcagttcaagctgatgttcgagaaggcccggctgatcggcaagggcacaacagagcctcatccatttctgtacaaggtgttcgcccgcagcatccccgccaatgccgtcgagttctacgagcgctacctgatcgagcggaagttctacctgaccggcctgtccaacgagatcaagaaaggcaacagagtggatgtgcccttcatccggcgggaccagaacaagtggaaaacacccgccatgaagaccctgggcagaatctacagcgaggatctgcccgtggaactgcccagacagatgttcgacaatgagatcaagtcccacctgaagtccctgccacagatggaaggcatcgacttcaacaatgccaacgtgacctatctgatcgccgagtacatgaagagagtgctggacgacgacttccagaccttctaccagtggaaccgcaactaccggtacatggacatgcttaagggcgagtacgacagaaagggctccctgcagcactgcttcaccagcgtggaagagagagaaggcctctggaaagagcgggcctccagaacagagcggtacagaaagcaggccagcaacaagatccgcagcaaccggcagatgagaaacgccagcagcgaagagatcgagacaatcctggataagcggctgagcaacagccggaacgagtaccagaaaagcgagaaagtgatccggcgctacagagtgcaggatgccctgctgtttctgctggccaaaaagaccctgaccgaactggccgatttcgacggcgagaggttcaaactgaaagaaatcatgcccgacgccgagaagggaatcctgagcgagatcatgcccatgagcttcaccttcgagaaaggcggcaagaagtacaccatcaccagcgagggcatgaagctgaagaactacggcgacttctttgtgctggctagcgacaagaggatcggcaacctgctggaactcgtgggcagcgacatcgtgtccaaagaggatatcatggaagagttcaacaaatacgaccagtgcaggcccgagatcagctccatcgtgttcaacctggaaaagtgggccttcgacacataccccgagctgtctgccagagtggaccgggaagagaaggtggacttcaagagcatcctgaaaatcctgctgaacaacaagaacatcaacaaagagcagagcgacatcctgcggaagatccggaacgccttcgatcacaacaattaccccgacaaaggcgtggtggaaatcaaggccctgcctgagatcgccatgagcatcaagaaggcctttggggagtacgccatcatgaagggatcccttcaactgcctccacttgaaagactgacactgggtagttcctacccatacgatgttccagattacgcttatccctacgacgtgcctgattatgcatacccatatgatgtccccgactatgcctaa

SEQ ID NO: 52 - DNA, 2262 bp, synthetic construct
  misc_feature 1..2262: note = N624-GS16-FRB-GS16 polynucleotide sequence
  source 1..2262: mol_type = other DNA
atgaacatccccgctctggtggaaaaccagaagaagtactttggcacctacagcgtgatggccatgctgaacgctcagaccgtgctggaccacatccagaaggtggccgatattgagggcgagcagaacgagaacaacgagaatctgtggtttcaccccgtgatgagccacctgtacaacgccaagaacggctacgacaagcagcccgagaaaaccatgttcatcatcgagcggctgcagagctacttcccattcctgaagatcatggccgagaaccagagagagtacagcaacggcaagtacaagcagaaccgcgtggaagtgaacagcaacgacatcttcgaggtgctgaagcgcgccttcggcgtgctgaagatgtacagggacctgaccaaccactacaagacctacgaggaaaagctgaacgacggctgcgagttcctgaccagcacagagcaacctctgagcggcatgatcaacaactactacacagtggccctgcggaacatgaacgagagatacggctacaagacagaggacctggccttcatccaggacaagcggttcaagttcgtgaaggacgcctacggcaagaaaaagtcccaagtgaataccggattcttcctgagcctgcaggactacaacggcgacacacagaagaagctgcacctgagcggagtgggaatcgccctgctgatctgcctgttcctggacaagcagtacatcaacatctttctgagcaggctgcccatcttctccagctacaatgcccagagcgaggaacggcggatcatcatcagatccttcggcatcaacagcatcaagctgcccaaggaccggatccacagcgagaagtccaacaagagcgtggccatggatatgctcaacgaagtgaagcggtgccccgacgagctgttcacaacactgtctgccgagaagcagtcccggttcagaatcatcagcgacgaccacaatgaagtgctgatgaagcggagcagcgacagattcgtgcctctgctgctgcagtatatcgattacggcaagctgttcgaccacatcaggttccacgtgaacatgggcaagctgagatacctgctgaaggccgacaagacctgcatcgacggccagaccagagtcagagtgatcgagcagcccctgaacggcttcggcagactggaagaggccgagacaatgcggaagcaagagaacggcaccttcggcaacagcggcatccggatcagagacttcgagaacatgaagcgggacgacgccaatcctgccaactatccctacatcgtggacacctacacacactacatcctggaaaacaacaaggtcgagatgtttatcaacgacaaagaggacagcgccccactgctgcccgtgatcgaggatgatagatacgtggtcaagacaatccccagctgccggatgagcaccctggaaattccagccatggccttccacatgtttctgttcggcagcaagaaaaccgagaagctgatcgtggacgtgcacaaccggtacaagagactgttccaggccatgcagaaagaagaagtgaccgccgagaatatcgccagcttcggaatcgccgagagcgacctgcctcagaagatcctggatctgatcagcggcaatgcccacggcaaggatgtggacgccttcatcagactgaccgtggacgacatgctgaccgacaccgagcggagaatcaagagattcaaggacgaccggaagtccattcggagcgccgacaacaagatgggaaagagaggcttcaagcagatctccacaggcaagctggccgacttcctggccaaggacatcgtgctgtttcagcccagcgtgaacgatggcgagaacaagatcaacccgggatccggaggaagtggcagctctggcggcagtggagggtctggtggcagcggaatcctctggcatgagatgtggcatgaaggcctggaagaggcatctcgtttgtactttggggaaaggaacgtgaaaggcatgtttgaggtgctggagcccttgcatgctatgatggaacggggcccccagactctgaaggaaacatcctttaatcaggcctatggtcgagatttaatggaggcccaagagtggtgcaggaagtacatgaaatcagggaatgtcaaggacctcacccaagcctgggacctctattatcatgtgttccgacgaatctcaaagggaggaagcggcggttccggggggggatccggaagtggttccggggggtag

SEQ ID NO: 53 - DNA, 1956 bp, synthetic construct
  misc_feature 1..1956: note = GS16-FKBP-GS16-C625 polynucleotide sequence
  source 1..1956: mol_type = other DNA
atgggaggaagtggcagctctggcggcagtggagggtctggtggcagcggaggagtgcaggtggaaaccatctccccaggagacgggcgcaccttccccaagcgcggccagacctgcgtggtgcactacaccgggatgcttgaagatggaaagaaatttgattcctcccgggacagaaacaagccctttaagtttatgctaggcaagcaggaggtgatccgaggctgggaagaaggggttgcccagatgagtgtgggtcagagagccaaactgactatatctccagattatgcctatggtgccactgggcacccaggcatcatcccaccacatgccactctcgtcttcgatgtggagcttctaaaactggaaggaggaagcggcggttccggggggggatccggaagtggttccggggggtgtacaaccggcctgaactaccggatcatgcagagcgccattgccgtgtacgatagcggcgacgattacgaggccaagcagcagttcaagctgatgttcgagaaggcccggctgatcggcaagggcacaacagagcctcatccatttctgtacaaggtgttcgcccgcagcatccccgccaatgccgtcgagttctacgagcgctacctgatcgagcggaagttctacctgaccggcctgtccaacgagatcaagaaaggcaacagagtggatgtgcccttcatccggcgggaccagaacaagtggaaaacacccgccatgaagaccctgggcagaatctacagcgaggatctgcccgtggaactgcccagacagatgttcgacaatgagatcaagtcccacctgaagtccctgccacagatggaaggcatcgacttcaacaatgccaacgtgacctatctgatcgccgagtacatgaagagagtgctggacgacgacttccagaccttctaccagtggaaccgcaactaccggtacatggacatgcttaagggcgagtacgacagaaagggctccctgcagcactgcttcaccagcgtggaagagagagaaggcctctggaaagagcgggcctccagaacagagcggtacagaaagcaggccagcaacaagatccgcagcaaccggcagatgagaaacgccagcagcgaagagatcgagacaatcctggataagcggctgagcaacagccggaacgagtaccagaaaagcgagaaagtgatccggcgctacagagtgcaggatgccctgctgtttctgctggccaaaaagaccctgaccgaactggccgatttcgacggcgagaggttcaaactgaaagaaatcatgcccgacgccgagaagggaatcctgagcgagatcatgcccatgagcttcaccttcgagaaaggcggcaagaagtacaccatcaccagcgagggcatgaagctgaagaactacggcgacttctttgtgctggctagcgacaagaggatcggcaacctgctggaactcgtgggcagcgacatcgtgtccaaagaggatatcatggaagagttcaacaaatacgaccagtgcaggcccgagatcagctccatcgtgttcaacctggaaaagtgggccttcgacacataccccgagctgtctgccagagtggaccgggaagagaaggtggacttcaagagcatcctgaaaatcctgctgaacaacaagaacatcaacaaagagcagagcgacatcctgcggaagatccggaacgccttcgatcacaacaattaccccgacaaaggcgtggtggaaatcaaggccctgcctgagatcgccatgagcatcaagaaggcctttggggagtacgccatcatgaagggatcccttcaactgcctccacttgaaagactgacactgggtagttcctacccatacgatgttccagattacgcttatccctacgacgtgcctgattatgcatacccatatgatgtccccgactatgcctaa

SEQ ID NO: 54 - DNA, 2565 bp, synthetic construct
  misc_feature 1..2565: note = N725-GS16-FRB-GS16 polynucleotide sequence
  source 1..2565: mol_type = other DNA
atgaacatccccgctctggtggaaaaccagaagaagtactttggcacctacagcgtgatggccatgctgaacgctcagaccgtgctggaccacatccagaaggtggccgatattgagggcgagcagaacgagaacaacgagaatctgtggtttcaccccgtgatgagccacctgtacaacgccaagaacggctacgacaagcagcccgagaaaaccatgttcatcatcgagcggctgcagagctacttcccattcctgaagatcatggccgagaaccagagagagtacagcaacggcaagtacaagcagaaccgcgtggaagtgaacagcaacgacatcttcgaggtgctgaagcgcgccttcggcgtgctgaagatgtacagggacctgaccaaccactacaagacctacgaggaaaagctgaacgacggctgcgagttcctgaccagcacagagcaacctctgagcggcatgatcaacaactactacacagtggccctgcggaacatgaacgagagatacggctacaagacagaggacctggccttcatccaggacaagcggttcaagttcgtgaaggacgcctacggcaagaaaaagtcccaagtgaataccggattcttcctgagcctgcaggactacaacggcgacacacagaagaagctgcacctgagcggagtgggaatcgccctgctgatctgcctgttcctggacaagcagtacatcaacatctttctgagcaggctgcccatcttctccagctacaatgcccagagcgaggaacggcggatcatcatcagatccttcggcatcaacagcatcaagctgcccaaggaccggatccacagcgagaagtccaacaagagcgtggccatggatatgctcaacgaagtgaagcggtgccccgacgagctgttcacaacactgtctgccgagaagcagtcccggttcagaatcatcagcgacgaccacaatgaagtgctgatgaagcggagcagcgacagattcgtgcctctgctgctgcagtatatcgattacggcaagctgttcgaccacatcaggttccacgtgaacatgggcaagctgagatacctgctgaaggccgacaagacctgcatcgacggccagaccagagtcagagtgatcgagcagcccctgaacggcttcggcagactggaagaggccgagacaatgcggaagcaagagaacggcaccttcggcaacagcggcatccggatcagagacttcgagaacatgaagcgggacgacgccaatcctgccaactatccctacatcgtggacacctacacacactacatcctggaaaacaacaaggtcgagatgtttatcaacgacaaagaggacagcgccccactgctgcccgtgatcgaggatgatagatacgtggtcaagacaatccccagctgccggatgagcaccctggaaattccagccatggccttccacatgtttctgttcggcagcaagaaaaccgagaagctgatcgtggacgtgcacaaccggtacaagagactgttccaggccatgcagaaagaagaagtgaccgccgagaatatcgccagcttcggaatcgccgagagcgacctgcctcagaagatcctggatctgatcagcggcaatgcccacggcaaggatgtggacgccttcatcagactgaccgtggacgacatgctgaccgacaccgagcggagaatcaagagattcaaggacgaccggaagtccattcggagcgccgacaacaagatgggaaagagaggcttcaagcagatctccacaggcaagctggccgacttcctggccaaggacatcgtgctgtttcagcccagcgtgaacgatggcgagaacaagatcaccggcctgaactaccggatcatgcagagcgccattgccgtgtacgatagcggcgacgattacgaggccaagcagcagttcaagctgatgttcgagaaggcccggctgatcggcaagggcacaacagagcctcatccatttctgtacaaggtgttcgcccgcagcatccccgccaatgccgtcgagttctacgagcgctacctgatcgagcggaagttctacctgaccggcctgtccaacgagatcaagaaaggcaacagagtggatgtgcccttcatccggcgggaccagaacaagtggaaacccccgggatccggaggaagtggcagctctggcggcagtggagggtctggtggcagcggaatcctctggcatgagatgtggcatgaaggcctggaagaggcatctcgtttgtactttggggaaaggaacgtgaaaggcatgtttgaggtgctggagcccttgcatgctatgatggaacggggcccccagactctgaaggaaacatcctttaatcaggcctatggtcgagatttaatggaggcccaagagtggtgcaggaagtacatgaaatcagggaatgtcaaggacctcacccaagcctgggacctctattatcatgtgttccgacgaatctcaaagggaggaagcggcggttccggggggggatccggaagtggttccggggggtag

SEQ ID NO: 55 - DNA, 1653 bp, synthetic construct
  misc_feature 1..1653: note = GS16-FKBP-GS16-C726 polynucleotide sequence
  source 1..1653: mol_type = other DNA
atgggaggaagtggcagctctggcggcagtggagggtctggtggcagcggaggagtgcaggtggaaaccatctccccaggagacgggcgcaccttccccaagcgcggccagacctgcgtggtgcactacaccgggatgcttgaagatggaaagaaatttgattcctcccgggacagaaacaagccctttaagtttatgctaggcaagcaggaggtgatccgaggctgggaagaaggggttgcccagatgagtgtgggtcagagagccaaactgactatatctccagattatgcctatggtgccactgggcacccaggcatcatcccaccacatgccactctcgtcttcgatgtggagcttctaaaactggaaggaggaagcggcggttccggggggggatccggaagtggttccggggggtgtacaacacccgccatgaagaccctgggcagaatctacagcgaggatctgcccgtggaactgcccagacagatgttcgacaatgagatcaagtcccacctgaagtccctgccacagatggaaggcatcgacttcaacaatgccaacgtgacctatctgatcgccgagtacatgaagagagtgctggacgacgacttccagaccttctaccagtggaaccgcaactaccggtacatggacatgcttaagggcgagtacgacagaaagggctccctgcagcactgcttcaccagcgtggaagagagagaaggcctctggaaagagcgggcctccagaacagagcggtacagaaagcaggccagcaacaagatccgcagcaaccggcagatgagaaacgccagcagcgaagagatcgagacaatcctggataagcggctgagcaacagccggaacgagtaccagaaaagcgagaaagtgatccggcgctacagagtgcaggatgccctgctgtttctgctggccaaaaagaccctgaccgaactggccgatttcgacggcgagaggttcaaactgaaagaaatcatgcccgacgccgagaagggaatcctgagcgagatcatgcccatgagcttcaccttcgagaaaggcggcaagaagtacaccatcaccagcgagggcatgaagctgaagaactacggcgacttctttgtgctggctagcgacaagaggatcggcaacctgctggaactcgtgggcagcgacatcgtgtccaaagaggatatcatggaagagttcaacaaatacgaccagtgcaggcccgagatcagctccatcgtgttcaacctggaaaagtgggccttcgacacataccccgagctgtctgccagagtggaccgggaagagaaggtggacttcaagagcatcctgaaaatcctgctgaacaacaagaacatcaacaaagagcagagcgacatcctgcggaagatccggaacgccttcgatcacaacaattaccccgacaaaggcgtggtggaaatcaaggccctgcctgagatcgccatgagcatcaagaaggcctttggggagtacgccatcatgaagggatcccttcaactgcctccacttgaaagactgacactgggtagttcctacccatacgatgttccagattacgcttatccctacgacgtgcctgattatgcatacccatatgatgtccccgactatgcctaa

SEQ ID NO: 56 - DNA, 3174 bp, synthetic construct
  misc_feature 1..3174: note = N928-GS16-FRB-GS16 polynucleotide sequence
  source 1..3174: mol_type = other DNA
atgaacatccccgctctggtggaaaaccagaagaagtactttggcacctacagcgtgatggccatgctgaacgctcagaccgtgctggaccacatccagaaggtggccgatattgagggcgagcagaacgagaacaacgagaatctgtggtttcaccccgtgatgagccacctgtacaacgccaagaacggctacgacaagcagcccgagaaaaccatgttcatcatcgagcggctgcagagctacttcccattcctgaagatcatggccgagaaccagagagagtacagcaacggcaagtacaagcagaaccgcgtggaagtgaacagcaacgacatcttcgaggtgctgaagcgcgccttcggcgtgctgaagatgtacagggacctgaccaaccactacaagacctacgaggaaaagctgaacgacggctgcgagttcctgaccagcacagagcaacctctgagcggcatgatcaacaactactacacagtggccctgcggaacatgaacgagagatacggctacaagacagaggacctggccttcatccaggacaagcggttcaagttcgtgaaggacgcctacggcaagaaaaagtcccaagtgaataccggattcttcctgagcctgcaggactacaacggcgacacacagaagaagctgcacctgagcggagtgggaatcgccctgctgatctgcctgttcctggacaagcagtacatcaacatctttctgagcaggctgcccatcttctccagctacaatgcccagagcgaggaacggcggatcatcatcagatccttcggcatcaacagcatcaagctgcccaaggaccggatccacagcgagaagtccaacaagagcgtggccatggatatgctcaacgaagtgaagcggtgccccgacgagctgttcacaacactgtctgccgagaagcagtcccggttcagaatcatcagcgacgaccacaatgaagtgctgatgaagcggagcagcgacagattcgtgcctctgctgctgcagtatatcgattacggcaagctgttcgaccacatcaggttccacgtgaacatgggcaagctgagatacctgctgaaggccgacaagacctgcatcgacggccagaccagagtcagagtgatcgagcagcccctgaacggcttcggcagactggaagaggccgagacaatgcggaagcaagagaacggcaccttcggcaacagcggcatccggatcagagacttcgagaacatgaagcgggacgacgccaatcctgccaactatccctacatcgtggacacctacacacactacatcctggaaaacaacaaggtcgagatgtttatcaacgacaaagaggacagcgccccactgctgcccgtgatcgaggatgatagatacgtggtcaagacaatccccagctgccggatgagcaccctggaaattccagccatggccttccacatgtttctgttcggcagcaagaaaaccgagaagctgatcgtggacgtgcacaaccggtacaagagactgttccaggccatgcagaaagaagaagtgaccgccgagaatatcgccagcttcggaatcgccgagagcgacctgcctcagaagatcctggatctgatcagcggcaatgcccacggcaaggatgtggacgccttcatcagactgaccgtggacgacatgctgaccgacaccgagcggagaatcaagagattcaaggacgaccggaagtccattcggagcgccgacaacaagatgggaaagagaggcttcaagcagatctccacaggcaagctggccgacttcctggccaaggacatcgtgctgtttcagcccagcgtgaacgatggcgagaacaagatcaccggcctgaactaccggatcatgcagagcgccattgccgtgtacgatagcggcgacgattacgaggccaagcagcagttcaagctgatgttcgagaaggcccggctgatcggcaagggcacaacagagcctcatccatttctgtacaaggtgttcgcccgcagcatccccgccaatgccgtcgagttctacgagcgctacctgatcgagcggaagttctacctgaccggcctgtccaacgagatcaagaaaggcaacagagtggatgtgcccttcatccggcgggaccagaacaagtggaaaacacccgccatgaagaccctgggcagaatctacagcgaggatctgcccgtggaactgcccagacagatgttcgacaatgagatcaagtcccacctgaagtccctgccacagatggaaggcatcgacttcaacaatgccaacgtgacctatctgatcgccgagtacatgaagagagtgctggacgacgacttccagaccttctaccagtggaaccgcaactaccggtacatggacatgcttaagggcgagtacgacagaaagggctccctgcagcactgcttcaccagcgtggaagagagagaaggcctctggaaagagcgggcctccagaacagagcggtacagaaagcaggccagcaacaagatccgcagcaaccggcagatgagaaacgccagcagcgaagagatcgagacaatcctggataagcggctgagcaacagccggaacgagtaccagaaaagcgagaaagtgatccggcgctacagagtgcaggatgccctgctgtttctgctggccaaaaagaccctgaccgaactggccgatttcgacggcgagaggttcaaactgaaagaaatcatgcccgacgccgagaagggaatcctgagcgagttcccgggatccggaggaagtggcagctctggcggcagtggagggtctggtggcagcggaatcctctggcatgagatgtggcatgaaggcctggaagaggcatctcgtttgtactttggggaaaggaacgtgaaaggcatgtttgaggtgctggagcccttgcatgctatgatggaacggggcccccagactctgaaggaaacatcctttaatcaggcctatggtcgagatttaatggaggcccaagagtggtgcaggaagtacatgaaatcagggaatgtcaaggacctcacccaagcctgggacctctattatcatgtgttccgacgaatctcaaagggaggaagcggcggttccggggggggatccggaagtggttccggggggtag

SEQ ID NO: 57 - DNA, 1044 bp, synthetic construct
  misc_feature 1..1044: note = GS16-FKBP-GS16-C929 polynucleotide sequence
  source 1..1044: mol_type = other DNA
atgggaggaagtggcagctctggcggcagtggagggtctggtggcagcggaggagtgcaggtggaaaccatctccccaggagacgggcgcaccttccccaagcgcggccagacctgcgtggtgcactacaccgggatgcttgaagatggaaagaaatttgattcctcccgggacagaaacaagccctttaagtttatgctaggcaagcaggaggtgatccgaggctgggaagaaggggttgcccagatgagtgtgggtcagagagccaaactgactatatctccagattatgcctatggtgccactgggcacccaggcatcatcccaccacatgccactctcgtcttcgatgtggagcttctaaaactggaaggaggaagcggcggttccggggggggatccggaagtggttccggggggtgtacaatcatgcccatgagcttcaccttcgagaaaggcggcaagaagtacaccatcaccagcgagggcatgaagctgaagaactacggcgacttctttgtgctggctagcgacaagaggatcggcaacctgctggaactcgtgggcagcgacatcgtgtccaaagaggatatcatggaagagttcaacaaatacgaccagtgcaggcccgagatcagctccatcgtgttcaacctggaaaagtgggccttcgacacataccccgagctgtctgccagagtggaccgggaagagaaggtggacttcaagagcatcctgaaaatcctgctgaacaacaagaacatcaacaaagagcagagcgacatcctgcggaagatccggaacgccttcgatcacaacaattaccccgacaaaggcgtggtggaaatcaaggccctgcctgagatcgccatgagcatcaagaaggcctttggggagtacgccatcatgaagggatcccttcaactgcctccacttgaaagactgacactgggtagttcctacccatacgatgttccagattacgcttatccctacgacgtgcctgattatgcatacccatatgatgtccccgactatgcctaa

SEQ ID NO: 58 - DNA, 1377 bp, synthetic construct
  misc_feature 1..1377: note = N272-GS16-pMag-GS16 polynucleotide sequence
  source 1..1377: mol_type = other DNA
atgaacatccccgctctggtggaaaaccagaagaagtactttggcacctacagcgtgatggccatgctgaacgctcagaccgtgctggaccacatccagaaggtggccgatattgagggcgagcagaacgagaacaacgagaatctgtggtttcaccccgtgatgagccacctgtacaacgccaagaacggctacgacaagcagcccgagaaaaccatgttcatcatcgagcggctgcagagctacttcccattcctgaagatcatggccgagaaccagagagagtacagcaacggcaagtacaagcagaaccgcgtggaagtgaacagcaacgacatcttcgaggtgctgaagcgcgccttcggcgtgctgaagatgtacagggacctgaccaaccactacaagacctacgaggaaaagctgaacgacggctgcgagttcctgaccagcacagagcaacctctgagcggcatgatcaacaactactacacagtggccctgcggaacatgaacgagagatacggctacaagacagaggacctggccttcatccaggacaagcggttcaagttcgtgaaggacgcctacggcaagaaaaagtcccaagtgaataccggattcttcctgagcctgcaggactacaacggcgacacacagaagaagctgcacctgagcggagtgggaatcgccctgctgatctgcctgttcctggacaagcagtacatcaacatctttctgagcaggctgcccatcttctccagctacaatgcccagagcgaggaacggcggatcatcatcagatccttcggcatcaacaacccgggatccggaggaagtggcagctctggcggcagtggagggtctggtggcagcggacacaccctgtacgcccccggcggctacgacatcatgggctacctgagacagatcagaaacagacccaacccccaggtggagctgggccccgtggacaccagctgcgccctgatcctgtgcgacctgaagcagaaggacacccccatcgtgtacgccagcgaggccttcctgtatatgaccggctacagcaacgccgaggtgctgggcagaaactgcagattcctgcagagccccgacggcatggtgaagcccaagagcaccagaaagtacgtggacagcaacaccatcaacaccatcagaaaggccatcgacagaaacgccgaggtgcaggtggaggtggtgaacttcaagaagaacggccagagattcgtgaacttcctgaccatcatccccgtgagagacgagaccggcgagtacagatacagcatgggcttccagtgcgagaccgagggaggaagcggcggttccggggggggatccggaagtggttccggggggtag

SEQ ID NO: 59 - DNA, 3141 bp, synthetic construct
  misc_feature 1..3141: note = GS16-nMag-GS16-C273 polynucleotide sequence
  source 1..3141: mol_type = other DNA
atgggaggaagtggcagctctggcggcagtggagggtctggtggcagcggacacaccctgtacgcccccggcggctacgacatcatgggctacctggaccagatcggcaacagacccaacccccaggtggagctgggccccgtggacaccagctgcgccctgatcctgtgcgacctgaagcagaaggacacccccatcgtgtacgccagcgaggccttcctgtatatgaccggctacagcaacgccgaggtgctgggcagaaactgcagattcctgcagagccccgacggcatggtgaagcccaagagcaccagaaagtacgtggacagcaacaccatcaacaccatgagaaaggccatcgacagaaacgccgaggtgcaggtggaggtggtgaacttcaagaagaacggccagagattcgtgaacttcctgaccatgatccccgtgagagacgagaccggcgagtacagatacagcatgggcttccagtgcgagaccgagggaggaagcggcggttccggggggggatccggaagtggttccggggggtgtacaagcatcaagctgcccaaggaccggatccacagcgagaagtccaacaagagcgtggccatggatatgctcaacgaagtgaagcggtgccccgacgagctgttcacaacactgtctgccgagaagcagtcccggttcagaatcatcagcgacgaccacaatgaagtgctgatgaagcggagcagcgacagattcgtgcctctgctgctgcagtatatcgattacggcaagctgttcgaccacatcaggttccacgtgaacatgggcaagctgagatacctgctgaaggccgacaagacctgcatcgacggccagaccagagtcagagtgatcgagcagcccctgaacggcttcggcagactggaagaggccgagacaatgcggaagcaagagaacggcaccttcggcaacagcggcatccggatcagagacttcgagaacatgaagcgggacgacgccaatcctgccaactatccctacatcgtggacacctacacacactacatcctggaaaacaacaaggtcgagatgtttatcaacgacaaagaggacagcgccccactgctgcccgtgatcgaggatgatagatacgtggtcaagacaatccccagctgccggatgagcaccctggaaattccagccatggccttccacatgtttctgttcggcagcaagaaaaccgagaagctgatcgtggacgtgcacaaccggtacaagagactgttccaggccatgcagaaagaagaagtgaccgccgagaatatcgccagcttcggaatcgccgagagcgacctgcctcagaagatcctggatctgatcagcggcaatgcccacggcaaggatgtggacgccttcatcagactgaccgtggacgacatgctgaccgacaccgagcggagaatcaagagattcaaggacgaccggaagtccattcggagcgccgacaacaagatgggaaagagaggcttcaagcagatctccacaggcaagctggccgacttcctggccaaggacatcgtgctgtttcagcccagcgtgaacgatggcgagaacaagatcaccggcctgaactaccggatcatgcagagcgccattgccgtgtacgatagcggcgacgattacgaggccaagcagcagttcaagctgatgttcgagaaggcccggctgatcggcaagggcacaacagagcctcatccatttctgtacaaggtgttcgcccgcagcatccccgccaatgccgtcgagttctacgagcgctacctgatcgagcggaagttctacctgaccggcctgtccaacgagatcaagaaaggcaacagagtggatgtgcccttcatccggcgggaccagaacaagtggaaaacacccgccatgaagaccctgggcagaatctacagcgaggatctgcccgtggaactgcccagacagatgttcgacaatgagatcaagtcccacctgaagtccctgccacagatggaaggcatcgacttcaacaatgccaacgtgacctatctgatcgccgagtacatgaagagagtgctggacgacgacttccagaccttctaccagtggaaccgcaactaccggtacatggacatgcttaagggcgagtacgacagaaagggctccctgcagcactgcttcaccagcgtggaagagagagaaggcctctggaaagagcgggcctccagaacagagcggtacagaaagcaggccagcaacaagatccgcagcaaccggcagatgagaaacgccagcagcgaagagatcgagacaatcctggataagcggctgagcaacagccggaacgagtaccagaaaagcgagaaagtgatccggcgctacagagtgcaggatgccctgctgtttctgctggccaaaaagaccctgaccgaactggccgatttcgacggcgagaggttcaaactgaaagaaatcatgcccgacgccgagaagggaatcctgagcgagatcatgcccatgagcttcaccttcgagaaaggcggcaagaagtacaccatcaccagcgagggcatgaagctgaagaactacggcgacttctttgtgctggctagcgacaagaggatcggcaacctgctggaactcgtgggcagcgacatcgtgtccaaagaggatatcatggaagagttcaacaaatacgaccagtgcaggcccgagatcagctccatcgtgttcaacctggaaaagtgggccttcgacacataccccgagctgtctgccagagtggaccgggaagagaaggtggacttcaagagcatcctgaaaatcctgctgaacaacaagaacatcaacaaagagcagagcgacatcctgcggaagatccggaacgccttcgatcacaacaattaccccgacaaaggcgtggtggaaatcaaggccctgcctgagatcgccatgagcatcaagaaggcctttggggagtacgccatcatgaagggatcccttcaactgcctccacttgaaagactgacactgggtagttcctacccatacgatgttccagattacgcttatccctacgacgtgcctgattatgcatacccatatgatgtccccgactatgcctaa

SEQ ID NO: 60 - DNA, 1419 bp, synthetic construct
  misc_feature 1..1419: note = N286-GS16- pMag -GS16 polynucleotide sequence
  source 1..1419: mol_type = other DNA
atgaacatccccgctctggtggaaaaccagaagaagtactttggcacctacagcgtgatggccatgctgaacgctcagaccgtgctggaccacatccagaaggtggccgatattgagggcgagcagaacgagaacaacgagaatctgtggtttcaccccgtgatgagccacctgtacaacgccaagaacggctacgacaagcagcccgagaaaaccatgttcatcatcgagcggctgcagagctacttcccattcctgaagatcatggccgagaaccagagagagtacagcaacggcaagtacaagcagaaccgcgtggaagtgaacagcaacgacatcttcgaggtgctgaagcgcgccttcggcgtgctgaagatgtacagggacctgaccaaccactacaagacctacgaggaaaagctgaacgacggctgcgagttcctgaccagcacagagcaacctctgagcggcatgatcaacaactactacacagtggccctgcggaacatgaacgagagatacggctacaagacagaggacctggccttcatccaggacaagcggttcaagttcgtgaaggacgcctacggcaagaaaaagtcccaagtgaataccggattcttcctgagcctgcaggactacaacggcgacacacagaagaagctgcacctgagcggagtgggaatcgccctgctgatctgcctgttcctggacaagcagtacatcaacatctttctgagcaggctgcccatcttctccagctacaatgcccagagcgaggaacggcggatcatcatcagatccttcggcatcaacagcatcaagctgcccaaggaccggatccacagcgagaagtccaacccgggatccggaggaagtggcagctctggcggcagtggagggtctggtggcagcggacacaccctgtacgcccccggcggctacgacatcatgggctacctgagacagatcagaaacagacccaacccccaggtggagctgggccccgtggacaccagctgcgccctgatcctgtgcgacctgaagcagaaggacacccccatcgtgtacgccagcgaggccttcctgtatatgaccggctacagcaacgccgaggtgctgggcagaaactgcagattcctgcagagccccgacggcatggtgaagcccaagagcaccagaaagtacgtggacagcaacaccatcaacaccatcagaaaggccatcgacagaaacgccgaggtgcaggtggaggtggtgaacttcaagaagaacggccagagattcgtgaacttcctgaccatcatccccgtgagagacgagaccggcgagtacagatacagcatgggcttccagtgcgagaccgagggaggaagcggcggttccggggggggatccggaagtggttccggggggtag

SEQ ID NO: 61 - DNA, 3099 bp, synthetic construct
  misc_feature 1..3099: note = GS16- nMag -GS16-C287 polynucleotide sequence
  source 1..3099: mol_type = other DNA
atgggaggaagtggcagctctggcggcagtggagggtctggtggcagcggacacaccctgtacgcccccggcggctacgacatcatgggctacctggaccagatcggcaacagacccaacccccaggtggagctgggccccgtggacaccagctgcgccctgatcctgtgcgacctgaagcagaaggacacccccatcgtgtacgccagcgaggccttcctgtatatgaccggctacagcaacgccgaggtgctgggcagaaactgcagattcctgcagagccccgacggcatggtgaagcccaagagcaccagaaagtacgtggacagcaacaccatcaacaccatgagaaaggccatcgacagaaacgccgaggtgcaggtggaggtggtgaacttcaagaagaacggccagagattcgtgaacttcctgaccatgatccccgtgagagacgagaccggcgagtacagatacagcatgggcttccagtgcgagaccgagggaggaagcggcggttccggggggggatccggaagtggttccggggggtgtacaaacaagagcgtggccatggatatgctcaacgaagtgaagcggtgccccgacgagctgttcacaacactgtctgccgagaagcagtcccggttcagaatcatcagcgacgaccacaatgaagtgctgatgaagcggagcagcgacagattcgtgcctctgctgctgcagtatatcgattacggcaagctgttcgaccacatcaggttccacgtgaacatgggcaagctgagatacctgctgaaggccgacaagacctgcatcgacggccagaccagagtcagagtgatcgagcagcccctgaacggcttcggcagactggaagaggccgagacaatgcggaagcaagagaacggcaccttcggcaacagcggcatccggatcagagacttcgagaacatgaagcgggacgacgccaatcctgccaactatccctacatcgtggacacctacacacactacatcctggaaaacaacaaggtcgagatgtttatcaacgacaaagaggacagcgccccactgctgcccgtgatcgaggatgatagatacgtggtcaagacaatccccagctgccggatgagcaccctggaaattccagccatggccttccacatgtttctgttcggcagcaagaaaaccgagaagctgatcgtggacgtgcacaaccggtacaagagactgttccaggccatgcagaaagaagaagtgaccgccgagaatatcgccagcttcggaatcgccgagagcgacctgcctcagaagatcctggatctgatcagcggcaatgcccacggcaaggatgtggacgccttcatcagactgaccgtggacgacatgctgaccgacaccgagcggagaatcaagagattcaaggacgaccggaagtccattcggagcgccgacaacaagatgggaaagagaggcttcaagcagatctccacaggcaagctggccgacttcctggccaaggacatcgtgctgtttcagcccagcgtgaacgatggcgagaacaagatcaccggcctgaactaccggatcatgcagagcgccattgccgtgtacgatagcggcgacgattacgaggccaagcagcagttcaagctgatgttcgagaaggcccggctgatcggcaagggcacaacagagcctcatccatttctgtacaaggtgttcgcccgcagcatccccgccaatgccgtcgagttctacgagcgctacctgatcgagcggaagttctacctgaccggcctgtccaacgagatcaagaaaggcaacagagtggatgtgcccttcatccggcgggaccagaacaagtggaaaacacccgccatgaagaccctgggcagaatctacagcgaggatctgcccgtggaactgcccagacagatgttcgacaatgagatcaagtcccacctgaagtccctgccacagatggaaggcatcgacttcaacaatgccaacgtgacctatctgatcgccgagtacatgaagagagtgctggacgacgacttccagaccttctaccagtggaaccgcaactaccggtacatggacatgcttaagggcgagtacgacagaaagggctccctgcagcactgcttcaccagcgtggaagagagagaaggcctctggaaagagcgggcctccagaacagagcggtacagaaagcaggccagcaacaagatccgcagcaaccggcagatgagaaacgccagcagcgaagagatcgagacaatcctggataagcggctgagcaacagccggaacgagtaccagaaaagcgagaaagtgatccggcgctacagagtgcaggatgccctgctgtttctgctggccaaaaagaccctgaccgaactggccgatttcgacggcgagaggttcaaactgaaagaaatcatgcccgacgccgagaagggaatcctgagcgagatcatgcccatgagcttcaccttcgagaaaggcggcaagaagtacaccatcaccagcgagggcatgaagctgaagaactacggcgacttctttgtgctggctagcgacaagaggatcggcaacctgctggaactcgtgggcagcgacatcgtgtccaaagaggatatcatggaagagttcaacaaatacgaccagtgcaggcccgagatcagctccatcgtgttcaacctggaaaagtgggccttcgacacataccccgagctgtctgccagagtggaccgggaagagaaggtggacttcaagagcatcctgaaaatcctgctgaacaacaagaacatcaacaaagagcagagcgacatcctgcggaagatccggaacgccttcgatcacaacaattaccccgacaaaggcgtggtggaaatcaaggccctgcctgagatcgccatgagcatcaagaaggcctttggggagtacgccatcatgaagggatcccttcaactgcctccacttgaaagactgacactgggtagttcctacccatacgatgttccagattacgcttatccctacgacgtgcctgattatgcatacccatatgatgtccccgactatgcctaa

SEQ ID NO: 62 - DNA, 1614 bp, synthetic construct
  misc_feature 1..1614: note = N351-GS16- pMag -GS16 polynucleotide sequence
  source 1..1614: mol_type = other DNA
atgaacatccccgctctggtggaaaaccagaagaagtactttggcacctacagcgtgatggccatgctgaacgctcagaccgtgctggaccacatccagaaggtggccgatattgagggcgagcagaacgagaacaacgagaatctgtggtttcaccccgtgatgagccacctgtacaacgccaagaacggctacgacaagcagcccgagaaaaccatgttcatcatcgagcggctgcagagctacttcccattcctgaagatcatggccgagaaccagagagagtacagcaacggcaagtacaagcagaaccgcgtggaagtgaacagcaacgacatcttcgaggtgctgaagcgcgccttcggcgtgctgaagatgtacagggacctgaccaaccactacaagacctacgaggaaaagctgaacgacggctgcgagttcctgaccagcacagagcaacctctgagcggcatgatcaacaactactacacagtggccctgcggaacatgaacgagagatacggctacaagacagaggacctggccttcatccaggacaagcggttcaagttcgtgaaggacgcctacggcaagaaaaagtcccaagtgaataccggattcttcctgagcctgcaggactacaacggcgacacacagaagaagctgcacctgagcggagtgggaatcgccctgctgatctgcctgttcctggacaagcagtacatcaacatctttctgagcaggctgcccatcttctccagctacaatgcccagagcgaggaacggcggatcatcatcagatccttcggcatcaacagcatcaagctgcccaaggaccggatccacagcgagaagtccaacaagagcgtggccatggatatgctcaacgaagtgaagcggtgccccgacgagctgttcacaacactgtctgccgagaagcagtcccggttcagaatcatcagcgacgaccacaatgaagtgctgatgaagcggagcagcgacagattcgtgcctctgctgctgcagtatatcgattacggcaagctgttcgaccttccgggatccggaggaagtggcagctctggcggcagtggagggtctggtggcagcggacacaccctgtacgcccccggcggctacgacatcatgggctacctgagacagatcagaaacagacccaacccccaggtggagctgggccccgtggacaccagctgcgccctgatcctgtgcgacctgaagcagaaggacacccccatcgtgtacgccagcgaggccttcctgtatatgaccggctacagcaacgccgaggtgctgggcagaaactgcagattcctgcagagccccgacggcatggtgaagcccaagagcaccagaaagtacgtggacagcaacaccatcaacaccatcagaaaggccatcgacagaaacgccgaggtgcaggtggaggtggtgaacttcaagaagaacggccagagattcgtgaacttcctgaccatcatccccgtgagagacgagaccggcgagtacagatacagcatgggcttccagtgcgagaccgagggaggaagcggcggttccggggggggatccggaagtggttccggggggtag

SEQ ID NO: 63 - DNA, 2904 bp, synthetic construct
  misc_feature 1..2904: note = GS16- nMag -GS16-C352 polynucleotide sequence
  source 1..2904: mol_type = other DNA
atgggaggaagtggcagctctggcggcagtggagggtctggtggcagcggacacaccctgtacgcccccggcggctacgacatcatgggctacctggaccagatcggcaacagacccaacccccaggtggagctgggccccgtggacaccagctgcgccctgatcctgtgcgacctgaagcagaaggacacccccatcgtgtacgccagcgaggccttcctgtatatgaccggctacagcaacgccgaggtgctgggcagaaactgcagattcctgcagagccccgacggcatggtgaagcccaagagcaccagaaagtacgtggacagcaacaccatcaacaccatgagaaaggccatcgacagaaacgccgaggtgcaggtggaggtggtgaacttcaagaagaacggccagagattcgtgaacttcctgaccatgatccccgtgagagacgagaccggcgagtacagatacagcatgggcttccagtgcgagaccgagggaggaagcggcggttccggggggggatccggaagtggttccggggggtgtacacacatcaggttccacgtgaacatgggcaagctgagatacctgctgaaggccgacaagacctgcatcgacggccagaccagagtcagagtgatcgagcagcccctgaacggcttcggcagactggaagaggccgagacaatgcggaagcaagagaacggcaccttcggcaacagcggcatccggatcagagacttcgagaacatgaagcgggacgacgccaatcctgccaactatccctacatcgtggacacctacacacactacatcctggaaaacaacaaggtcgagatgtttatcaacgacaaagaggacagcgccccactgctgcccgtgatcgaggatgatagatacgtggtcaagacaatccccagctgccggatgagcaccctggaaattccagccatggccttccacatgtttctgttcggcagcaagaaaaccgagaagctgatcgtggacgtgcacaaccggtacaagagactgttccaggccatgcagaaagaagaagtgaccgccgagaatatcgccagcttcggaatcgccgagagcgacctgcctcagaagatcctggatctgatcagcggcaatgcccacggcaaggatgtggacgccttcatcagactgaccgtggacgacatgctgaccgacaccgagcggagaatcaagagattcaaggacgaccggaagtccattcggagcgccgacaacaagatgggaaagagaggcttcaagcagatctccacaggcaagctggccgacttcctggccaaggacatcgtgctgtttcagcccagcgtgaacgatggcgagaacaagatcaccggcctgaactaccggatcatgcagagcgccattgccgtgtacgatagcggcgacgattacgaggccaagcagcagttcaagctgatgttcgagaaggcccggctgatcggcaagggcacaacagagcctcatccatttctgtacaaggtgttcgcccgcagcatccccgccaatgccgtcgagttctacgagcgctacctgatcgagcggaagttctacctgaccggcctgtccaacgagatcaagaaaggcaacagagtggatgtgcccttcatccggcgggaccagaacaagtggaaaacacccgccatgaagaccctgggcagaatctacagcgaggatctgcccgtggaactgcccagacagatgttcgacaatgagatcaagtcccacctgaagtccctgccacagatggaaggcatcgacttcaacaatgccaacgtgacctatctgatcgccgagtacatgaagagagtgctggacgacgacttccagaccttctaccagtggaaccgcaactaccggtacatggacatgcttaagggcgagtacgacagaaagggctccctgcagcactgcttcaccagcgtggaagagagagaaggcctctggaaagagcgggcctccagaacagagcggtacagaaagcaggccagcaacaagatccgcagcaaccggcagatgagaaacgccagcagcgaagagatcgagacaatcctggataagcggctgagcaacagccggaacgagtaccagaaaagcgagaaagtgatccggcgctacagagtgcaggatgccctgctgtttctgctggccaaaaagaccctgaccgaactggccgatttcgacggcgagaggttcaaactgaaagaaatcatgcccgacgccgagaagggaatcctgagcgagatcatgcccatgagcttcaccttcgagaaaggcggcaagaagtacaccatcaccagcgagggcatgaagctgaagaactacggcgacttctttgtgctggctagcgacaagaggatcggcaacctgctggaactcgtgggcagcgacatcgtgtccaaagaggatatcatggaagagttcaacaaatacgaccagtgcaggcccgagatcagctccatcgtgttcaacctggaaaagtgggccttcgacacataccccgagctgtctgccagagtggaccgggaagagaaggtggacttcaagagcatcctgaaaatcctgctgaacaacaagaacatcaacaaagagcagagcgacatcctgcggaagatccggaacgccttcgatcacaacaattaccccgacaaaggcgtggtggaaatcaaggccctgcctgagatcgccatgagcatcaagaaggcctttggggagtacgccatcatgaagggatcccttcaactgcctccacttgaaagactgacactgggtagttcctacccatacgatgttccagattacgcttatccctacgacgtgcctgattatgcatacccatatgatgtccccgactatgcctaa

SEQ ID NO: 64 - DNA, 2001 bp, synthetic construct
  misc_feature 1..2001: note = N480-GS16- pMag -GS16 polynucleotide sequence
  source 1..2001: mol_type = other DNA
atgaacatccccgctctggtggaaaaccagaagaagtactttggcacctacagcgtgatggccatgctgaacgctcagaccgtgctggaccacatccagaaggtggccgatattgagggcgagcagaacgagaacaacgagaatctgtggtttcaccccgtgatgagccacctgtacaacgccaagaacggctacgacaagcagcccgagaaaaccatgttcatcatcgagcggctgcagagctacttcccattcctgaagatcatggccgagaaccagagagagtacagcaacggcaagtacaagcagaaccgcgtggaagtgaacagcaacgacatcttcgaggtgctgaagcgcgccttcggcgtgctgaagatgtacagggacctgaccaaccactacaagacctacgaggaaaagctgaacgacggctgcgagttcctgaccagcacagagcaacctctgagcggcatgatcaacaactactacacagtggccctgcggaacatgaacgagagatacggctacaagacagaggacctggccttcatccaggacaagcggttcaagttcgtgaaggacgcctacggcaagaaaaagtcccaagtgaataccggattcttcctgagcctgcaggactacaacggcgacacacagaagaagctgcacctgagcggagtgggaatcgccctgctgatctgcctgttcctggacaagcagtacatcaacatctttctgagcaggctgcccatcttctccagctacaatgcccagagcgaggaacggcggatcatcatcagatccttcggcatcaacagcatcaagctgcccaaggaccggatccacagcgagaagtccaacaagagcgtggccatggatatgctcaacgaagtgaagcggtgccccgacgagctgttcacaacactgtctgccgagaagcagtcccggttcagaatcatcagcgacgaccacaatgaagtgctgatgaagcggagcagcgacagattcgtgcctctgctgctgcagtatatcgattacggcaagctgttcgaccacatcaggttccacgtgaacatgggcaagctgagatacctgctgaaggccgacaagacctgcatcgacggccagaccagagtcagagtgatcgagcagcccctgaacggcttcggcagactggaagaggccgagacaatgcggaagcaagagaacggcaccttcggcaacagcggcatccggatcagagacttcgagaacatgaagcgggacgacgccaatcctgccaactatccctacatcgtggacacctacacacactacatcctggaaaacaacaaggtcgagatgtttatcaacgacaaagaggacagcgccccactgctgcccgtgatcgaggatgatagatacgtggtcaagacaatccccagctgccggatgagcacccttccgggatccggaggaagtggcagctctggcggcagtggagggtctggtggcagcggacacaccctgtacgcccccggcggctacgacatcatgggctacctgagacagatcagaaacagacccaacccccaggtggagctgggccccgtggacaccagctgcgccctgatcctgtgcgacctgaagcagaaggacacccccatcgtgtacgccagcgaggccttcctgtatatgaccggctacagcaacgccgaggtgctgggcagaaactgcagattcctgcagagccccgacggcatggtgaagcccaagagcaccagaaagtacgtggacagcaacaccatcaacaccatcagaaaggccatcgacagaaacgccgaggtgcaggtggaggtggtgaacttcaagaagaacggccagagattcgtgaacttcctgaccatcatccccgtgagagacgagaccggcgagtacagatacagcatgggcttccagtgcgagaccgagggaggaagcggcggttccggggggggatccggaagtggttccggggggtag

SEQ ID NO: 65 - DNA, 2517 bp, synthetic construct
  misc_feature 1..2517: note = GS16- nMag -GS16-C481 polynucleotide sequence
  source 1..2517: mol_type = other DNA
atgggaggaagtggcagctctggcggcagtggagggtctggtggcagcggacacaccctgtacgcccccggcggctacgacatcatgggctacctggaccagatcggcaacagacccaacccccaggtggagctgggccccgtggacaccagctgcgccctgatcctgtgcgacctgaagcagaaggacacccccatcgtgtacgccagcgaggccttcctgtatatgaccggctacagcaacgccgaggtgctgggcagaaactgcagattcctgcagagccccgacggcatggtgaagcccaagagcaccagaaagtacgtggacagcaacaccatcaacaccatgagaaaggccatcgacagaaacgccgaggtgcaggtggaggtggtgaacttcaagaagaacggccagagattcgtgaacttcctgaccatgatccccgtgagagacgagaccggcgagtacagatacagcatgggcttccagtgcgagaccgagggaggaagcggcggttccggggggggatccggaagtggttccggggggtgtacactggaaattccagccatggccttccacatgtttctgttcggcagcaagaaaaccgagaagctgatcgtggacgtgcacaaccggtacaagagactgttccaggccatgcagaaagaagaagtgaccgccgagaatatcgccagcttcggaatcgccgagagcgacctgcctcagaagatcctggatctgatcagcggcaatgcccacggcaaggatgtggacgccttcatcagactgaccgtggacgacatgctgaccgacaccgagcggagaatcaagagattcaaggacgaccggaagtccattcggagcgccgacaacaagatgggaaagagaggcttcaagcagatctccacaggcaagctggccgacttcctggccaaggacatcgtgctgtttcagcccagcgtgaacgatggcgagaacaagatcaccggcctgaactaccggatcatgcagagcgccattgccgtgtacgatagcggcgacgattacgaggccaagcagcagttcaagctgatgttcgagaaggcccggctgatcggcaagggcacaacagagcctcatccatttctgtacaaggtgttcgcccgcagcatccccgccaatgccgtcgagttctacgagcgctacctgatcgagcggaagttctacctgaccggcctgtccaacgagatcaagaaaggcaacagagtggatgtgcccttcatccggcgggaccagaacaagtggaaaacacccgccatgaagaccctgggcagaatctacagcgaggatctgcccgtggaactgcccagacagatgttcgacaatgagatcaagtcccacctgaagtccctgccacagatggaaggcatcgacttcaacaatgccaacgtgacctatctgatcgccgagtacatgaagagagtgctggacgacgacttccagaccttctaccagtggaaccgcaactaccggtacatggacatgcttaagggcgagtacgacagaaagggctccctgcagcactgcttcaccagcgtggaagagagagaaggcctctggaaagagcgggcctccagaacagagcggtacagaaagcaggccagcaacaagatccgcagcaaccggcagatgagaaacgccagcagcgaagagatcgagacaatcctggataagcggctgagcaacagccggaacgagtaccagaaaagcgagaaagtgatccggcgctacagagtgcaggatgccctgctgtttctgctggccaaaaagaccctgaccgaactggccgatttcgacggcgagaggttcaaactgaaagaaatcatgcccgacgccgagaagggaatcctgagcgagatcatgcccatgagcttcaccttcgagaaaggcggcaagaagtacaccatcaccagcgagggcatgaagctgaagaactacggcgacttctttgtgctggctagcgacaagaggatcggcaacctgctggaactcgtgggcagcgacatcgtgtccaaagaggatatcatggaagagttcaacaaatacgaccagtgcaggcccgagatcagctccatcgtgttcaacctggaaaagtgggccttcgacacataccccgagctgtctgccagagtggaccgggaagagaaggtggacttcaagagcatcctgaaaatcctgctgaacaacaagaacatcaacaaagagcagagcgacatcctgcggaagatccggaacgccttcgatcacaacaattaccccgacaaaggcgtggtggaaatcaaggccctgcctgagatcgccatgagcatcaagaaggcctttggggagtacgccatcatgaagggatcccttcaactgcctccacttgaaagactgacactgggtagttcctacccatacgatgttccagattacgcttatccctacgacgtgcctgattatgcatacccatatgatgtccccgactatgcctaa

SEQ ID NO: 66 - DNA, 2211 bp, synthetic construct
  misc_feature 1..2211: note = N550-GS16- pMag -GS16 polynucleotide sequence
  source 1..2211: mol_type = other DNA
atgaacatccccgctctggtggaaaaccagaagaagtactttggcacctacagcgtgatggccatgctgaacgctcagaccgtgctggaccacatccagaaggtggccgatattgagggcgagcagaacgagaacaacgagaatctgtggtttcaccccgtgatgagccacctgtacaacgccaagaacggctacgacaagcagcccgagaaaaccatgttcatcatcgagcggctgcagagctacttcccattcctgaagatcatggccgagaaccagagagagtacagcaacggcaagtacaagcagaaccgcgtggaagtgaacagcaacgacatcttcgaggtgctgaagcgcgccttcggcgtgctgaagatgtacagggacctgaccaaccactacaagacctacgaggaaaagctgaacgacggctgcgagttcctgaccagcacagagcaacctctgagcggcatgatcaacaactactacacagtggccctgcggaacatgaacgagagatacggctacaagacagaggacctggccttcatccaggacaagcggttcaagttcgtgaaggacgcctacggcaagaaaaagtcccaagtgaataccggattcttcctgagcctgcaggactacaacggcgacacacagaagaagctgcacctgagcggagtgggaatcgccctgctgatctgcctgttcctggacaagcagtacatcaacatctttctgagcaggctgcccatcttctccagctacaatgcccagagcgaggaacggcggatcatcatcagatccttcggcatcaacagcatcaagctgcccaaggaccggatccacagcgagaagtccaacaagagcgtggccatggatatgctcaacgaagtgaagcggtgccccgacgagctgttcacaacactgtctgccgagaagcagtcccggttcagaatcatcagcgacgaccacaatgaagtgctgatgaagcggagcagcgacagattcgtgcctctgctgctgcagtatatcgattacggcaagctgttcgaccacatcaggttccacgtgaacatgggcaagctgagatacctgctgaaggccgacaagacctgcatcgacggccagaccagagtcagagtgatcgagcagcccctgaacggcttcggcagactggaagaggccgagacaatgcggaagcaagagaacggcaccttcggcaacagcggcatccggatcagagacttcgagaacatgaagcgggacgacgccaatcctgccaactatccctacatcgtggacacctacacacactacatcctggaaaacaacaaggtcgagatgtttatcaacgacaaagaggacagcgccccactgctgcccgtgatcgaggatgatagatacgtggtcaagacaatccccagctgccggatgagcaccctggaaattccagccatggccttccacatgtttctgttcggcagcaagaaaaccgagaagctgatcgtggacgtgcacaaccggtacaagagactgttccaggccatgcagaaagaagaagtgaccgccgagaatatcgccagcttcggaatcgccgagagcgacctgcctcagaagatcctggatctgatcagcggcaatgcccacggcttcccgggatccggaggaagtggcagctctggcggcagtggagggtctggtggcagcggacacaccctgtacgcccccggcggctacgacatcatgggctacctgagacagatcagaaacagacccaacccccaggtggagctgggccccgtggacaccagctgcgccctgatcctgtgcgacctgaagcagaaggacacccccatcgtgtacgccagcgaggccttcctgtatatgaccggctacagcaacgccgaggtgctgggcagaaactgcagattcctgcagagccccgacggcatggtgaagcccaagagcaccagaaagtacgtggacagcaacaccatcaacaccatcagaaaggccatcgacagaaacgccgaggtgcaggtggaggtggtgaacttcaagaagaacggccagagattcgtgaacttcctgaccatcatccccgtgagagacgagaccggcgagtacagatacagcatgggcttccagtgcgagaccgagggaggaagcggcggttccggggggggatccggaagtggttccggggggtag

SEQ ID NO: 67 - DNA, 2307 bp, synthetic construct
  misc_feature 1..2307: note = GS16- nMag -GS16-C551 polynucleotide sequence
  source 1..2307: mol_type = other DNA
atgggaggaagtggcagctctggcggcagtggagggtctggtggcagcggacacaccctgtacgcccccggcggctacgacatcatgggctacctggaccagatcggcaacagacccaacccccaggtggagctgggccccgtggacaccagctgcgccctgatcctgtgcgacctgaagcagaaggacacccccatcgtgtacgccagcgaggccttcctgtatatgaccggctacagcaacgccgaggtgctgggcagaaactgcagattcctgcagagccccgacggcatggtgaagcccaagagcaccagaaagtacgtggacagcaacaccatcaacaccatgagaaaggccatcgacagaaacgccgaggtgcaggtggaggtggtgaacttcaagaagaacggccagagattcgtgaacttcctgaccatgatccccgtgagagacgagaccggcgagtacagatacagcatgggcttccagtgcgagaccgagggaggaagcggcggttccggggggggatccggaagtggttccggggggtgtacaaaggatgtggacgccttcatcagactgaccgtggacgacatgctgaccgacaccgagcggagaatcaagagattcaaggacgaccggaagtccattcggagcgccgacaacaagatgggaaagagaggcttcaagcagatctccacaggcaagctggccgacttcctggccaaggacatcgtgctgtttcagcccagcgtgaacgatggcgagaacaagatcaccggcctgaactaccggatcatgcagagcgccattgccgtgtacgatagcggcgacgattacgaggccaagcagcagttcaagctgatgttcgagaaggcccggctgatcggcaagggcacaacagagcctcatccatttctgtacaaggtgttcgcccgcagcatccccgccaatgccgtcgagttctacgagcgctacctgatcgagcggaagttctacctgaccggcctgtccaacgagatcaagaaaggcaacagagtggatgtgcccttcatccggcgggaccagaacaagtggaaaacacccgccatgaagaccctgggcagaatctacagcgaggatctgcccgtggaactgcccagacagatgttcgacaatgagatcaagtcccacctgaagtccctgccacagatggaaggcatcgacttcaacaatgccaacgtgacctatctgatcgccgagtacatgaagagagtgctggacgacgacttccagaccttctaccagtggaaccgcaactaccggtacatggacatgcttaagggcgagtacgacagaaagggctccctgcagcactgcttcaccagcgtggaagagagagaaggcctctggaaagagcgggcctccagaacagagcggtacagaaagcaggccagcaacaagatccgcagcaaccggcagatgagaaacgccagcagcgaagagatcgagacaatcctggataagcggctgagcaacagccggaacgagtaccagaaaagcgagaaagtgatccggcgctacagagtgcaggatgccctgctgtttctgctggccaaaaagaccctgaccgaactggccgatttcgacggcgagaggttcaaactgaaagaaatcatgcccgacgccgagaagggaatcctgagcgagatcatgcccatgagcttcaccttcgagaaaggcggcaagaagtacaccatcaccagcgagggcatgaagctgaagaactacggcgacttctttgtgctggctagcgacaagaggatcggcaacctgctggaactcgtgggcagcgacatcgtgtccaaagaggatatcatggaagagttcaacaaatacgaccagtgcaggcccgagatcagctccatcgtgttcaacctggaaaagtgggccttcgacacataccccgagctgtctgccagagtggaccgggaagagaaggtggacttcaagagcatcctgaaaatcctgctgaacaacaagaacatcaacaaagagcagagcgacatcctgcggaagatccggaacgccttcgatcacaacaattaccccgacaaaggcgtggtggaaatcaaggccctgcctgagatcgccatgagcatcaagaaggcctttggggagtacgccatcatgaagggatcccttcaactgcctccacttgaaagactgacactgggtagttcctacccatacgatgttccagattacgcttatccctacgacgtgcctgattatgcatacccatatgatgtccccgactatgcctaa

SEQ ID NO: 68 - DNA, 2433 bp, synthetic construct
  misc_feature 1..2433: note = N624-GS16- pMag -GS16 polynucleotide sequence
  source 1..2433: mol_type = other DNA
atgaacatccccgctctggtggaaaaccagaagaagtactttggcacctacagcgtgatggccatgctgaacgctcagaccgtgctggaccacatccagaaggtggccgatattgagggcgagcagaacgagaacaacgagaatctgtggtttcaccccgtgatgagccacctgtacaacgccaagaacggctacgacaagcagcccgagaaaaccatgttcatcatcgagcggctgcagagctacttcccattcctgaagatcatggccgagaaccagagagagtacagcaacggcaagtacaagcagaaccgcgtggaagtgaacagcaacgacatcttcgaggtgctgaagcgcgccttcggcgtgctgaagatgtacagggacctgaccaaccactacaagacctacgaggaaaagctgaacgacggctgcgagttcctgaccagcacagagcaacctctgagcggcatgatcaacaactactacacagtggccctgcggaacatgaacgagagatacggctacaagacagaggacctggccttcatccaggacaagcggttcaagttcgtgaaggacgcctacggcaagaaaaagtcccaagtgaataccggattcttcctgagcctgcaggactacaacggcgacacacagaagaagctgcacctgagcggagtgggaatcgccctgctgatctgcctgttcctggacaagcagtacatcaacatctttctgagcaggctgcccatcttctccagctacaatgcccagagcgaggaacggcggatcatcatcagatccttcggcatcaacagcatcaagctgcccaaggaccggatccacagcgagaagtccaacaagagcgtggccatggatatgctcaacgaagtgaagcggtgccccgacgagctgttcacaacactgtctgccgagaagcagtcccggttcagaatcatcagcgacgaccacaatgaagtgctgatgaagcggagcagcgacagattcgtgcctctgctgctgcagtatatcgattacggcaagctgttcgaccacatcaggttccacgtgaacatgggcaagctgagatacctgctgaaggccgacaagacctgcatcgacggccagaccagagtcagagtgatcgagcagcccctgaacggcttcggcagactggaagaggccgagacaatgcggaagcaagagaacggcaccttcggcaacagcggcatccggatcagagacttcgagaacatgaagcgggacgacgccaatcctgccaactatccctacatcgtggacacctacacacactacatcctggaaaacaacaaggtcgagatgtttatcaacgacaaagaggacagcgccccactgctgcccgtgatcgaggatgatagatacgtggtcaagacaatccccagctgccggatgagcaccctggaaattccagccatggccttccacatgtttctgttcggcagcaagaaaaccgagaagctgatcgtggacgtgcacaaccggtacaagagactgttccaggccatgcagaaagaagaagtgaccgccgagaatatcgccagcttcggaatcgccgagagcgacctgcctcagaagatcctggatctgatcagcggcaatgcccacggcaaggatgtggacgccttcatcagactgaccgtggacgacatgctgaccgacaccgagcggagaatcaagagattcaaggacgaccggaagtccattcggagcgccgacaacaagatgggaaagagaggcttcaagcagatctccacaggcaagctggccgacttcctggccaaggacatcgtgctgtttcagcccagcgtgaacgatggcgagaacaagatcaacccgggatccggaggaagtggcagctctggcggcagtggagggtctggtggcagcggacacaccctgtacgcccccggcggctacgacatcatgggctacctgagacagatcagaaacagacccaacccccaggtggagctgggccccgtggacaccagctgcgccctgatcctgtgcgacctgaagcagaaggacacccccatcgtgtacgccagcgaggccttcctgtatatgaccggctacagcaacgccgaggtgctgggcagaaactgcagattcctgcagagccccgacggcatggtgaagcccaagagcaccagaaagtacgtggacagcaacaccatcaacaccatcagaaaggccatcgacagaaacgccgaggtgcaggtggaggtggtgaacttcaagaagaacggccagagattcgtgaacttcctgaccatcatccccgtgagagacgagaccggcgagtacagatacagcatgggcttccagtgcgagaccgagggaggaagcggcggttccggggggggatccggaagtggttccggggggtag

SEQ ID NO: 69 - DNA, 2085 bp, synthetic construct
  misc_feature 1..2085: note = GS16- nMag -GS16-C625 polynucleotide sequence
  source 1..2085: mol_type = other DNA
atgggaggaagtggcagctctggcggcagtggagggtctggtggcagcggacacaccctgtacgcccccggcggctacgacatcatgggctacctggaccagatcggcaacagacccaacccccaggtggagctgggccccgtggacaccagctgcgccctgatcctgtgcgacctgaagcagaaggacacccccatcgtgtacgccagcgaggccttcctgtatatgaccggctacagcaacgccgaggtgctgggcagaaactgcagattcctgcagagccccgacggcatggtgaagcccaagagcaccagaaagtacgtggacagcaacaccatcaacaccatgagaaaggccatcgacagaaacgccgaggtgcaggtggaggtggtgaacttcaagaagaacggccagagattcgtgaacttcctgaccatgatccccgtgagagacgagaccggcgagtacagatacagcatgggcttccagtgcgagaccgagggaggaagcggcggttccggggggggatccggaagtggttccggggggtgtacaaccggcctgaactaccggatcatgcagagcgccattgccgtgtacgatagcggcgacgattacgaggccaagcagcagttcaagctgatgttcgagaaggcccggctgatcggcaagggcacaacagagcctcatccatttctgtacaaggtgttcgcccgcagcatccccgccaatgccgtcgagttctacgagcgctacctgatcgagcggaagttctacctgaccggcctgtccaacgagatcaagaaaggcaacagagtggatgtgcccttcatccggcgggaccagaacaagtggaaaacacccgccatgaagaccctgggcagaatctacagcgaggatctgcccgtggaactgcccagacagatgttcgacaatgagatcaagtcccacctgaagtccctgccacagatggaaggcatcgacttcaacaatgccaacgtgacctatctgatcgccgagtacatgaagagagtgctggacgacgacttccagaccttctaccagtggaaccgcaactaccggtacatggacatgcttaagggcgagtacgacagaaagggctccctgcagcactgcttcaccagcgtggaagagagagaaggcctctggaaagagcgggcctccagaacagagcggtacagaaagcaggccagcaacaagatccgcagcaaccggcagatgagaaacgccagcagcgaagagatcgagacaatcctggataagcggctgagcaacagccggaacgagtaccagaaaagcgagaaagtgatccggcgctacagagtgcaggatgccctgctgtttctgctggccaaaaagaccctgaccgaactggccgatttcgacggcgagaggttcaaactgaaagaaatcatgcccgacgccgagaagggaatcctgagcgagatcatgcccatgagcttcaccttcgagaaaggcggcaagaagtacaccatcaccagcgagggcatgaagctgaagaactacggcgacttctttgtgctggctagcgacaagaggatcggcaacctgctggaactcgtgggcagcgacatcgtgtccaaagaggatatcatggaagagttcaacaaatacgaccagtgcaggcccgagatcagctccatcgtgttcaacctggaaaagtgggccttcgacacataccccgagctgtctgccagagtggaccgggaagagaaggtggacttcaagagcatcctgaaaatcctgctgaacaacaagaacatcaacaaagagcagagcgacatcctgcggaagatccggaacgccttcgatcacaacaattaccccgacaaaggcgtggtggaaatcaaggccctgcctgagatcgccatgagcatcaagaaggcctttggggagtacgccatcatgaagggatcccttcaactgcctccacttgaaagactgacactgggtagttcctacccatacgatgttccagattacgcttatccctacgacgtgcctgattatgcatacccatatgatgtccccgactatgcctaa

SEQ ID NO: 70 - DNA, 2736 bp, synthetic construct
  misc_feature 1..2736: note = N725-GS16- pMag -GS16 polynucleotide sequence
  source 1..2736: mol_type = other DNA
atgaacatccccgctctggtggaaaaccagaagaagtactttggcacctacagcgtgatggccatgctgaacgctcagaccgtgctggaccacatccagaaggtggccgatattgagggcgagcagaacgagaacaacgagaatctgtggtttcaccccgtgatgagccacctgtacaacgccaagaacggctacgacaagcagcccgagaaaaccatgttcatcatcgagcggctgcagagctacttcccattcctgaagatcatggccgagaaccagagagagtacagcaacggcaagtacaagcagaaccgcgtggaagtgaacagcaacgacatcttcgaggtgctgaagcgcgccttcggcgtgctgaagatgtacagggacctgaccaaccactacaagacctacgaggaaaagctgaacgacggctgcgagttcctgaccagcacagagcaacctctgagcggcatgatcaacaactactacacagtggccctgcggaacatgaacgagagatacggctacaagacagaggacctggccttcatccaggacaagcggttcaagttcgtgaaggacgcctacggcaagaaaaagtcccaagtgaataccggattcttcctgagcctgcaggactacaacggcgacacacagaagaagctgcacctgagcggagtgggaatcgccctgctgatctgcctgttcctggacaagcagtacatcaacatctttctgagcaggctgcccatcttctccagctacaatgcccagagcgaggaacggcggatcatcatcagatccttcggcatcaacagcatcaagctgcccaaggaccggatccacagcgagaagtccaacaagagcgtggccatggatatgctcaacgaagtgaagcggtgccccgacgagctgttcacaacactgtctgccgagaagcagtcccggttcagaatcatcagcgacgaccacaatgaagtgctgatgaagcggagcagcgacagattcgtgcctctgctgctgcagtatatcgattacggcaagctgttcgaccacatcaggttccacgtgaacatgggcaagctgagatacctgctgaaggccgacaagacctgcatcgacggccagaccagagtcagagtgatcgagcagcccctgaacggcttcggcagactggaagaggccgagacaatgcggaagcaagagaacggcaccttcggcaacagcggcatccggatcagagacttcgagaacatgaagcgggacgacgccaatcctgccaactatccctacatcgtggacacctacacacactacatcctggaaaacaacaaggtcgagatgtttatcaacgacaaagaggacagcgccccactgctgcccgtgatcgaggatgatagatacgtggtcaagacaatccccagctgccggatgagcaccctggaaattccagccatggccttccacatgtttctgttcggcagcaagaaaaccgagaagctgatcgtggacgtgcacaaccggtacaagagactgttccaggccatgcagaaagaagaagtgaccgccgagaatatcgccagcttcggaatcgccgagagcgacctgcctcagaagatcctggatctgatcagcggcaatgcccacggcaaggatgtggacgccttcatcagactgaccgtggacgacatgctgaccgacaccgagcggagaatcaagagattcaaggacgaccggaagtccattcggagcgccgacaacaagatgggaaagagaggcttcaagcagatctccacaggcaagctggccgacttcctggccaaggacatcgtgctgtttcagcccagcgtgaacgatggcgagaacaagatcaccggcctgaactaccggatcatgcagagcgccattgccgtgtacgatagcggcgacgattacgaggccaagcagcagttcaagctgatgttcgagaaggcccggctgatcggcaagggcacaacagagcctcatccatttctgtacaaggtgttcgcccgcagcatccccgccaatgccgtcgagttctacgagcgctacctgatcgagcggaagttctacctgaccggcctgtccaacgagatcaagaaaggcaacagagtggatgtgcccttcatccggcgggaccagaacaagtggaaacccccgggatccggaggaagtggcagctctggcggcagtggagggtctggtggcagcggacacaccctgtacgcccccggcggctacgacatcatgggctacctgagacagatcagaaacagacccaacccccaggtggagctgggccccgtggacaccagctgcgccctgatcctgtgcgacctgaagcagaaggacacccccatcgtgtacgccagcgaggccttcctgtatatgaccggctacagcaacgccgaggtgctgggcagaaactgcagattcctgcagagccccgacggcatggtgaagcccaagagcaccagaaagtacgtggacagcaacaccatcaacaccatcagaaaggccatcgacagaaacgccgaggtgcaggtggaggtggtgaacttcaagaagaacggccagagattcgtgaacttcctgaccatcatccccgtgagagacgagaccggcgagtacagatacagcatgggcttccagtgcgagaccgagggaggaagcggcggttccggggggggatccggaagtggttccggggggtag

SEQ ID NO: 71 - DNA, 1782 bp, synthetic construct
  misc_feature 1..1782: note = GS16- nMag -GS16-C726 polynucleotide sequence
  source 1..1782: mol_type = other DNA
atgggaggaagtggcagctctggcggcagtggagggtctggtggcagcggacacaccctgtacgcccccggcggctacgacatcatgggctacctggaccagatcggcaacagacccaacccccaggtggagctgggccccgtggacaccagctgcgccctgatcctgtgcgacctgaagcagaaggacacccccatcgtgtacgccagcgaggccttcctgtatatgaccggctacagcaacgccgaggtgctgggcagaaactgcagattcctgcagagccccgacggcatggtgaagcccaagagcaccagaaagtacgtggacagcaacaccatcaacaccatgagaaaggccatcgacagaaacgccgaggtgcaggtggaggtggtgaacttcaagaagaacggccagagattcgtgaacttcctgaccatgatccccgtgagagacgagaccggcgagtacagatacagcatgggcttccagtgcgagaccgagggaggaagcggcggttccggggggggatccggaagtggttccggggggtgtacaacacccgccatgaagaccctgggcagaatctacagcgaggatctgcccgtggaactgcccagacagatgttcgacaatgagatcaagtcccacctgaagtccctgccacagatggaaggcatcgacttcaacaatgccaacgtgacctatctgatcgccgagtacatgaagagagtgctggacgacgacttccagaccttctaccagtggaaccgcaactaccggtacatggacatgcttaagggcgagtacgacagaaagggctccctgcagcactgcttcaccagcgtggaagagagagaaggcctctggaaagagcgggcctccagaacagagcggtacagaaagcaggccagcaacaagatccgcagcaaccggcagatgagaaacgccagcagcgaagagatcgagacaatcctggataagcggctgagcaacagccggaacgagtaccagaaaagcgagaaagtgatccggcgctacagagtgcaggatgccctgctgtttctgctggccaaaaagaccctgaccgaactggccgatttcgacggcgagaggttcaaactgaaagaaatcatgcccgacgccgagaagggaatcctgagcgagatcatgcccatgagcttcaccttcgagaaaggcggcaagaagtacaccatcaccagcgagggcatgaagctgaagaactacggcgacttctttgtgctggctagcgacaagaggatcggcaacctgctggaactcgtgggcagcgacatcgtgtccaaagaggatatcatggaagagttcaacaaatacgaccagtgcaggcccgagatcagctccatcgtgttcaacctggaaaagtgggccttcgacacataccccgagctgtctgccagagtggaccgggaagagaaggtggacttcaagagcatcctgaaaatcctgctgaacaacaagaacatcaacaaagagcagagcgacatcctgcggaagatccggaacgccttcgatcacaacaattaccccgacaaaggcgtggtggaaatcaaggccctgcctgagatcgccatgagcatcaagaaggcctttggggagtacgccatcatgaagggatcccttcaactgcctccacttgaaagactgacactgggtagttcctacccatacgatgttccagattacgcttatccctacgacgtgcctgattatgcatacccatatgatgtccccgactatgcctaa

SEQ ID NO: 72 - DNA, 3345 bp, synthetic construct
  misc_feature 1..3345: note = N928-GS16- pMag -GS16 polynucleotide sequence
  source 1..3345: mol_type = other DNA
atgaacatccccgctctggtggaaaaccagaagaagtactttggcacctacagcgtgatggccatgctgaacgctcagaccgtgctggaccacatccagaaggtggccgatattgagggcgagcagaacgagaacaacgagaatctgtggtttcaccccgtgatgagccacctgtacaacgccaagaacggctacgacaagcagcccgagaaaaccatgttcatcatcgagcggctgcagagctacttcccattcctgaagatcatggccgagaaccagagagagtacagcaacggcaagtacaagcagaaccgcgtggaagtgaacagcaacgacatcttcgaggtgctgaagcgcgccttcggcgtgctgaagatgtacagggacctgaccaaccactacaagacctacgaggaaaagctgaacgacggctgcgagttcctgaccagcacagagcaacctctgagcggcatgatcaacaactactacacagtggccctgcggaacatgaacgagagatacggctacaagacagaggacctggccttcatccaggacaagcggttcaagttcgtgaaggacgcctacggcaagaaaaagtcccaagtgaataccggattcttcctgagcctgcaggactacaacggcgacacacagaagaagctgcacctgagcggagtgggaatcgccctgctgatctgcctgttcctggacaagcagtacatcaacatctttctgagcaggctgcccatcttctccagctacaatgcccagagcgaggaacggcggatcatcatcagatccttcggcatcaacagcatcaagctgcccaaggaccggatccacagcgagaagtccaacaagagcgtggccatggatatgctcaacgaagtgaagcggtgccccgacgagctgttcacaacactgtctgccgagaagcagtcccggttcagaatcatcagcgacgaccacaatgaagtgctgatgaagcggagcagcgacagattcgtgcctctgctgctgcagtatatcgattacggcaagctgttcgaccacatcaggttccacgtgaacatgggcaagctgagatacctgctgaaggccgacaagacctgcatcgacggccagaccagagtcagagtgatcgagcagcccctgaacggcttcggcagactggaagaggccgagacaatgcggaagcaagagaacggcaccttcggcaacagcggcatccggatcagagacttcgagaacatgaagcgggacgacgccaatcctgccaactatccctacatcgtggacacctacacacactacatcctggaaaacaacaaggtcgagatgtttatcaacgacaaagaggacagcgccccactgctgcccgtgatcgaggatgatagatacgtggtcaagacaatccccagctgccggatgagcaccctggaaattccagccatggccttccacatgtttctgttcggcagcaagaaaaccgagaagctgatcgtggacgtgcacaaccggtacaagagactgttccaggccatgcagaaagaagaagtgaccgccgagaatatcgccagcttcggaatcgccgagagcgacctgcctcagaagatcctggatctgatcagcggcaatgcccacggcaaggatgtggacgccttcatcagactgaccgtggacgacatgctgaccgacaccgagcggagaatcaagagattcaaggacgaccggaagtccattcggagcgccgacaacaagatgggaaagagaggcttcaagcagatctccacaggcaagctggccgacttcctggccaaggacatcgtgctgtttcagcccagcgtgaacgatggcgagaacaagatcaccggcctgaactaccggatcatgcagagcgccattgccgtgtacgatagcggcgacgattacgaggccaagcagcagttcaagctgatgttcgagaaggcccggctgatcggcaagggcacaacagagcctcatccatttctgtacaaggtgttcgcccgcagcatccccgccaatgccgtcgagttctacgagcgctacctgatcgagcggaagttctacctgaccggcctgtccaacgagatcaagaaaggcaacagagtggatgtgcccttcatccggcgggaccagaacaagtggaaaacacccgccatgaagaccctgggcagaatctacagcgaggatctgcccgtggaactgcccagacagatgttcgacaatgagatcaagtcccacctgaagtccctgccacagatggaaggcatcgacttcaacaatgccaacgtgacctatctgatcgccgagtacatgaagagagtgctggacgacgacttccagaccttctaccagtggaaccgcaactaccggtacatggacatgcttaagggcgagtacgacagaaagggctccctgcagcactgcttcaccagcgtggaagagagagaaggcctctggaaagagcgggcctccagaacagagcggtacagaaagcaggccagcaacaagatccgcagcaaccggcagatgagaaacgccagcagcgaagagatcgagacaatcctggataagcggctgagcaacagccggaacgagtaccagaaaagcgagaaagtgatccggcgctacagagtgcaggatgccctgctgtttctgctggccaaaaagaccctgaccgaactggccgatttcgacggcgagaggttcaaactgaaagaaatcatgcccgacgccgagaagggaatcctgagcgagttcccgggatccggaggaagtggcagctctggcggcagtggagggtctggtggcagcggacacaccctgtacgcccccggcggctacgacatcatgggctacctgagacagatcagaaacagacccaacccccaggtggagctgggccccgtggacaccagctgcgccctgatcctgtgcgacctgaagcagaaggacacccccatcgtgtacgccagcgaggccttcctgtatatgaccggctacagcaacgccgaggtgctgggcagaaactgcagattcctgcagagccccgacggcatggtgaagcccaagagcaccagaaagtacgtggacagcaacaccatcaacaccatcagaaaggccatcgacagaaacgccgaggtgcaggtggaggtggtgaacttcaagaagaacggccagagattcgtgaacttcctgaccatcatccccgtgagagacgagaccggcgagtacagatacagcatgggcttccagtgcgagaccgagggaggaagcggcggttccggggggggatccggaagtggttccggggggtag

SEQ ID NO: 73 - DNA, 1173 bp, synthetic construct
  misc_feature 1..1173: note = GS16- nMag -GS16-C929 polynucleotide sequence
  source 1..1173: mol_type = other DNA
atgggaggaagtggcagctctggcggcagtggagggtctggtggcagcggacacaccctgtacgcccccggcggctacgacatcatgggctacctggaccagatcggcaacagacccaacccccaggtggagctgggccccgtggacaccagctgcgccctgatcctgtgcgacctgaagcagaaggacacccccatcgtgtacgccagcgaggccttcctgtatatgaccggctacagcaacgccgaggtgctgggcagaaactgcagattcctgcagagccccgacggcatggtgaagcccaagagcaccagaaagtacgtggacagcaacaccatcaacaccatgagaaaggccatcgacagaaacgccgaggtgcaggtggaggtggtgaacttcaagaagaacggccagagattcgtgaacttcctgaccatgatccccgtgagagacgagaccggcgagtacagatacagcatgggcttccagtgcgagaccgagggaggaagcggcggttccggggggggatccggaagtggttccggggggtgtacaatcatgcccatgagcttcaccttcgagaaaggcggcaagaagtacaccatcaccagcgagggcatgaagctgaagaactacggcgacttctttgtgctggctagcgacaagaggatcggcaacctgctggaactcgtgggcagcgacatcgtgtccaaagaggatatcatggaagagttcaacaaatacgaccagtgcaggcccgagatcagctccatcgtgttcaacctggaaaagtgggccttcgacacataccccgagctgtctgccagagtggaccgggaagagaaggtggacttcaagagcatcctgaaaatcctgctgaacaacaagaacatcaacaaagagcagagcgacatcctgcggaagatccggaacgccttcgatcacaacaattaccccgacaaaggcgtggtggaaatcaaggccctgcctgagatcgccatgagcatcaagaaggcctttggggagtacgccatcatgaagggatcccttcaactgcctccacttgaaagactgacactgggtagttcctacccatacgatgttccagattacgcttatccctacgacgtgcctgattatgcatacccatatgatgtccccgactatgcctaa

SEQ ID NO: 74 - protein, 150 aa, synthetic construct
  REGION 1..150: note = nMagHigh1 amino acid sequence
HTLYAPGGYDIMGYLDQIGNRPNPQVELGPVDTSCALILCDLKQKDTPIVYASEAFLYMTGYSNAEVLGRNCRFLQSPDGMVKPKSTRKYVDSNTINTIRKAIDRNAEVQVEVVNFKKNGQRFVNFLTIIPVRDETGEYRYSMGFQCETE

SEQ ID NO: 75 - DNA, 450 bp, synthetic construct
  misc_feature 1..450: note = nMagHigh1 polynucleotide sequence
  source 1..450: mol_type = other DNA
cacaccctgtacgcccccggcggctacgacatcatgggctacctggaccagatcggcaacagacccaacccccaggtggagctgggccccgtggacaccagctgcgccctgatcctgtgcgacctgaagcagaaggacacccccatcgtgtacgccagcgaggccttcctgtatatgaccggctacagcaacgccgaggtgctgggcagaaactgcagattcctgcagagccccgacggcatggtgaagcccaagagcaccagaaagtacgtggacagcaacaccatcaacaccatcagaaaggccatcgacagaaacgccgaggtgcaggtggaggtggtgaacttcaagaagaacggccagagattcgtgaacttcctgaccatcatccccgtgagagacgagaccggcgagtacagatacagcatgggcttccagtgcgagaccgag